European Patent Application EP 4 365 309 A2, published May 8, 2024. Title: Methods and Systems for Analyzing Nucleic Acid Molecules. Applicant: The Board of Trustees of the Leland Stanford Junior University. The sequence listing filed with the application follows.

SEQUENCE LISTING (1358 sequences)

SEQ ID NO: 1 - DNA, 100 bp, Homo sapiens
  source 1..100: mol_type = other DNA
tctcttctggcccacagccgcagcaatggcgctgagttcctctgctggagttcatcctgctagctgggttcccgagctgccggtctgagcctgaggcatg

SEQ ID NO: 2 - DNA, 100 bp, Homo sapiens
  source 1..100: mol_type = other DNA
gagcctcctggagactgggggcctcctccctggagatccacccccaaaaccgacgtcttgaggctggtgagcccccgagcctcctctccgtctgctcgca

SEQ ID NO: 3 - DNA, 100 bp, Homo sapiens
  source 1..100: mol_type = other DNA
gatcccagttctgaccccagggcctcccacagatctcttccccatgcccctgtcctggccgttgctggctccggcgtccagcccgtcccctgctgcctgg

SEQ ID NO: 4 - DNA, 100 bp, Homo sapiens
  source 1..100: mol_type = other DNA
ccatgttgctggcttacttggcatttcccatgatctcacactgctggcttatttggcatttcccatgatcccctgctgctggtttacttggcattcccta

SEQ ID NO: 5 - DNA, 100 bp, Homo sapiens
  source 1..100: mol_type = other DNA
tgatcccatgttgctggtttacttagcatttcccatgatcccatgttgctggcttacttggcatttcccatgataccatgttgctggcttacttggcatt

SEQ ID NO: 6 - DNA, 100 bp, Homo sapiens
  source 1..100: mol_type = other DNA
atagattagaggaaggaattctagatgaaattaagtaaatgagttatttaagtcaactaatacaagtcctcaaaactttgattatatagagagctaaact

SEQ ID NO: 7 - DNA, 100 bp, Homo sapiens
  source 1..100: mol_type = other DNA
gataaatatagacaaatatagtgagcctataaattaaagctatactatgatgaaaaaataaatgaataattgtgaaatagccaaaaatactaaaatacag

SEQ ID NO: 8 - DNA, 100 bp, Homo sapiens
  source 1..100: mol_type = other DNA
aatgaataattgtgaaatagccaaaaatactaaaatacagctataaggttaaaaataaatctgaataaaaaatgtaggagggaaaagtgattaccttacc

SEQ ID NO: 9 - DNA, 100 bp, Homo sapiens
  source 1..100: mol_type = other DNA
gacatgcatcaaatgtaaacaaatgattacagccattttataaaaagtcatattctttaaaacattttttgtcatcattaaaaattaaaaggcaataaag

SEQ ID NO: 10 - DNA, 100 bp, Homo sapiens
  source 1..100: mol_type = other DNA
tgtcattgtcgtgaaacagtacgtgatcttaagggaagaaacatctcactagagtttgcacaagttccttcttcttctaactgtagatctggtggcaaag

SEQ ID NO: 11 - DNA, 100 bp, Homo sapiens
  source 1..100: mol_type = other DNA
gaggagcccctgggtccccaggtctgggaagtgtagttgaagagaagatggtattttcagttctgcctacttctagaacaggcaaattcagagaagaatt

SEQ ID NO: 12 - DNA, 100 bp, Homo sapiens
  source 1..100: mol_type = other DNA
agtagaaaaaaagggcgtcgtgctggattctccttctggatggtacatgacagtggatgccctcagtttttcagagaaattactctcatctgaatttgat

SEQ ID NO: 13 - DNA, 100 bp, Homo sapiens
  source 1..100: mol_type = other DNA
ctggagaggttgttcgtggctccatctggaaaaggttcacaactgctacattttagtcctacaataaaattattcagatgtaaatgaaaaagtaactaaa

SEQ ID NO: 14 - DNA, 100 bp, Homo sapiens
  source 1..100: mol_type = other DNA
acccgagacctctcactgagcccgagccgcgcgcgacatgagccacgggaagggaaccgacatgctcccggagatcgccgccgccgtgggcttcctctcc

SEQ ID NO: 15 - DNA, 100 bp, Homo sapiens
  source 1..100: mol_type = other DNA
agcctcctgaggacccggggctgcgtgagcgagcagaggcttaaggtcttcagcggggcgctccaggaggcactcacaggtgagcgcatgccgaggggcc

SEQ ID NO: 16 - DNA, 100 bp, Homo sapiens
  source 1..100: mol_type = other DNA
tggcgccaccgggggtcggccccatccctgccagggccgtctttcttctactcctgcggcagggtgacccacgggagcagctttgggactcggtggccct

SEQ ID NO: 17 - DNA, 100 bp, Homo sapiens
  source 1..100: mol_type = other DNA
cctccgacccccggggcggcccgcagtccccagtttcctgggtcctcctccccagccctgtgctcgggtctcggccgtggcggttctgatggggcgcgcc

SEQ ID NO: 18 - DNA, 100 bp, Homo sapiens
  source 1..100: mol_type = other DNA
cctctacgctctcggaggcgcagaccctggtcctggagtgccagcccgagtccccagcttatgcccctgtctcattacgggctcgtctccctcgctggac

SEQ ID NO: 19 - DNA, 100 bp, Homo sapiens
  source 1..100: mol_type = other DNA
cctcgagatcttaagaccctcgatggatgttgttgcgggccgcccggtcggccgaggggtcccgatgagggaagaaggtgcagtcgagccttttcaacaa

SEQ ID NO: 20 - DNA, 100 bp, Homo sapiens
  source 1..100: mol_type = other DNA
tttggagtcccagtgcggttcttcctgccggtcggggtgcgctgtgcctggggtagtccactggttgctgactggcttcaagttggaatttgggccccct

SEQ ID NO: 21 - DNA, 100 bp, Homo sapiens
  source 1..100: mol_type = other DNA
ttgtgttatctttggttccccttagccatctgccacctattgtggtagggaggagagcctcgtagctcgtgaccctgccgtgcgggccttcaagttggga

SEQ ID NO: 22 - DNA, 100 bp, Homo sapiens
  source 1..100: mol_type = other DNA
ggtgaagagataagcagcccgctcgctggctggggagagacctctctcccagctgtttctagctggttactgtcagttttgggaagcgatagccatctcg

SEQ ID NO: 23 - DNA, 100 bp, Homo sapiens
  source 1..100: mol_type = other DNA
gaacgcacccacacagaccctgccttctgaggaaaacagatgtttcatcaaaacaacccagttttcactcccttaggcactgctaaggaaggttctctga

SEQ ID NO: 24 - DNA, 100 bp, Homo sapiens
  source 1..100: mol_type = other DNA
ctcttctgaaggaagcagagggaacacagggtgggaggtccagtgacttgctgtggacccaacaatgttggcagccttcctggccctgaaacttcagctc

SEQ ID NO: 25 - DNA, 100 bp, Homo sapiens
  source 1..100: mol_type = other DNA
acaggtctccagaggccctgcctggacatgccagtcccagtcacacccttcccttgctttgggggtgtgccaaaagcaatacactggccactagagagta

SEQ ID NO: 26 - DNA, 100 bp, Homo sapiens
  source 1..100: mol_type = other DNA
ccctagagctctagaatcccctcccaacacgcacacacacacacacacacactctctctctcacacacacacactcagtcacacacacacacacacacac

SEQ ID NO: 27 - DNA, 100 bp, Homo sapiens
  source 1..100: mol_type = other DNA
ctttcagatctttcgcagcgtcccaacagggcaaaggctccagcattctgccagaaggaattcccgcctccacattcccggtccccggctgtgctgaggg

SEQ ID NO: 28 - DNA, 100 bp, Homo sapiens
  source 1..100: mol_type = other DNA
gctgcccccaagcaagcccagcgttggggaccctccctccactctgtcggagagctgccaacgccccccgcccacgggggccccacttcgggcctcctca

SEQ ID NO: 29 - DNA, 100 bp, Homo sapiens
  source 1..100: mol_type = other DNA
gggcctacggaggccagggccctgggcagcctggaccagctcagggaatcagaggactctgcgctttgcacgctcacagtcgtctcctctggccttttgc

SEQ ID NO: 30 - DNA, 100 bp, Homo sapiens
  source 1..100: mol_type = other DNA
ccacttcaggctccccagagcccggcatgccacagggcagatatcctttccccatcttcccagggggttctccatcgcggggcccgcccctttctggggc

SEQ ID NO: 31 - DNA, 100 bp, Homo sapiens
  source 1..100: mol_type = other DNA
tgggcttgtctcactgcccagaaactgcccctgcctctccaccagggcctctgggggctgcaggtcctcaagctcacgggctctcccagacggctcagtg

SEQ ID NO: 32 - DNA, 100 bp, Homo sapiens
  source 1..100: mol_type = other DNA
agggcaagatcctgtggacggtgtggcccagtggatgtaactctcgctgccacttccgtggccatcgttaagctagctccgaacagccccaatgagggag

SEQ ID NO: 33 - DNA, 100 bp, Homo sapiens
  source 1..100: mol_type = other DNA
ctaggcagctccgagttcccggggtaggagagccccttttgtcaatttccatagctgtgggtgagccacagcggggactggcagggatacccttctccat

SEQ ID NO: 34 - DNA, 100 bp, Homo sapiens
  source 1..100: mol_type = other DNA
ccttacaaaagcggatggaccctgagcctctgatcctgtaggggcagcccggccgggaagaggtggcattcctttcttcacctgcgaggagcataggctg

SEQ ID NO: 35 - DNA, 100 bp, Homo sapiens
  source 1..100: mol_type = other DNA
ggccctcctttcctcccggagtcggttcctgaagtctctggacattgctccccccaggactttgtcctccgttcctcgctccgggcgccctgaaccagga

SEQ ID NO: 36 - DNA, 100 bp, Homo sapiens
  source 1..100: mol_type = other DNA
cccttccagggggctgactgctgctgcggaaggggcacggggagggcgagcgagccctgcccaaacgcgggctgcggggcgcttgaatggcggagctctg

SEQ ID NO: 37 - DNA, 100 bp, Homo sapiens
  source 1..100: mol_type = other DNA
tgcctggatgtgcgcctcaaacatgcccactttctggttcacctgcacgttctgcaactcgcgctgcaagatccgcagcttcctcttggcctcctccggc

SEQ ID NO: 38 - DNA, 100 bp, Homo sapiens
  source 1..100: mol_type = other DNA
cctggcggggagagggtaccggctgccaccacctgctgccggtcccctcgcaggcgaccagcccaacttgggctgctcacgctactgccgctgctgccgc

SEQ ID NO: 39 - DNA, 100 bp, Homo sapiens
  source 1..100: mol_type = other DNA
tgccactgccgctgctactattcagcctgcgccggccgctccgccagcccccggggctccggggctcctcgggggacagcgactcggctggggggaagag

SEQ ID NO: 40 - DNA, 100 bp, Homo sapiens
  source 1..100: mol_type = other DNA
gaaagaggcgcctctcccggggctgaaaacgctgccggggctcagcactgccctcctcgggggcgggggcgtctcgctgccactgggccccgggccgccg

SEQ ID NO: 41 - DNA, 100 bp, Homo sapiens
  source 1..100: mol_type = other DNA
ccgctcttcatctcgttggcgctattcatgatcaccaggctattgagcgcatagcagtacacagccatagtactgggtcccgcgctgcccgccgccgcgg

SEQ ID NO: 42 - DNA, 100 bp, Homo sapiens
  source 1..100: mol_type = other DNA
ctcccgctcctgctccgccgccggcgcctcctcctcccggcgctcccggctcagccccggaggcccggcagccgcggctccgcgcgcagatggggcggca

SEQ ID NO: 43 - DNA, 100 bp, Homo sapiens
  source 1..100: mol_type = other DNA
aagtgcgaaggaagtgtcaggctggatgtcaaaatgaacaccttggagaactggatgatggaacagacggtaaaaatcagctaaacatcagagaaaatgg

SEQ ID NO: 44 - DNA, 100 bp, Homo sapiens
  source 1..100: mol_type = other DNA
aggaagaggtcaaaactgtgaacaggaactagaagaaagtgtagcagaaaaagacttgtcacaaacttcgagagatttggagaaaatgatgtcaaaacac

SEQ ID NO: 45 - DNA, 100 bp, Homo sapiens
  source 1..100: mol_type = other DNA
atcttcctcaagcccatgctgagtatctctgatttggttaatttcttggtaagtgttccaagtacagacaacaaagcagaaaagcactgattacagggaa

SEQ ID NO: 46 - DNA, 100 bp, Homo sapiens
  source 1..100: mol_type = other DNA
tatgcagaatgatccttcagatcatgtgaacgctataattaaatgttgctaccaaatccccactaccctttctcccacctagaaaaagttaatgcatgaa

SEQ ID NO: 47 - DNA, 100 bp, Homo sapiens
  source 1..100: mol_type = other DNA
ttcagtatgagcaaattgtgatttataaaaacaaacaaacaaacaaacaaacaaaacccaccctattcactccgtaggggaataaagctttcttgcatta

SEQ ID NO: 48 - DNA, 100 bp, Homo sapiens
  source 1..100: mol_type = other DNA
aacaaacaaaacccaccctattcactccgtaggggaataaagctttcttgcattaagtcacgcatcatgggggtaggaaaaaagcacagtactgaaagaa

SEQ ID NO: 49 - DNA, 100 bp, Homo sapiens
  source 1..100: mol_type = other DNA
gtgaagtgatccaaatgtagcccagagatcctaaagaaaaaacgatgctcatgtgttacaaaacaaaattttaaggcaatcagtgaggaatcacagacaa

SEQ ID NO: 50 - DNA, 100 bp, Homo sapiens
  source 1..100: mol_type = other DNA
atttccttagtgcttttatcaaggttgaatctgaatataaattactagaggaaagcaaatcagatttcacatctgaaaattaaaaacaaaattcttagct

SEQ ID NO: 51 - DNA, 100 bp, Homo sapiens
  source 1..100: mol_type = other DNA
aggcaacaaaatgagatcctgtccctagaaaacatttcaaaaaattaacagcatggtgacgcacacttgtagccctagctacttgggaggctgagtggga

SEQ ID NO: 52 - DNA, 100 bp, Homo sapiens
  source 1..100: mol_type = other DNA
aagaacttaagcagactaggatataaagtataggagcgtattgtgtacaggaacgggaaatactgtttcctggatcttttgtttcacttacgcacacacc

SEQ ID NO: 53 - DNA, 100 bp, Homo sapiens
  source 1..100: mol_type = other DNA
cacacccgccagtagtgtaccaggttgcgatggaaatctctctctttctgtggatgagtttgtggaagcccttgctccagcatgccctccttcctgccca

SEQ ID NO: 54 - DNA, 100 bp, Homo sapiens
  source 1..100: mol_type = other DNA
cccctggaccattccttcccttcacagcactgtcccatgggtaggccacagcccagcacaggccccagcctggcggctgcagcaggagccccatcccagg

SEQ ID NO: 55 - DNA, 100 bp, Homo sapiens
  source 1..100: mol_type = other DNA
gcctgaggggccatgcgggggtctgggtgggagtgggaaccgctgaggaaggtgaagggaaatatggtgagatgacaggcccgctgtcagggagagtggg

SEQ ID NO: 56 - DNA, 100 bp, Homo sapiens
  source 1..100: mol_type = other DNA
aggagccctggagtgccctacctctgtggggctggaactccctgtatccgagctagggtcttccacacgcatgctactaccccaagtgccacagctggag

SEQ ID NO: 57 - DNA, 100 bp, Homo sapiens
  source 1..100: mol_type = other DNA
tcatctcccactggataacagtgttgtcgggaacttccatccagcactggcggacactcccgtcgcagctgctcctgactgagcaagtcatttaaggggg

SEQ ID NO: 58 - DNA, 100 bp, Homo sapiens
  source 1..100: mol_type = other DNA
tccttggcactcataagcactcacagaatggggctggcagtgcgcccggcctccctgggatgggtccagaatggtaggaagcgcagtccgggagggaccc

SEQ ID NO: 59 - DNA, 100 bp, Homo sapiens
  source 1..100: mol_type = other DNA
actgcttagagctctcagccctagatggcgtatcacagttaatgctctataaaacccatcatggcttttccctagtaagcctcaaatcgctgcaagcaag

SEQ ID NO: 60 - DNA, 100 bp, Homo sapiens
  source 1..100: mol_type = other DNA
gcttcatatatgagagtttctgctgtctcctggagccatctcacccaaagccactgactctgggagaccagcccaggccacaaaccagcaaagcaccagt

SEQ ID NO: 61 - DNA, 100 bp, Homo sapiens
  source 1..100: mol_type = other DNA
tatagttagagctgcattataaagtggccagaggacatttctttgcagtgagatgtgtatcgtgaacgtttggggcctgtgctcgcctagtcctcatctt

SEQ ID NO: 62 - DNA, 100 bp, Homo sapiens
  source 1..100: mol_type = other DNA
tgcttttctaggtacacaaagccatcccatggctgcaaatgttagctgggctgggctccctacttgcctcaagccccttcatagacccttcaggcacatg

SEQ ID NO: 63 - DNA, 100 bp, Homo sapiens
  source 1..100: mol_type = other DNA
cttttctctggacgtttacagacaggtcctcagaggtcagagcaggttgtcctagggagcagggaggcttcctagggaggtcagactccaaatagtggat

SEQ ID NO: 64 - DNA, 100 bp, Homo sapiens
  source 1..100: mol_type = other DNA
atggcaaaaatgcagctgcagactcatgaggagtcgccctgggctgccactagggctcccacagtgtgcgctgccaacctgctgcccgtgcagaaactct

SEQ ID NO: 65 - DNA, 100 bp, Homo sapiens
  source 1..100: mol_type = other DNA
caactgtgccctgcactgttagggcccttgtcaaaacaacacatttctcagtgattctgagactctttctcttatctatagaagtcataactcaagagta

SEQ ID NO: 66 - DNA, 100 bp, Homo sapiens
  source 1..100: mol_type = other DNA
aaatcataccaatattttacataaaccctagaatttttatagatctattatttctttttagagtacatattggaagtaacttcacaaggaacattttctt

SEQ ID NO: 67 - DNA, 100 bp, Homo sapiens
  source 1..100: mol_type = other DNA
tctggtcaaaccactccacaaataaagtggactgatcctcttgactctatgtgtaagtgcccattgtgtgtgcacagagctggtgagaacggccatggtg

SEQ ID NO: 68 - DNA, 100 bp, Homo sapiens
  source 1..100: mol_type = other DNA
ctaggtgggggtggtgttggtggagttggactagattatctgggatcatgcgaaatggaaattcatttctagctggctggcttcagaaggtgccatctcc

SEQ ID NO: 69 - DNA, 100 bp, Homo sapiens
  source 1..100: mol_type = other DNA
tatttttatatgaagcgtgctttggaactcagggcaacgaagggtgggtgtgctgcacaaggacagcagaagagtgagctgactggtccctgaaatcgca

SEQ ID NO: 70 - DNA, 100 bp, Homo sapiens
  source 1..100: mol_type = other DNA
gttggaaagtggattaccagtgcagtagaactcttcacggaggcctggaccatcaggtctaatggtgttgttccaggtgggtggtcatgtggagcaaaaa

SEQ ID NO: 71 - DNA, 100 bp, Homo sapiens
  source 1..100: mol_type = other DNA
tatttgaaatcagcgagcacgtacctgagagatgacttttccacttgggctagtctcttgatatttctggtcctgtttcttcatctgtaaactgggttag

SEQ ID NO: 72 - DNA, 100 bp, Homo sapiens
  source 1..100: mol_type = other DNA
aaggagaccaagaagcgtatttaaaatcttgatgttttgagtttcttcctagcttccccctattccttaataaagttctaaattgttttgttggagctct

SEQ ID NO: 73 - DNA, 100 bp, Homo sapiens
  source 1..100: mol_type = other DNA
ttgcagccattctgagggctttgcatgcttttctgaccttgcagtaaactcaatgctttaggcaaagaatggccacgtcatccgaccccctcagagttta

SEQ ID NO: 74 - DNA, 100 bp, Homo sapiens
  source 1..100: mol_type = other DNA
gaattcagaacaggtctgaagaagaccaggcagcggctgagtcaaggaaagcctccgtccgcttttatttcccctgtgcctcttccaggactgtgctggg

SEQ ID NO: 75 - DNA, 100 bp, Homo sapiens
  source 1..100: mol_type = other DNA
ataacaggctcccgggggttactttggctgggctgggctaaaacctccctgcagagcaggccctgagccctgcctctgcgcctgggtggtgtcagcccct

SEQ ID NO: 76 - DNA, 100 bp, Homo sapiens
  source 1..100: mol_type = other DNA
ccaccttctgactgttccagcaactctctaagccctcccaaaggcctcaaggcctgtaaccatatgcagcaattttcagccataccaggagaggtcaact

SEQ ID NO: 77 - DNA, 100 bp, Homo sapiens
  source 1..100: mol_type = other DNA
gtaatcttggccacctgcctaagaggaagtggctagcttcacttctgaccctcagcaactgccaggtggcctcttggaaatccccctctgggggattcca

SEQ ID NO: 78 - DNA, 100 bp, Homo sapiens
  source 1..100: mol_type = other DNA
cccgttgggtgggagagcagtagttaaaatgtaaaataagaatcttttgctgggagaagtcaacagatagggagaagtcagctgataacagaaatagttt

SEQ ID NO: 79 - DNA, 100 bp, Homo sapiens
  source 1..100: mol_type = other DNA
taaaactaacttcactgttaaccaagcagttcaacatgaaagactgaatctcttatgtttaatattttcttctcttttaatcttcataactaattttttt

SEQ ID NO: 80 - DNA, 100 bp, Homo sapiens
  source 1..100: mol_type = other DNA
cagataattgtataaaataaccatggtagcaaaataatgtgatcactggaaaataagcagggaaaaacatgctatgaagatactcctatctgggtgaatt

SEQ ID NO: 81 - DNA, 100 bp, Homo sapiens
  source 1..100: mol_type = other DNA
cttgatagctttacatttttcatctggcatttaaacattaaacagttaatgtatttgacatgaaaattatttcaagttatcttattagttttaatagagt

SEQ ID NO: 82 - DNA, 100 bp, Homo sapiens
  source 1..100: mol_type = other DNA
ttaaaaagtgtttaaaagagttttcaaaaggctctaaaatcattttgaaatagtttaaaacagttttgaatcgttgtaagttagttttaatagagcttta

SEQ ID NO: 83 - DNA, 100 bp, Homo sapiens
  source 1..100: mol_type = other DNA
aaaaggccctaaaatagtcctatcaagttgttgcagaccaaaataatctccttaaatatcacttttgagatcagctggggtaaacgacagcaacacaatg

SEQ ID NO: 84 - DNA, 100 bp, Homo sapiens
  source 1..100: mol_type = other DNA
acaaatcattaaactattttagagattatgaaattaaaatactcagattaaaattttcctatcacagaattaaggtactggaaaatatgtttaagttttt

SEQ ID NO: 85 - DNA, 100 bp, Homo sapiens
  source 1..100: mol_type = other DNA
attaatcacattgctataggtttagatattttgtacaactgaaataaaatcacacactggcagctacatttttgaaagttaaaaacatggtcacgaatat

SEQ ID NO: 86 - DNA, 100 bp, Homo sapiens
  source 1..100: mol_type = other DNA
atcttattttaaaatcagttaatataccttaatggtatttaatgccaaattcaaagtgaattgatcaagccctcagtggccaggtcatgggtgtgatttt

SEQ ID NO: 87 - DNA, 100 bp, Homo sapiens
  source 1..100: mol_type = other DNA
tactctgaaagaattacatatttctttctttttggttgagcttttgttatttaaatacatttgatgagaggatattgaaataattaaatagcactgaaaa

SEQ ID NO: 88 - DNA, 100 bp, Homo sapiens
  source 1..100: mol_type = other DNA
aaaaaaagctttaaattatttacaatcccctaatggaaattttcactaatgagatatcataatgaatgtgaattttatttctgaaatctctaataaatca

SEQ ID NO: 89 - DNA, 100 bp, Homo sapiens
  source 1..100: mol_type = other DNA
aagctttaaattatttacaatcccctaatggaaattttcactaatgagatatcataatgaatgtgaattttatttctgaaatctctaataaatcagtctt

SEQ ID NO: 90 - DNA, 100 bp, Homo sapiens
  source 1..100: mol_type = other DNA
ctccctggttttcccagctcagcgcccattacgtttctgttctctttcccttagtggcattatttgtatcactgtgcatcaggaaagctggctacggcag

SEQ ID NO: 91 - DNA, 100 bp, Homo sapiens
  source 1..100: mol_type = other DNA
catcaatcgggcagacacagggtggccacggccactagcggcaaggcggctgccccaagagcgcggtggcatggccaccaaagccactcaatcgagaaag

SEQ ID NO: 92 - DNA, 100 bp, Homo sapiens
  source 1..100: mol_type = other DNA
accgcggctctgtctacagctcgcggtgccacggccttcttggcagaataaaaatgtagacaagtaataacagaggataatgaaagaacatactctttaa

SEQ ID NO: 93 - DNA, 100 bp, Homo sapiens
  source 1..100: mol_type = other DNA
aatatttcctatttttttcacagacccacggtcattaaaaaatgcaattatttactttttttcatttaaacacatttctttgagattgagcttttgggaa

SEQ ID NO: 94 - DNA, 100 bp, Homo sapiens
  source 1..100: mol_type = other DNA
taaccacctttccaccattacaataagagataatttcacgtttagtctaatgtacaaattggatttttaaaaaatgagctctatctgtgaagcccttatt

SEQ ID NO: 95 - DNA, 100 bp, Homo sapiens
  source 1..100: mol_type = other DNA
aaaatgagctctatctgtgaagcccttattcctatagaatgtgtctttttgagtttattacttattacagactctaaaaacaacattgctgctgattttc

SEQ ID NO: 96 - DNA, 100 bp, Homo sapiens
  source 1..100: mol_type = other DNA
aagtaagctgcctcttctacatagcaaataggtacacttcacttttccctgatttttcttagggcgtgctattgatttttattgttgtctgacaaaataa

SEQ ID NO: 97 - DNA, 100 bp, Homo sapiens
  source 1..100: mol_type = other DNA
tttatcaaacaaaagggagaaagactaaaaaatgtatttttccacttttctgtatcatgcataatcagcaacaaccaatacaatatttggcaagagtgaa

SEQ ID NO: 98 - DNA, 100 bp, Homo sapiens
  source 1..100: mol_type = other DNA
caaaaataaatttacttttgctccttagaaatacaagggttcctttttagttacactttttttttttactttgtgtcattcagtttagagcaatttaatc

SEQ ID NO: 99 - DNA, 100 bp, Homo sapiens
  source 1..100: mol_type = other DNA
tttttttctccaaatccatttttgaagctgagtttaacttttgcaacccatggcaaatcttaaatgccctcatttaccaatctttaccaaactcctattt

SEQ ID NO: 100 - DNA, 100 bp, Homo sapiens
  source 1..100: mol_type = other DNA
aagcctctaaaagtcaatactggccatcagacccaaatttcagaagacaatagtgaaaaattacttacgtttaatctccagtcgtgtcccttggccgaag

SEQ ID NO: 101 - DNA, 100 bp, Homo sapiens
  source 1..100: mol_type = other DNA
gtgatccacagtgttaacttaattactttccccttaacaaaaatctcttttcgctgttaatatcactaacctgaccgatgcagagaaaatcttgcaattg

SEQ ID NO: 102 - DNA, 100 bp, Homo sapiens
  source 1..100: mol_type = other DNA
agatgcctcacttaactggctagcgcttggctgttccttaagatgaactaattttctatcccttactcatctgactttttgaaagaatctggtactcttt

SEQ ID NO: 103 - DNA, 100 bp, Homo sapiens
  source 1..100: mol_type = other DNA
ggaattgacctgagctaatatctcaaacacaaaaacgctccaaatttaaaaccttataagaaaaagcattaggaaagtgcacttacgtttgatctccacc

SEQ ID NO: 104 - DNA, 100 bp, Homo sapiens
  source 1..100: mol_type = other DNA
ttggtccctccgccgaaagtgagccacagtgagggatctcaccctttcccctcaacaaaaacctctcttgaagccaatcatatgagataggctgcttgtt

SEQ ID NO: 105 - DNA, 100 bp, Homo sapiens
  source 1..100: mol_type = other DNA
cagagaaaaatctagctatttcttccccatttcccccatgaatcctattctcctctcaaacccaatgattcgtctatttgctcagctttttaagttcatt

SEQ ID NO: 106 - DNA, 100 bp, Homo sapiens
  source 1..100: mol_type = other DNA
ttctggtgtcctgctatttacttctgggtcaccaggtttattcaaccaaaatatcacaaaacttgcacaaatgatacaatggcactaaaatctcacgaat

SEQ ID NO: 107 - DNA, 100 bp, Homo sapiens
  source 1..100: mol_type = other DNA
aattgagacagatgtacttacgtttgatatccactttggtcccagggccgaaagtgaatcacagtgattcgtcttaacttttccctttacaaaaacctcc

SEQ ID NO: 108 - DNA, 100 bp, Homo sapiens
  source 1..100: mol_type = other DNA
ctgaaagctcagcaagcctctttcccccaatgaagttattttgatttagaaatcttaaaaattagccacaagctagcgtcctgtggaacaatttcccctc

SEQ ID NO: 109 - DNA, 100 bp, Homo sapiens
  source 1..100: mol_type = other DNA
ctctgtacctaacctgggaatgaagtttgttagatccctggcatccgactaatgaaaatccacacaaaggaacacaaagtaaactaattagcaacagtga

SEQ ID NO: 110 - DNA, 100 bp, Homo sapiens
  source 1..100: mol_type = other DNA
agaatcagtggaaaaaagtacttacgtttgatctccagcttggtcccctggccaaaagtgtacacacaatggttcctcttaacttccctcctatacaaaa

SEQ ID NO: 111 - DNA, 100 bp, Homo sapiens
  source 1..100: mol_type = other DNA
actccctttctgacaattgaccaaggctctgtccagaacatgttatgttccccaggacatttctgaagctattacttagacaagttattctcacccaatg

SEQ ID NO: 112 - DNA, 100 bp, Homo sapiens
  source 1..100: mol_type = other DNA
actgaatcttgcttgctcttcaaagaaaatgtgcaatcaattctcgagtttgactacagacttatctttatcttttccctgaaggatatcagaggctgat

SEQ ID NO: 113 - DNA, 100 bp, Homo sapiens
  source 1..100: mol_type = other DNA
tgcagagtcaccttatagatcacttcatagacacagggaacagaagacacagacaactgaggaagcaaagtttaaattctactcacgtttgatttccacc

SEQ ID NO: 114 - DNA, 100 bp, Homo sapiens
  source 1..100: mol_type = other DNA
ttggtcccttggccgaacgtccaccacagtgagagctctccattgtcttgctgaacaaaaacccttctcaccaaaggggaacagagtcctgggtcagctg

SEQ ID NO: 115 - DNA, 100 bp, Homo sapiens
  source 1..100: mol_type = other DNA
atcaacttaaggctcataactttgaaatgcattttgaaatgtagctccagatggtatacgaaaccaaagtgaagactaatagagtagaaaagtagacttt

SEQ ID NO: 116 - DNA, 100 bp, Homo sapiens
  source 1..100: mol_type = other DNA
acttggttggtttgtctgttttcacagcacaggaagagctcagctcttactgagctggaccaggcgcatgccatctttggagctgccatggagtcccagt

SEQ ID NO: 117 - DNA, 100 bp, Homo sapiens
  source 1..100: mol_type = other DNA
gttccatagtgtttccatagtaatctcatcaacaacactgaagaccttttcagtattttcttttgagtccagctccatttttgcagccttgtatctctct

SEQ ID NO: 118 - DNA, 100 bp, Homo sapiens
  source 1..100: mol_type = other DNA
ccgcgcccagccgagtgcctgtttatttttacctgctttcagattctcttctacccttctaaattataagctgtttgatgttttatttgccctgtatttg

SEQ ID NO: 119 - DNA, 100 bp, Homo sapiens
  source 1..100: mol_type = other DNA
ggaggctccgtccagtatctttacttagcaaatgcttaacaaacattttcagaataaataaaaaaaaatacctaattgaaagtcaataatagatcagaga

SEQ ID NO: 120 - DNA, 100 bp, Homo sapiens
  source 1..100: mol_type = other DNA
tgctatcatagaccaaagactaatactgactgccacaacagtaacttttacaacagaaatcataactacaattctaaagattaggggtaggtttatttga

SEQ ID NO: 121 - DNA, 100 bp, Homo sapiens
  source 1..100: mol_type = other DNA
ttctgtcactggcagctttgctagttgccttgaatagcagaattagcatttggtctcaccagaagatgaggaaggagagggatcaagttagaggtggaga

SEQ ID NO: 122 - DNA, 100 bp, Homo sapiens
  source 1..100: mol_type = other DNA
gttaacattggcaagtgaaatttaatgtgcaaaatagctgaccaagggcatagtccttttttaaaggggacacaaagtgattttctctgcagacatacac

SEQ ID NO: 123 - DNA, 100 bp, Homo sapiens
  source 1..100: mol_type = other DNA
gcaataccaatcataaagggtgacatttattgagcacttactaagtgccagacattgtacatggatcatcacatttaattattcccaagactctatgaac

SEQ ID NO: 124 - DNA, 100 bp, Homo sapiens
  source 1..100: mol_type = other DNA
tgagcacttactaagtgccagacattgtacatggatcatcacatttaattattcccaagactctatgaactaggaactaatattatcccctactttgtag

SEQ ID NO: 125 - DNA, 100 bp, Homo sapiens
  source 1..100: mol_type = other DNA
gtgcaaaaacttgagggcagagaggtcaaggaactggcttatggcagtaagtggcagagctgtgacctaaactcagatcccatgtttttaactgaactat

SEQ ID NO: 126 - DNA, 100 bp, Homo sapiens
  source 1..100: mol_type = other DNA
atgcagattatactccaggagtaaagtcactcaacggaagcaacaagcgtgacagggaatgctgggatgggggaaggtaaaaggaactccttagactggg

SEQ ID NO: 127 - DNA, 100 bp, Homo sapiens
  source 1..100: mol_type = other DNA
ataagtgtgtacagacgtatgtataagactacacatggaaatattgtttaaagagtgaaaaataactaaaatcctcattaataggagtttggttaaactg

SEQ ID NO: 128 - DNA, 100 bp, Homo sapiens
  source 1..100: mol_type = other DNA
tgctagagctttacaatgtagcacaaagcagacattaaggggaagacgtagacttctatatagttacgtggaaggtgtttgtgaaaatgcaggtcactga

SEQ ID NO: 129 - DNA, 100 bp, Homo sapiens
  source 1..100: mol_type = other DNA
agagtatgtgtggtgagatatcatgatcccatctacattgaatatatatgtatataaatacgggctgaattttaaaagacataaattgtgcttggtagtt

SEQ ID NO: 130 - DNA, 100 bp, Homo sapiens
  source 1..100: mol_type = other DNA
aaatacgggctgaattttaaaagacataaattgtgcttggtagttatctcctgggattgcagaggaggaacaatgacactttatgccatctcctcctact

SEQ ID NO: 131 - DNA, 100 bp, Homo sapiens
  source 1..100: mol_type = other DNA
cttctgtatggtgatgtgaatatattcattttatagtttttagaaataataaaactgtactaattttgaaaaacagtaaactctgacattgcctattagc

SEQ ID NO: 132 - DNA, 100 bp, Homo sapiens
  source 1..100: mol_type = other DNA
attctcgatattcctgtgcaatgcataaacataactttttaaaagatatgtacacacatgtgtgagttttctttgtcaaatacttttctataatctttaa

SEQ ID NO: 133 - DNA, 100 bp, Homo sapiens
  source 1..100: mol_type = other DNA
atcaagcatgccaaaaaggtaaaagctttcctgtttcagtgtaggagatagtcgtctgcaaaggaaagagatgtaggggatagaaacaggaatgaaaaag

SEQ ID NO: 134 - DNA, 100 bp, Homo sapiens
  source 1..100: mol_type = other DNA
atgactgagctgttcgagggacttatgttcctaagtgagctaattggaaatctaatatgaacagtgcaaccgaataactattgtaaagcagtatttgtaa

SEQ ID NO: 135 - DNA, 100 bp, Homo sapiens
  source 1..100: mol_type = other DNA
acaataaaagatgattatcataagtaccattgttgcaaaaactattttattgatcacatgcagtggtgatctgtaggaatgattgttgtgatgtttgctg

SEQ ID NO: 136 - DNA, 100 bp, Homo sapiens
  source 1..100: mol_type = other DNA
taacataaaatgaaacatgggaagtggctgagatctttaggatgtgtgtggttcattttttgaaagcaaatgttgtctcagaagcatctgtgagactctg

SEQ ID NO: 137 - DNA, 100 bp, Homo sapiens
  source 1..100: mol_type = other DNA
ccaggatccaccgttctacaaaatatctgtgatggacattgataagattgatctgttgaggaaaggcaaggtgtcagtaagatagtctgagagcttcttg

SEQ ID NO: 138 - DNA, 100 bp, Homo sapiens
  source 1..100: mol_type = other DNA
gatttcatgtaaaagagtgctggaaatagaatttcttggggaacattccaactaactcatcactgaaggtgctttacattgaaccctcagcaaagttaga

SEQ ID NO: 139 - DNA, 100 bp, Homo sapiens
  source 1..100: mol_type = other DNA
ttatcagaaaaaaaatataaactgctgtggaggggacaggaaggaaagtcagggagggaggggggcaaggagagaaagagcgagagagaggagagaaaga

SEQ ID NO: 140 - DNA, 100 bp, Homo sapiens
  source 1..100: mol_type = other DNA
agagaggagagagagagcacaagtacacacttcaatgcacatctataaatcatcctgaaaactactgataaattattttagcaatgttcctcagatgtaa

SEQ ID NO: 141 - DNA, 100 bp, Homo sapiens
  source 1..100: mol_type = other DNA
catttcaagaaatatcatttttgctttttatttggcataatttactagccaatttaggaagttcccctcacatcagtaacatacagtacatcacccagta

SEQ ID NO: 142 - DNA, 100 bp, Homo sapiens
  source 1..100: mol_type = other DNA
tgtcagaggacacaatggcataagtttgccttttgcaaggtttgagggatggccatttccctacctgactcaggaaagtctgtagctgatatccatcttc

SEQ ID NO: 143 - DNA, 100 bp, Homo sapiens
  source 1..100: mol_type = other DNA
aagtttgtggttctttctctctatatatatatttgagctcagcagtcatgctggagtccagagtaggtgattctttctgctttagcttgactcctcctta

SEQ ID NO: 144 - DNA, 100 bp, Homo sapiens
  source 1..100: mol_type = other DNA
tatatatttgagctcagcagtcatgctggagtccagagtaggtgattctttctgctttagcttgactcctccttaagattgtaactctctcagttttaca

SEQ ID NO: 145 - DNA, 100 bp, Homo sapiens
  source 1..100: mol_type = other DNA
ttttttgtcagacgtaagctgacattccacaaggagaggaggaaattctgtggttcacatccagtggtgcttggaacctgattggttgtcattcttccag

SEQ ID NO: 146 - DNA, 100 bp, Homo sapiens
  source 1..100: mol_type = other DNA
ctagtttgtcacgagtggatatctgtcctggattcccaaggatcaaggctgccccattagccaggaagtagggagatagaggaggtcacttgagaaagag

SEQ ID NO: 147 - DNA, 100 bp, Homo sapiens
  source 1..100: mol_type = other DNA
ctgcttctttgccgcctccaggttgtgtctgtttcctctcatatctgaagacagatgtgctggcagaagcaaagtcctttgtccggccacgtgcaaatgc

SEQ ID NO: 148 - DNA, 100 bp, Homo sapiens
  source 1..100: mol_type = other DNA
atgggacataaatatgaacagagattcttgtcccactctagaaaatgtagatgttcatcttgtttccaaggggacagtaaggctgcaggtgttttttgac

SEQ ID NO: 149 - DNA, 100 bp, Homo sapiens
  source 1..100: mol_type = other DNA
cttttgtactcactggttgtttttgcataggcccctccaggccacgaccagctgtttggattttataaacgggccgtttgcattgtgaactgagctacaa

SEQ ID NO: 150 - DNA, 100 bp, Homo sapiens
  source 1..100: mol_type = other DNA
caggcaggcaggggcagcaagatggtgttgcagacccaggtcttcatttctctgttgctctggatctctggtgaggaattaaaaagtgccacagtctttt

SEQ ID NO: 151 - DNA, 100 bp, Homo sapiens
  source 1..100: mol_type = other DNA
cagagtaatatctgtgtagaaataaaaaaaattaagatatagttggaaataatgactatttccaatatggatccaattatctgctgacttataatactac

SEQ ID NO: 152 - DNA, 100 bp, Homo sapiens
  source 1..100: mol_type = other DNA
attaagatatagttggaaataatgactatttccaatatggatccaattatctgctgacttataatactactagaaagcaaatttaaatgacatatttcaa

SEQ ID NO: 153 - DNA, 100 bp, Homo sapiens
  source 1..100: mol_type = other DNA
ttatatctgagacagcgtgtataagtttatgtataatcattgtccattactgactacaggtgcctacggggacatcgtgatgacccagtctccagactcc

SEQ ID NO: 154 - DNA, 100 bp, Homo sapiens
  source 1..100: mol_type = other DNA
ctggctgtgtctctgggcgagagggccaccatcaactgcaagtccagccagagtgttttatacagctccaacaataagaactacttagcttggtaccagc

SEQ ID NO: 155 - DNA, 100 bp, Homo sapiens
  source 1..100: mol_type = other DNA
agaaaccaggacagcctcctaagctgctcatttactgggcatctacccgggaatccggggtccctgaccgattcagtggcagcgggtctgggacagattt

SEQ ID NO: 156 - DNA, 100 bp, Homo sapiens
  source 1..100: mol_type = other DNA
cactctcaccatcagcagcctgcaggctgaagatgtggcagtttattactgtcagcaatattatagtactcctcccacagtgcttcagcctcgaacacaa

SEQ ID NO: 157 - DNA, 100 bp, Homo sapiens
  source 1..100: mol_type = other DNA
acctcctccccatacgctgggccagtaggtctttgctgcagcagctgcttcctctgcacacagcccccaacatgcatgcttcctctgtgtgttggggagg

SEQ ID NO: 158 - DNA, 100 bp, Homo sapiens
  source 1..100: mol_type = other DNA
aatacatgaaaacaactaccgaaatgttatgaaattatagtttagtagaactaacaagtgcattaatgcaaaagaaaagtagggctcagtaatcagggaa

SEQ ID NO: 159 - DNA, 100 bp, Homo sapiens
  source 1..100: mol_type = other DNA
ccaagtgtgcattgtaaaagtgcagcctctctaacactgggtttcatcacaagtaacagaacaggatgcctgatgcagggaaaaaagaaaggcaattgtt

SEQ ID NO: 160 - DNA, 100 bp, Homo sapiens
  source 1..100: mol_type = other DNA
gatctctggtaagagaaacacttcctctcctctgtgccaccaagtcccctgcatatccacaaaaataatatattttcataaggaattgattttcctcatt

SEQ ID NO: 161 - DNA, 100 bp, Homo sapiens
  source 1..100: mol_type = other DNA
ctctgcaaatatgatgcatttgatttatgttttttactttgctccataatcagataccagggcagaaacgacactcacgcagtctccagcattcatgtca

SEQ ID NO: 162 - DNA, 100 bp, Homo sapiens
  source 1..100: mol_type = other DNA
gcgactccaggagacaaagtcaacatctcctgcaaagccagccaagacattgatgatgatatgaactggtaccaacagaaaccaggagaagctgctattt

SEQ ID NO: 163 - DNA, 100 bp, Homo sapiens
  source 1..100: mol_type = other DNA
tcattattcaagaagctactactctcgttcctggaatcccacctcgattcagtggcagcgggtatggaacagattttaccctcacaattaataacataga

SEQ ID NO: 164 - DNA, 100 bp, Homo sapiens
  source 1..100: mol_type = other DNA
atctgaggatgctgcatattacttctgtctacaacatgataatttccctctcacagtgatacaccctgttacaaaaacctccaagttctctcagtgggat

SEQ ID NO: 165 - DNA, 100 bp, Homo sapiens
  source 1..100: mol_type = other DNA
gccctctgtcctggagacacggccaaggaggctggagactgggtcagcacaatgtccccattgcagcctgaaatgataaagacagataaattatatcaga

SEQ ID NO: 166 - DNA, 100 bp, Homo sapiens
  source 1..100: mol_type = other DNA
tatactgagactgtccccatgtaggccatgcattggtgacacttgtaaccacagtcatatgcaacatcttgagtaaccagaaaacaaaagataactgggg

SEQ ID NO: 167 - DNA, 100 bp, Homo sapiens
  source 1..100: mol_type = other DNA
aacttacaacctacaatgagtgccctaaatccaacaaccaagaatccagagacacaaaaaacaatgatggccacatgagtttgcccgatgtttccctata

SEQ ID NO: 168 - DNA, 100 bp, Homo sapiens
  source 1..100: mol_type = other DNA
taccaacaccatcagagtgtggctgcatctgaggaccactctcagctgatagaggcatcaggaggagcagctggggcagccctgcctcacacatctgctt

SEQ ID NO: 169 - DNA, 100 bp, Homo sapiens
  source 1..100: mol_type = other DNA
ggggtttatgttcgggtgtgtaacactgtgggagaataactattatactgttggcagtaataagttgcaaaatcatcaggctgcaggctgctgatggtga

SEQ ID NO: 170 - DNA, 100 bp, Homo sapiens
  source 1..100: mol_type = other DNA
gccgctgaaccttgatgggaccccactttctaaactagacgccttatagatcaggagcttaggggctttccctggtttctgctgataccaggccaaccag

SEQ ID NO: 171 - DNA, 100 bp, Homo sapiens
  source 1..100: mol_type = other DNA
ctactaatactctgactggcccggcaagtgatggtgactctgtctcctacagatgcagacagggtggaaggagactgggtcatctggatgtcacatttgg

SEQ ID NO: 172 - DNA, 100 bp, Homo sapiens
  source 1..100: mol_type = other DNA
ggatgtcacatttggcacctgagattggaaatagaaacacaaatattcatactattgatcatattataggaagacttccctgaataaccaggcagtactg

SEQ ID NO: 173 - DNA, 100 bp, Homo sapiens
  source 1..100: mol_type = other DNA
agcacactgggctgagtaaattcctagtgttctccttccttacctgggagccagagcagcaggagccccaggagctgagcggggaccctcatgtccatgc

SEQ ID NO: 174 - DNA, 100 bp, Homo sapiens
  source 1..100: mol_type = other DNA
gggactattttattatgagaaacaatttttaggtatttttttgagaattttaaatattcctcaggagccgatagagtaatgtatttcattggtgtatcag

SEQ ID NO: 175 - DNA, 100 bp, Homo sapiens
  source 1..100: mol_type = other DNA
gattatttaggagaatattcttgtttgtaggaaacacatagtaaaatgttagatggtaggattctcaagtcttcaaaagactctcataagattccgggta

SEQ ID NO: 176 - DNA, 100 bp, Homo sapiens
  source 1..100: mol_type = other DNA
tattcttgtttgtaggaaacacatagtaaaatgttagatggtaggattctcaagtcttcaaaagactctcataagattccgggtagggaagggggtaatt

SEQ ID NO: 177 - DNA, 100 bp, Homo sapiens
  source 1..100: mol_type = other DNA
tgtaagtattaggtaatggtgttatgcctttgttcttactagtattagatcaagcaatttattacagatatacaaagatgataccgtgttgtctccatgc

SEQ ID NO: 178 - DNA, 100 bp, Homo sapiens
  source 1..100: mol_type = other DNA
atgcagcactcacagatccaccactatcaagaactgcaggtctctttaatacccagagactaaatgaggtgcaccttattcttgttttgggtaccttcat

SEQ ID NO: 179 - DNA, 100 bp, Homo sapiens
  source 1..100: mol_type = other DNA
ttgggtgtgtaacactgtgggagggtaactataatactgttgacagtaataagttgcaaaatcttcagactgcaggcagctgatggtgagagtgaaatct

SEQ ID NO: 180 - DNA, 100 bp, Homo sapiens
  source 1..100: mol_type = other DNA
ctgactcgcccgacaagtgatggtgactctgtctcctgtagatgcagagaatgaggatggagactgggtcatccggatggcacatctggcacctgagatt

SEQ ID NO: 181 - DNA, 100 bp, Homo sapiens
  source 1..100: mol_type = other DNA
ctttcccctggagacaaagacagggtgcctggagactgcgtcaacacaatttctccggtggtatctgagattggaaataaaacagaaaagtcacccatgt

SEQ ID NO: 182 - DNA, 100 bp, Homo sapiens
  source 1..100: mol_type = other DNA
aatctaaatcaaacccattgtcttcccagaagagccagaattattgctttatattgagctttaattattgtattgactgagcagagttgccaggtaacag

SEQ ID NO: 183 - DNA, 100 bp, Homo sapiens
  source 1..100: mol_type = other DNA
gacttgagagggttttcactgacatgcaaaaccatcccatgttcccctcacctgggagccagagtagcaggaggaagagaagctgcgctggggtttccat

SEQ ID NO: 184 - DNA, 100 bp, Homo sapiens
  source 1..100: mol_type = other DNA
agctcttctccagagctctgacccaggcattgatatgggctctggactgcagggcggctgggagggacatgcaaagcagctggggcgggtgctgggcttg

SEQ ID NO: 185 - DNA, 100 bp, Homo sapiens
  source 1..100: mol_type = other DNA
cagctgcagagacaatctgcctcccctttctgctctcagcagcccatgcccaggtgatcaggccagaaaaggccgttggctcagtctgagggtagaactt

SEQ ID NO: 186 - DNA, 100 bp, Homo sapiens
  source 1..100: mol_type = other DNA
ctcccctgcggccacagaatttaacccctgtgtcctcttgtctcaccatcacctagattgagccacagaatgtttggtacaagtctgttagaaacaaaat

SEQ ID NO: 187 - DNA, 100 bp, Homo sapiens
  source 1..100: mol_type = other DNA
agaaggctgtggtttcatttttctctttctgctccaacttgtgcccagtcagctccctaaatgcatgatggatcaggttgaaaggaagagtctattacaa

SEQ ID NO: 188 - DNA, 100 bp, Homo sapiens
  source 1..100: mol_type = other DNA
ctttatcttccggatatacttgtatttacttgttagtgatctttcctgagggtccagaagctgtctcattctttgcagaaattaaaagagtaacattcaa

SEQ ID NO: 189 - DNA, 100 bp, Homo sapiens
  source 1..100: mol_type = other DNA
ttaacctcagcactgtgggtgtgaggactttcacaactgcacagataagtgagacctgggctccaaatcctcagggtagtgataccatttccctaaagac

SEQ ID NO: 190 - DNA, 100 bp, Homo sapiens
  source 1..100: mol_type = other DNA
agaagatggttttgtccatgcaggcaaagaactatttcttgggtgatcctctaaactatccagtctttttattctgtatagctggtatagtttaccctta

SEQ ID NO: 191 - DNA, 100 bp, Homo sapiens
  source 1..100: mol_type = other DNA
ggctatatatgtatttgttcatatttcaaaaatacacagtttcaaaatggaactcaagggatccaaggctcaaaggggtctccagaagaccccacaccat

SEQ ID NO: 192 - DNA, 100 bp, Homo sapiens
  source 1..100: mol_type = other DNA
cccctttctgtgtcagtcttccccagagcacagatccttgtttctgcttgaatcttcctcactctcacagatctgatcatcacatgccccactctggagg

SEQ ID NO: 193 - DNA, 100 bp, Homo sapiens
  source 1..100: mol_type = other DNA
acaacatgtgcatgtccaatacaggaaaggaacacacataggagtgtagtgagacccccagagatcactgttgttagaggcagtggggccccagaactca

SEQ ID NO: 194 - DNA, 100 bp, Homo sapiens
  source 1..100: mol_type = other DNA
ggagcagcagcgggtggagaccccatgggctggccgagacaagaggactcctcagccagtcctcctgacctgagacaggtctcaggaatgtgcggaggac

SEQ ID NO: 195 - DNA, 100 bp, Homo sapiens
  source 1..100: mol_type = other DNA
acaccgggacatacatttcccttcatgctcccaacatacacatgcaaacatacacagacccatacaggcacgcgcgagcagccatgccccaccccctccc

SEQ ID NO: 196 - DNA, 100 bp, Homo sapiens
  source 1..100: mol_type = other DNA
ccaacacacacacgtataaaagtgtgtgtatatgggcaaactgctcgcatccccaaatggcaggctctttccctagaggcgcccagtccgcggcggggag

SEQ ID NO: 197 - DNA, 100 bp, Homo sapiens
  source 1..100: mol_type = other DNA
aagctcactcactggggccattgactgggatccagtctgtggccatgtcatggtttctatttttgaggttatagctaatgagcaacatgaggttaagaca

SEQ ID NO: 198 - DNA, 100 bp, Homo sapiens
  source 1..100: mol_type = other DNA
cacttttcataaggccccagccagcatcataaatatgtgtgtgagcatgttcacactcaggttatgtcttctttatgtgcaccctctaccacacacacac

SEQ ID NO: 199 - DNA, 100 bp, Homo sapiens
  source 1..100: mol_type = other DNA
gccaagaaccacgactctctaattttacttcccagcaggtattcagtgcataatagttcctacttagaagtatcatatttgcccaaacacaaggtgatac

SEQ ID NO: 200 - DNA, 100 bp, Homo sapiens
  source 1..100: mol_type = other DNA
ccaaaatgaggtaagtttcctgttttctcagtgagatcttttgttgttgttgttgttgttgttgttttgttgtcgatgttgttgtttttggttttggtct

SEQ ID NO: 201 - DNA, 100 bp, Homo sapiens
  source 1..100: mol_type = other DNA
ccgggtcgtccagccccgggccgccgcggctgcccactacacccacgccaaccgcccgcaagcagcgctgcaggggctccgctgggcgacacgccaggct

SEQ ID NO: 202 - DNA, 100 bp, Homo sapiens
  source 1..100: mol_type = other DNA
ctgtcccacagggtgctggggagcgactgggcggctccgccgcgagcgtctttgaattgcgcgccgctgcaggaaaccaaaaactccctagcaagagggt

SEQ ID NO: 203 - DNA, 100 bp, Homo sapiens
  source 1..100: mol_type = other DNA
ttcaaaaggtttctggaaaccaccgacggttaaacatcacaactggactcggagagagccaaacggtttccccacttgcacctgccagtcttcgcggcgg

SEQ ID NO: 204 - DNA, 100 bp, Homo sapiens
  source 1..100: mol_type = other DNA
cgacctggcagcccaggtgcggtcttaaccgcccccgcccctcaccccgtacccgctcctatccccggagcgcaaatctcagggctggcagctgcgcggt

SEQ ID NO: 205 - DNA, 100 bp, Homo sapiens
  source 1..100: mol_type = other DNA
ggaaggttttccccctcaaacccaaagcgcgcgggcggatcaactcctagctgctgccaccactcgatcccctcagaggatcggcgcggtgggtccaccc

SEQ ID NO: 206 - DNA, 100 bp, Homo sapiens
  source 1..100: mol_type = other DNA
gcctctcccgccctctgcctactgtgctgggagactggcacagctccgtcggccgcacagagtttaacaaacacgcacccagtgtcaagaacagtcacca

SEQ ID NO: 207 - DNA, 100 bp, Homo sapiens
  source 1..100: mol_type = other DNA
ggcgcttaaccccgaagttaaagcgggcgcaatctcctcctgggaactcagcccaggcacgccgccctccgcctctaaattcagacaatgtaactcgctc

SEQ ID NO: 208 - DNA, 100 bp, Homo sapiens
  source 1..100: mol_type = other DNA
caagacatccccgcttccccaaggaagagaccggtggtctgagtcccgaggcagcgcgcacgccttctctgcacttgtgcacagaatgttcttacgtttg

SEQ ID NO: 209 - DNA, 100 bp, Homo sapiens
  source 1..100: mol_type = other DNA
caaacagcgtgcaagccgccgcgcgcggcgggactcaagggggagacacatgcagccactggaacgctctttccagtcgtttctcctcgactcacagaga

SEQ ID NO: 210 - DNA, 100 bp, Homo sapiens
  source 1..100: mol_type = other DNA
aaaagattccaatcctgctccccccccacccacccgcactatataggcatggtcaagaaaactcctttcggtgacccttttttggagtacgggtacctcc

SEQ ID NO: 211 - DNA, 100 bp, Homo sapiens
  source 1..100: mol_type = other DNA
aatgtcctggccgcttctgcccgctcggagaggggctgcgctctaagttcaaacgtttgtacatttatgacaaagcaggttgaaactggacttacactga

SEQ ID NO: 212 - DNA, 100 bp, Homo sapiens
  source 1..100: mol_type = other DNA
tcccctccatggtaaccgctggttctccagatgcggtggctactggagcactcaggccctcggcgtcactttgctacctgctgccgcagccaacaaactg

SEQ ID NO: 213 - DNA, 100 bp, Homo sapiens
  source 1..100: mol_type = other DNA
cccattgctgacatacttactccctgagagtggctcttcatgcacctccaaggggttgctctccggtccatccagtgtcttgctcaccccctgtggtgaa

SEQ ID NO: 214 - DNA, 100 bp, Homo sapiens
  source 1..100: mol_type = other DNA
agttctccaccatctccctctccggagggtgagctgggctgcttggcgaggggcacctcccctctggggcctgagctgggctctgggctttggtttctcc

SEQ ID NO: 215 - DNA, 100 bp, Homo sapiens
  source 1..100: mol_type = other DNA
cagccggagcactgcacacatccccagtccccggtttctcattctccagtgacgcgtgatccccacgtgcgttttttgcatctctggcatcctcggtgct

SEQ ID NO: 216 - DNA, 100 bp, Homo sapiens
  source 1..100: mol_type = other DNA
atttgcaggttatatcctggatggtggcacgacagcgcctggaacacagaaggttgggaggcgtgacgctcatcaggaaggctcttttggggagccagga

SEQ ID NO: 217 - DNA, 100 bp, Homo sapiens
  source 1..100: mol_type = other DNA
agagtcccccagaagcccacttggcaccctatctataacaagttgctctttaagaatcatgggaactccagaatcattttcacaaataccttccactcat

SEQ ID NO: 218 - DNA, 100 bp, Homo sapiens
  source 1..100: mol_type = other DNA
gattcaattaaatggcagaaaacacaaaccttccgttcccactggcaaactgggtctagctaactgagcacagctagcacaaggcaggccccctgctagc

SEQ ID NO: 219 - DNA, 100 bp, Homo sapiens
  source 1..100: mol_type = other DNA
agggcaagtggcggcccggtccccaaggcccaggggagcctctgcagctccctggaaggacggtcaagtgaacagagagctggctgccatctgggttctt

SEQ ID NO: 220 - DNA, 100 bp, Homo sapiens
  source 1..100: mol_type = other DNA
atgagatcaccagtttatcgtaactagaggcctctcccatctaaagcatctttgtaactgctttccctttccccacactgcctacacataaagaagcccc

SEQ ID NO: 221 - DNA, 100 bp, Homo sapiens
  source 1..100: mol_type = other DNA
taatttgtaacaagtcatttgacaactccagaagaggggccacatcctttttctctatgtctgttgattaacaaagacaacattatgtttccaacaccag

SEQ ID NO: 222 - DNA, 100 bp, Homo sapiens
  source 1..100: mol_type = other DNA
tcagaccaagggggaaaaaagtccccatgacttcagtaattttccatcctttggaacaaggaaatatacacaaaaggtttactatagaatgtaagcattg

SEQ ID NO: 223 - DNA, 100 bp, Homo sapiens
  source 1..100: mol_type = other DNA
aactgttcaagattgggctctcacactaacacacctcttccttgcaacttgcacccaatttgactctggtcctaggcatgctgacctgaaatagttgctg

SEQ ID NO: 224 - DNA, 100 bp, Homo sapiens
  source 1..100: mol_type = other DNA
gctgcggcaagcaccacgcggtggcaggagaattcctgaatgtccacacacaagatgacatctgtcagagcgttttccattcgcagggtttccaggccat

SEQ ID NO: 225 - DNA, 100 bp, Homo sapiens
  source 1..100: mol_type = other DNA
tctgaagaattaaggagagtcccgcgtcgtcaaatttgaccttttccccatttaagatctcgaccaagtctcctgttttctgggagggctcatctgtaga

SEQ ID NO: 226 - DNA, 100 bp, Homo sapiens
  source 1..100: mol_type = other DNA
aggtgccaggggcccttccaaactcttctcgaccacatcacccatggtccaggcgcccctttgtcctgccatcaacatcgagactgaaggagcgcccaag

SEQ ID NO: 227 - DNA, 100 bp, Homo sapiens
  source 1..100: mol_type = other DNA
ccttcctgttggccactacatacgtgtcccccgcttcttgcccctctctgcttgggtccctgctacactggtatcctgcactttccaccttgtattgcca

SEQ ID NO: 228 - DNA, 100 bp, Homo sapiens
  source 1..100: mol_type = other DNA
gtttgtttccaaggccatctccactttgagcttgttcatgaccacctcacacagcacacttggtctgtgtggtggtttgaggggttctgtctgtacactg

SEQ ID NO: 229 - DNA, 100 bp, Homo sapiens
  source 1..100: mol_type = other DNA
tgctttggctgtgttggaggcgggcaggtgggaaggaagaaatgtattcttggggagatttgtttttagagacatgagacatggaaaatagttaagtaat

SEQ ID NO: 230 - DNA, 100 bp, Homo sapiens
  source 1..100: mol_type = other DNA
aatataatatgggaggcatggactatcagaggaggcaggcaggactgcccaacctcctcactgggcacgttacgctacttcctcctgacctctatagtcc

SEQ ID NO: 231 - DNA, 100 bp, Homo sapiens
  source 1..100: mol_type = other DNA
ctatcattgccctttcttaccttgatatcctaaaaagctggtggtctgtcttctctatcttttgtcctggtcagttatcctaactattttgtgtctgttt

SEQ ID NO: 232 - DNA, 100 bp, Homo sapiens
  source 1..100: mol_type = other DNA
ctgtggattagtaaacggggtccccacccccactccacaaggagaacatctggcacccagaagtcactgagagaatagctgttgctttggtagaattctg

SEQ ID NO: 233 - DNA, 100 bp, Homo sapiens
  source 1..100: mol_type = other DNA
cctctgagtggcttgttcttttcccagacggagaggtctcctgacagcagctctcttctttttctttttttttttttttgagacagagttttgctcttgc

SEQ ID NO: 234 - DNA, 100 bp, Homo sapiens
  source 1..100: mol_type = other DNA
ctcctgtaccctgtgggcctgagagaggagacaatgggacaagaagacccagtggcttccttggaagcttttgtgctagctggagagagaagacctactt

SEQ ID NO: 235 - DNA, 100 bp, Homo sapiens
  source 1..100: mol_type = other DNA
cctatatgcctagcaacagtccacactgactggactgcaaccaggacatttccagattactcagtggggcttatcttgaaataatagttgatgccatttg

SEQ ID NO: 236 - DNA, 100 bp, Homo sapiens
  source 1..100: mol_type = other DNA
ttaaatatattatatataccatctaagggtcttacatgccttctctcatttgatcttcatggcaaaccctgtgaggtatgaccaccaaccaccattttac

SEQ ID NO: 237 - DNA, 100 bp, Homo sapiens
  source 1..100: mol_type = other DNA
ctcagaactcaggctcccagagtttaagttgctcacaggagcccagaaagtaagcgacagaggtgggatttggttctaggtgtttgccaccagcacttta

SEQ ID NO: 238 - DNA, 100 bp, Homo sapiens
  source 1..100: mol_type = other DNA
aatcaccaaagctttctggaagctccaacttttcttctcaagatactgaaagacaggtatctggatgggttggcagggcgggtgggaggtgggcgagatt

SEQ ID NO: 239 - DNA, 100 bp, Homo sapiens
  source 1..100: mol_type = other DNA
tccatcaacaacgggtctaaaaccagcgatggtgagctgggtgattttgatggaacccctgccatacagtctattaatatcataattggagctaaaattt

SEQ ID NO: 240 - DNA, 100 bp, Homo sapiens
  source 1..100: mol_type = other DNA
aatcatgatggcaatcatgagttctggggcttcttgatttgggccagcagacacagtctcagtcactagttctccgaatcagagaaaggatgccttcagg

SEQ ID NO: 241 - DNA, 100 bp, Homo sapiens
  source 1..100: mol_type = other DNA
ctgtgtcttcacatggcttttcctctgtgcgtggtggaaagagagagctctgcgggtctcttcttgttgtaaggacactggccccattggattagggccc

SEQ ID NO: 242 - DNA, 100 bp, Homo sapiens
  source 1..100: mol_type = other DNA
caccacatgacacatttaatcctaattacctccctcacagccctatttccaaacagggtattagtcacattagggattagggcttcaacataggaattct

SEQ ID NO: 243 - DNA, 100 bp, Homo sapiens
  source 1..100: mol_type = other DNA
gggggcacacaattcagtctataacagagggaaaacagatttgagaagaaaaaagtccaaaatatgcacagtggtaatatctgaagatgtgcgtgcgtgc

SEQ ID NO: 244 - DNA, 100 bp, Homo sapiens
  source 1..100: mol_type = other DNA
tcaagggctcagcaaacgacaacttaagcatttagagtcccatccctatccaccaaacccagaataagttagtcttttcaagaaagcattggtataaaac

SEQ ID NO: 245 - DNA, 100 bp, Homo sapiens
  source 1..100: mol_type = other DNA
ccttcaaaactgaaaagaagaaaggggcaattggagaattcccactttttctggctgtctccttcaagtcgcccagtttttatgaacagcatctagcctt

SEQ ID NO: 246 - DNA, 100 bp, Homo sapiens
  source 1..100: mol_type = other DNA
actgtcactatcaacaacccttaaaactagccaatgcttcggcctctagtattggaaagtcttccaaataggatactggaaacttctatttataagcttg

SEQ ID NO: 247 - DNA, 100 bp, Homo sapiens
  source 1..100: mol_type = other DNA
gggtggcgggcggggcggggaggtggagagagagttgccatctacaggtttctattttggcctgaagactcaactgcagtcattagagtaagggaatgcc

SEQ ID NO: 248 - DNA, 100 bp, Homo sapiens
  source 1..100: mol_type = other DNA
ttatttattaaaaccacacacaccttgcaaagaaaaagggaaactggcagtctctgtagaggaagccggtggcatcgctcagagccacaaactgtatttc

SEQ ID NO: 249 - DNA, 100 bp, Homo sapiens
  source 1..100: mol_type = other DNA
taaacagccctttccctggttccctctctcctgccccactttttttaaaatccagactgtaaaaaacacatctactgacactcactttactttaaaaaaa

SEQ ID NO: 250 - DNA, 100 bp, Homo sapiens
  source 1..100: mol_type = other DNA
gaagagaaaaagtaaagcgttacaagactttcctcctggaaactataaactgaaaaaaaaatccataaaagattaaatcctggcgggttgtggggtggcg

SEQ ID NO: 251 - DNA, 100 bp, Homo sapiens
  source 1..100: mol_type = other DNA
ggggccggcggggagggggcgcggagtggagattggctctctgaggtggtcaggggccctgtgacagcttgggactttcagcacctggtttggggtcatt

SEQ ID NO: 252 - DNA, 100 bp, Homo sapiens
  source 1..100: mol_type = other DNA
tatctgctcaactgtcaggaccccccacccccaaaccccagccaccaacacaaccatcgtagaagggaacacaacacagagggtcttttttcattttttt

SEQ ID NO: 253 - DNA, 100 bp, Homo sapiens
  source 1..100: mol_type = other DNA
tttttaaaaaatcggtttggttgtgtttttgttttccatgggggagctttaaaactcattattgcaacactagttccatttttcgccagggttccaataa

SEQ ID NO: 254 - DNA, 100 bp, Homo sapiens
  source 1..100: mol_type = other DNA
caagacatttaccacggtcactacatccggcagcggggtggcccctagctcctgctgcccccccgccctttctccccgcccgcccccggagctcagccga

SEQ ID NO: 255 - DNA, 100 bp, Homo sapiens
  source 1..100: mol_type = other DNA
tttctgaggctccaactctacccactccctccccgggccgccgccgccgcgccttcccccattcttactccctcgaggagagccacaggttgcaaatcca

SEQ ID NO: 256 - DNA, 100 bp, Homo sapiens
  source 1..100: mol_type = other DNA
accaacctcgcaatctatttttgcaaaatcactcacaaagatctccctttcgcgcccgcgcccgctcctcccgcgccgggtcccctcagccacggccaca

SEQ ID NO: 257 - DNA, 100 bp, Homo sapiens
  source 1..100: mol_type = other DNA
aagtgcccttctctcctcctgagtcttgcacataaggaacgcgggctggggctctgttcgtctttctcctcgcccaaggtaaggacctcgggaatctgaa

SEQ ID NO: 258 - DNA, 100 bp, Homo sapiens
  source 1..100: mol_type = other DNA
gcctggcgtccactacgctcaggcccgcagttccctttttacagagcttgcaccatgggaaaaaataaaataaaatttaggaaagggaggcaacagccat

SEQ ID NO: 259 - DNA, 100 bp, Homo sapiens
  source 1..100: mol_type = other DNA
taaaatttaggaaagggaggcaacagccattgggagccaacacagagtcacgcagcgcccaaaatacaaacaccgcagcggccagaaatcccgccacctt

SEQ ID NO: 260 - DNA, 100 bp, Homo sapiens
  source 1..100: mol_type = other DNA
tctcgttctcccaggctgtcctgtcgaggttccctgagtccccccgcacactgaaaggcatcgcaggtgcagtgcgcacccctttcccacccaccccaag

SEQ ID NO: 261 - DNA, 100 bp, Homo sapiens
  source 1..100: mol_type = other DNA
aagccctgtcccgccatcagtctctctcctcgggatgagcagggagagcgcgcggaggttcccgactccctcgactacaaccaagaaagaataattttca

SEQ ID NO: 262 - DNA, 100 bp, Homo sapiens
  source 1..100: mol_type = other DNA
aagtgttcaacatccccgcccccaagctccccaaaacacaggggcagggaacaccaaaacactcggctctcattaggaagatcacggctctgaaaggaaa

SEQ ID NO: 263 - DNA, 100 bp, Homo sapiens
  source 1..100: mol_type = other DNA
tagtagacacgatacttcatctcatctggatttatgaccaaaaaaacaaaaacaaaaacccaaagagttcgcttgcattttttccttccaaatctcggtt

SEQ ID NO: 264 - DNA, 100 bp, Homo sapiens
  source 1..100: mol_type = other DNA
aacaaaaacccaaagagttcgcttgcattttttccttccaaatctcggttcggctcgaaggcagggaatctaaaagaccgaggccgatggaagagagcca

SEQ ID NO: 265 - DNA, 100 bp, Homo sapiens
  source 1..100: mol_type = other DNA
gcggggcgagcgagcgggcagcctccctttttgcctcccggagttacccagaaggacaggggaagggaaggaagaagaggcgaggaaaaagaggagggag

SEQ ID NO: 266 - DNA, 100 bp, Homo sapiens
  source 1..100: mol_type = other DNA
ggaagcggaggccaggagcgacggagcaaggaaagcagtttgcaagcgagaaaagagggaaaaaacacagccgcacgaatccagagagatcacaagccgt

SEQ ID NO: 267 - DNA, 100 bp, Homo sapiens
  source 1..100: mol_type = other DNA
acgcaagcagcagcagaaagagcgagagcgcgagcgcgcgtcctctccgcggtctggggccagacagcccccagactagcccgaatcaccccccaagcac

SEQ ID NO: 268 - DNA, 100 bp, Homo sapiens
  source 1..100: mol_type = other DNA
tgtctcgtcctctctgctccggccgccccctaattcccctccttcctctcctccacctcctttccaaaaaccaaaacaacacaagggagggtggcaaaag

SEQ ID NO: 269 - DNA, 100 bp, Homo sapiens
  source 1..100: mol_type = other DNA
cctccccaaaccggccgattcactcaaagacaacaataataataataaatacataacaatctatatcctatggtgggagagacgtgggactaatcttcgg

SEQ ID NO: 270 - DNA, 100 bp, Homo sapiens
  source 1..100: mol_type = other DNA
acataacaatctatatcctatggtgggagagacgtgggactaatcttcggcatttattttaacacctgacagctagaataaataaatatatacatttata

SEQ ID NO: 271 - DNA, 100 bp, Homo sapiens
  source 1..100: mol_type = other DNA
aataaatatatacatttatatcaatagatacacatagaaaacttggagccaaagcatttggcaagagcggaaaaaaaaagaattaaaaggtaaaataatg

SEQ ID NO: 272 - DNA, 100 bp, Homo sapiens
  source 1..100: mol_type = other DNA
atcatgagcagcggcggcggcagcggcaccagcggcaacagcggcggcggcggcagtagcagcagcagcggcggcagcaacagcaataatcacctggtgt

SEQ ID NO: 273 - DNA, 100 bp, Homo sapiens
  source 1..100: mol_type = other DNA
ccggcctttcctagaaacttcttgcatcaccacttctaagaaccccagttctaagaatcaacagagctcaattctcggaatttgagcttcggactttacc

SEQ ID NO: 274 - DNA, 100 bp, Homo sapiens
  source 1..100: mol_type = other DNA
actgctacgtggcaggggaggacttggtgtcagctctccgagatttttactgcccctggccaaccaaaagccctcaaagccacaagattttttcactggc

SEQ ID NO: 275 - DNA, 100 bp, Homo sapiens
  source 1..100: mol_type = other DNA
cggcatatttcgaggtcctcataagcagagcgtctcggatttggaggttccggttcgaggctcgaggggcctgaaggtggctctccctccccgggcccaa

SEQ ID NO: 276 - DNA, 100 bp, Homo sapiens
  source 1..100: mol_type = other DNA
gacgatggtatggcctgctccgccaccatcacgtgggctcctcctctgtgacgtcggcgccttcgctgtagcaaagctcggcctctggaattctgagaac

SEQ ID NO: 277 - DNA, 100 bp, Homo sapiens
  source 1..100: mol_type = other DNA
gcacaaaagggagcgagaggtttgaaccactgggaaaagtatgttatatatatagtagggttagagaggcgagtaagagaaaaataaaataaaataaaca

SEQ ID NO: 278 - DNA, 100 bp, Homo sapiens
  source 1..100: mol_type = other DNA
aaaataaaataaacatcacagctctttccaactagaatattaggcaccacgagaaaaatatttgccaagcagttttcggtgggttcatttgctttatttt

SEQ ID NO: 279 - DNA, 100 bp, Homo sapiens
  source 1..100: mol_type = other DNA
tatttaggacaggggtttttgctgttgttctgggtttttttctttctggtgtggtggcttgggatttttggtttctgtattttgatggtttatggatttt

SEQ ID NO: 280 - DNA, 100 bp, Homo sapiens
  source 1..100: mol_type = other DNA
tgcttctgattttttgccttttgcaagtttgtggtgttacgtaaatcacaggatcggcatcggttggatttttttgtacgtgccttttctttccctatct

SEQ ID NO: 281 - DNA, 100 bp, Homo sapiens
  source 1..100: mol_type = other DNA
aatccctcaagcgttttaaagatgtattatttcaatactaatactattgaaagaagcttaaatttttggccatatgtaacaatcccagcccccacttttt

SEQ ID NO: 282 - DNA, 100 bp, Homo sapiens
  source 1..100: mol_type = other DNA
attatcatcatcaccaccaacatcctctgccctggagaccaagagaattcaaacaggtcagcacctctaattgctgtatagaacattgaccctactgtct

SEQ ID NO: 283 - DNA, 100 bp, Homo sapiens
  source 1..100: mol_type = other DNA
cccagttcctgaggatggtgtgataataatacatctcagagttctgtagtttcttcaccactgtgcaggtgtggttggtgggagcaatgccctggatgga

SEQ ID NO: 284 - DNA, 100 bp, Homo sapiens
  source 1..100: mol_type = other DNA
taagccaagctcttgtgtcctggcagataaacaaggtgaaccctcaatccgtgtagcaggagtttccagacaaactcactttgcatggaaggacactaac

SEQ ID NO: 285 - DNA, 100 bp, Homo sapiens
  source 1..100: mol_type = other DNA
ccttccaggtgcatggaaatattttgtagtttttactgtctcccccttcctccactgcctcatcttttttgttttttcccctgtgagactatttgctctg

SEQ ID NO: 286 - DNA, 100 bp, Homo sapiens
  source 1..100: mol_type = other DNA
cctttccaacactggcctgccttagggactcaccgtctgcactccgcctgcacaggtggaactgagttcagatgagggagaattgctttccattgttcag

SEQ ID NO: 287 - DNA, 100 bp, Homo sapiens
  source 1..100: mol_type = other DNA
taggctttttgtaatttctagttttgcttacctttcctactcaccacacacacaaaacagtgtgagctttctcattctagtgcataaacacaggtcggtc

SEQ ID NO: 288 - DNA, 100 bp, Homo sapiens
  source 1..100: mol_type = other DNA
aatacccacaagtgttccaaaaggtgagctggcattgctgcccaactgggcattatagtcccttctgtccctgcccatcaggcttgccttcctcggcaac

SEQ ID NO: 289 - DNA, 100 bp, Homo sapiens
  source 1..100: mol_type = other DNA
ctttctagcttgaattgtactgtgactccttctcacggaccactcccggagactggtgaaagttgggcccattcttgaagcctctgcttctaaatcatgt

SEQ ID NO: 290 - DNA, 100 bp, Homo sapiens
  source 1..100: mol_type = other DNA
tttccataaagtctccctcatcgtgcttgcttccaccttctcctatttggaattactggtgggctcttccactgtcccatagcaagtgttctatacattc

SEQ ID NO: 291 - DNA, 100 bp, Homo sapiens
  source 1..100: mol_type = other DNA
tgaaggcacatttgaatatatactttgtcatggttgcttggaaccatgtcgtcttttccaagtaggctgtgaacattcagtggcatggatcataccgtgc

SEQ ID NO: 292 - DNA, 100 bp, Homo sapiens
  source 1..100: mol_type = other DNA
cccattgttcaaagaaaggcattatggagtctccaaaagccattggcaggtggtgtctgtgacttccttagcctggaaataaacaaataaacaagcacaa

SEQ ID NO: 293 - DNA, 100 bp, Homo sapiens
  source 1..100: mol_type = other DNA
aaacaaataaacaagcacaaattagaagtctttgccctattactgcactattagtattgattgcgcaacatcatgcaaaaagtcactttaatttatctgg

SEQ ID NO: 294 - DNA, 100 bp, Homo sapiens
  source 1..100: mol_type = other DNA
caggtcctatgtaaacaccaatacagtcaagagggcttggatgggtatttgctttcatttctaatgaaatttcaggcctctagggtaggatatcaaaatt

SEQ ID NO: 295 - DNA, 100 bp, Homo sapiens
  source 1..100: mol_type = other DNA
ggtagatcatttgcaatttattttatcccaaacacctcactttacagtcagagaaactgaggcccagagaagtaaaatgagttgctcaaggtctcagaga

SEQ ID NO: 296 - DNA, 100 bp, Homo sapiens
  source 1..100: mol_type = other DNA
actgaggcccagagaagtaaaatgagttgctcaaggtctcagagagcaagaaatagagatgggacttgagcacctagatctctggtattgctgtcctgta

SEQ ID NO: 297 - DNA, 100 bp, Homo sapiens
  source 1..100: mol_type = other DNA
gttcatggagctggcagatggatacatctgtgacctgggatgatggagagactgctggacccttcagaggatctcatctcaaggtggggtttatgtgtaa

SEQ ID NO: 298 - DNA, 100 bp, Homo sapiens
  source 1..100: mol_type = other DNA
atgatatctgtgtgtttcattttcctttcataaactaatttaaaaatccttttggtatcaaattttaagccaaaaagtagtgagggggaacatgggtagg

SEQ ID NO: 299 - DNA, 100 bp, Homo sapiens
  source 1..100: mol_type = other DNA
aatagcttacagcttgcctaacaaggttgttgactgcataagagtcaggagttttgggtaagagtgtgtgtgtgtgtgtgtgtgtgtgtgtgtgtgtgag

SEQ ID NO: 300 - DNA, 100 bp, Homo sapiens
  source 1..100: mol_type = other DNA
cgtactgaatttgactgctttattttgtagggaaggaaactgatgtgcctagagtagttgagagctttattcaaactcattccactgttattgagtagtt

SEQ ID NO: 301 - DNA, 100 bp, Homo sapiens
  source 1..100: mol_type = other DNA
aggatattagaccagcaacatatttgggtagaaactttcatataaaaaagcgtaatcataactatccaatcatgtcaactagtaaggctgctcaggtggg

SEQ ID NO: 302 - DNA, 100 bp, Homo sapiens
  source 1..100: mol_type = other DNA
ataacacatcaaccttctttgggattcttccctcagacatggttttggtgggaggagcatggcaagggaggggcgagctccaaatgcagggctgctctgt

SEQ ID NO: 303 - DNA, 100 bp, Homo sapiens
  source 1..100: mol_type = other DNA
cctcggcgacctgagcagacacacgagcagagatcagagacactcttagtgaatgaacctccctattggctatattaaagtaatgctctgaaaaagttcc

SEQ ID NO: 304 - DNA, 100 bp, Homo sapiens
  source 1..100: mol_type = other DNA
tatgtatgcatagtctaaagtgatgattttagaggtagcaagacagtgagaatgtccctacatgtgaaatgggcacagttttatcagggaagtgtcaata

SEQ ID NO: 305 - DNA, 100 bp, Homo sapiens
  source 1..100: mol_type = other DNA
gagggttaatgttccacgtagtggctgcaagaatgataagtggtcatggggatagcctgacactctaggagcagaaggtggtgggtatggatagaactac

SEQ ID NO: 306 - DNA, 100 bp, Homo sapiens
  source 1..100: mol_type = other DNA
tgatatagcatgaatccaacctgctgttatctgcgcaggcctctctgcagctgtttgccctgaagtacatgctgtacgtttctccagctgatcctgcatg

SEQ ID NO: 307 - DNA, 100 bp, Homo sapiens
  source 1..100: mol_type = other DNA
actgggtataaacgcctgtccgctgtgtgctggacagccccagacaccctcggcagcctgctgtgtttgtgtgagacatgctgtgttagggatttaagca

SEQ ID NO: 308 - DNA, 100 bp, Homo sapiens
  source 1..100: mol_type = other DNA
acagctttctcatctacatggacaacctatttttaaagaatcttcagagagtcgttgactttgttataactactactatatacgtaatttcagatgatag

SEQ ID NO: 309 - DNA, 100 bp, Homo sapiens
  source 1..100: mol_type = other DNA
aattgaaaatttaacttgtttttctagaaagagtttattttccctataacttcaaagagtaatggtggggagtaggacattctgaaaataagaagaaaca

SEQ ID NO: 310 - DNA, 100 bp, Homo sapiens
  source 1..100: mol_type = other DNA
tgtcaaatgaatttctgacttccagctaggcatatggaataaaggtctttattccagtgacctctgctcattggaaaactttgggctggtagatttcatg

SEQ ID NO: 311 - DNA, 100 bp, Homo sapiens
  source 1..100: mol_type = other DNA
tctcttgcattcttaacttgcaatttagtactgtttatattctgcttgaaggttagagacattcgactaaatggtcttttctccacattgctgtcattca

SEQ ID NO: 312 - DNA, 100 bp, Homo sapiens
  source 1..100: mol_type = other DNA
ttaatgtcctggtcctggactttactcattgaccacaggacaagtggctcaactctctcctgccactacccaggctgttagtcctgttgggaggctcagg

SEQ ID NO: 313 - DNA, 100 bp, Homo sapiens
  source 1..100: mol_type = other DNA
gcccaactcactcatctgtaactctcatctccattcagctgcagcctctacagcccctggttataccctggatcttatcattgcttcgctctattttacc

SEQ ID NO: 314 - DNA, 100 bp, Homo sapiens
  source 1..100: mol_type = other DNA
tcctaaatcgtaaaaattaaaaccagcctcggaacacaacccctcattcttccagcactctctctcattcaggtaactcctattctacttttcttcagca

SEQ ID NO: 315 - DNA, 100 bp, Homo sapiens
  source 1..100: mol_type = other DNA
ttgtttttttttactttaccttaatttctctttttggactaagatgttaaaatgtttcttaatgtgactgtctccgaaactgttttgtgtctaccactca

SEQ ID NO: 316 - DNA, 100 bp, Homo sapiens
  source 1..100: mol_type = other DNA
tcctagtggcagtcattgatccttttcttgttgcgagtgtttgagtgtgggtgtgtgtgagtgtgtatatgtatttgtagagggaaaaacaagagagagg

SEQ ID NO: 317 - DNA, 100 bp, Homo sapiens
  source 1..100: mol_type = other DNA
tgtgagtgtgtatatgtatttgtagagggaaaaacaagagagagggaaacagacattggagccacctttcccccactagccacgtacctgttgaaccttc

SEQ ID NO: 318 - DNA, 100 bp, Homo sapiens
  source 1..100: mol_type = other DNA
aagcctctctatagaatcagatatacacaagcacagtgacagaactacatgtgtcctacagtccagcttttaagatatgataaaaactcttgtattcaca

SEQ ID NO: 319 - DNA, 100 bp, Homo sapiens
  source 1..100: mol_type = other DNA
gagctaaatggcaataaccataggagattgcatattgctacattatgtaaagacagagtcccaagaaaatagtgagaactcagtttgatgtatgatgtga

SEQ ID NO: 320 - DNA, 100 bp, Homo sapiens
  source 1..100: mol_type = other DNA
tatgtgatatcttactttacatggctaacagttgacattctttgtggattctatattgtctaaggctacagaagagccatatgataaattcatcggcaac

SEQ ID NO: 321 - DNA, 100 bp, Homo sapiens
  source 1..100: mol_type = other DNA
cagtgaaaaggcttgggccgcttttgttttcacctgcttttgttgaacaaatttgatttccggagtcagtcattttactgtcaagacatttcttcggcat

SEQ ID NO: 322 - DNA, 100 bp, Homo sapiens
  source 1..100: mol_type = other DNA
tctgcaacaggtaaggattttgcttccttaaaagtatttctttggtgtcaaaagaaatttttctaattttatttagcttttactctaggccaaacatcgt

SEQ ID NO: 323 - DNA, 100 bp, Homo sapiens
  source 1..100: mol_type = other DNA
aatgactctgagctacctgctgtaaggtgtagaatcaatttacagggggacgggggtcgggggggtgagtgttgctttgatattcactgcccctcaccac

SEQ ID NO: 324 - DNA, 100 bp, Homo sapiens
  source 1..100: mol_type = other DNA
agtcctaacaagatttttgaaacatgaaaagttacaatagttggctttttggttttccagatattctagagaatgcatatgcttgtgactgtggctgagc

SEQ ID NO: 325 - DNA, 100 bp, Homo sapiens
  source 1..100: mol_type = other DNA
tcaactgtatgggtagtttaaatactacccaaggtttgatgaagtaaatctaaagatgctctaagttgtgcaaatatgaattttaaagttgtctagttca

SEQ ID NO: 326 - DNA, 100 bp, Homo sapiens
  source 1..100: mol_type = other DNA
gaaaagaaacagaaccgaagtctaaatgatgtagatttcaatctggaatttctagcttgtgtttttcacctattgccaatgttaatgaccatttcccaaa

SEQ ID NO: 327 - DNA, 100 bp, Homo sapiens
  source 1..100: mol_type = other DNA
agtgctctatgatgtataacatgtattttttaattaaatttaatctttcttctgaggtggtttgatttggagatatgctacgaggtaccagtcagtagcc

SEQ ID NO: 328 - DNA, 100 bp, Homo sapiens
  source 1..100: mol_type = other DNA
tgagttgtaactaaacaaagtttgggaaatcaccggttttaggtgctttactaaatgaaagttgccattgacgtattcaagcaggcaacaagtagttggt

SEQ ID NO: 329 - DNA, 100 bp, Homo sapiens
  source 1..100: mol_type = other DNA
gtccccttattggttctaagctggtgccgtggaggatataagagaaatattttaaaaatctctactttgaaggaccctataatctggtagttgtgataag

SEQ ID NO: 330 - DNA, 100 bp, Homo sapiens
  source 1..100: mol_type = other DNA
tttaaaaatctctactttgaaggaccctataatctggtagttgtgataagaagtaaaatttaggaagcaatgcaagatgagaattcagtgatgagtgggg

SEQ ID NO: 331 - DNA, 100 bp, Homo sapiens
  source 1..100: mol_type = other DNA
cagcacaggcttgaagagttctgtgaattccatggagggggcctgggggcaaactggagttgtcaggaagatctgggctttggaagaatgcgaagtgtcg

SEQ ID NO: 332 - DNA, 100 bp, Homo sapiens
  source 1..100: mol_type = other DNA
gtagaaggagaaggggcaggtgatttcagactgggaggaccttgtgggcaaaggcacaaaggcgagactgacctggagatgataaggccagttgaagaga

SEQ ID NO: 333 - DNA, 100 bp, Homo sapiens
  source 1..100: mol_type = other DNA
acattgcaggaaatcagattagacagttagggtgtggacacaaaagcgaggaccttgcaggcactggggagaagtgaccccattcaatagtccttggtct

SEQ ID NO: 334 - DNA, 100 bp, Homo sapiens
  source 1..100: mol_type = other DNA
ccttctgccctgcggctgcgcttcctcggctctcacggcaccagcagaattccatgtgagagggagcttgtcgagcgtggcctcttcccacttggggctg

SEQ ID NO: 335 - DNA, 100 bp, Homo sapiens
  source 1..100: mol_type = other DNA
ctttctgcatccctgtgcctggctgtgggcctccatttgccctctactgtcttcccttaggacatcatttatgcagagaaaggttcgtgtggctcggggt

SEQ ID NO: 336 - DNA, 100 bp, Homo sapiens
  source 1..100: mol_type = other DNA
ggacgttgtttagagagtcagtagatcataataattcagacactttttttctggaccataaaatatctgaacccatataataacaaacatacagcacggt

SEQ ID NO: 337 - DNA, 100 bp, Homo sapiens
  source 1..100: mol_type = other DNA
gaataagaacccaacttttgagccagatcactttgcatggaatccccattctatcattctatcatttctgggctgtgggaacctcagacaagttacttaa

SEQ ID NO: 338 - DNA, 100 bp, Homo sapiens
  source 1..100: mol_type = other DNA
cttcttcaatgctcagattaaaaaaaaaattcacaaaatatctctaataacagtaataataactgaaaatacctacctcagagggttgtcgtagagatca

SEQ ID NO: 339 - DNA, 100 bp, Homo sapiens
  source 1..100: mol_type = other DNA
aaaattcacaaaatatctctaataacagtaataataactgaaaatacctacctcagagggttgtcgtagagatcaaatgagataaaaatatgtaaagcat

SEQ ID NO: 340 - DNA, 100 bp, Homo sapiens
  source 1..100: mol_type = other DNA
gtagcctagtgcctgactgaaaaaaaaatctctcaatagatgcaactcttatgattcttattaaggacttggctattgccacaaatgaaggtgttatgag

SEQ ID NO: 341 - DNA, 100 bp, Homo sapiens
  source 1..100: mol_type = other DNA
ccctggcttaagagcaagaagcctgcaaagctaactctcctaatcccaacattcctttccagggaaagtagggtgacaggtggaggctgggaattaacgt

SEQ ID NO: 342 - DNA, 100 bp, Homo sapiens
  source 1..100: mol_type = other DNA
tttttgagcaccaaatatggacaaggcacaggggttgggtgtttttctagtgagaatacatatgaaagaaggaaaacaaacttggaaaccgctattttaa

SEQ ID NO: 343 - DNA, 100 bp, Homo sapiens
  source 1..100: mol_type = other DNA
gccatttggtaacagtttctctagcttatgagatgagagaggtcctctcagtatccgctgcattacttgtgggcctccttggttgacgtcgctctctgaa

SEQ ID NO: 344 - DNA, 100 bp, Homo sapiens
  source 1..100: mol_type = other DNA
cgcttggggtggaattctagaggtgcttttcattagaggcagagagcatgacctttcttccttgcccagtttaaattaaattattttatcttacaatgtg

SEQ ID NO: 345 - DNA, 100 bp, Homo sapiens
  source 1..100: mol_type = other DNA
ttaattttagtgctagcaaggcacagctaaaattccatttctacttaggagtggggatcattgtggcagtgagtgcttatttgggtttgggatgcttgga

SEQ ID NO: 346 - DNA, 100 bp, Homo sapiens
  source 1..100: mol_type = other DNA
tctgggtgaaagccaggattaaaaagcatcctccttccccattccactctctaggttataaatatttttttggattaaaagcctcctttaaaaaaatgca

SEQ ID NO: 347 - DNA, 100 bp, Homo sapiens
  source 1..100: mol_type = other DNA
aatccacctggcatgttaattgtgcaggggattcctaattatgtgtgcagatgacgtgagtcacacggtgatagtgttccttctagagtcccactggtgt

SEQ ID NO: 348 - DNA, 100 bp, Homo sapiens
  source 1..100: mol_type = other DNA
actaggcgttcatcctgtgtaatttgaaaatatgtcacacgtggtgatgagaatctatttgaggaacatgggcagtttgaaataatatatgcaatgtatg

SEQ ID NO: 349 - DNA, 100 bp, Homo sapiens
  source 1..100: mol_type = other DNA
actagtttatataatgaaaggaagtatttaaaaagatagaatgacatagactaatctaattgagaaatatgaaagtctaacagaaatgattgcttgtgaa

SEQ ID NO: 350 - DNA, 100 bp, Homo sapiens
  source 1..100: mol_type = other DNA
attttatgaagaaatccacagataaattctccaccttgatctatgtaatccgaaatttagatgttaaaaatatgttgattctgaaaatttatatttattc

SEQ ID NO: 351 - DNA, 100 bp, Homo sapiens
  source 1..100: mol_type = other DNA
tttggtatgaataggtcaaaacaagtcaccattaactgacaggaagcacagaattctcaatttagttttggcaaagacattattttataaatatgagttt

SEQ ID NO: 352 - DNA, 100 bp, Homo sapiens
  source 1..100: mol_type = other DNA
ttaaatgattcttatgaagaaactagcaccaaagtgaatgcactctgcaaataactcccagcttctctgaatttcaaaagcagccactaaatattattag

SEQ ID NO: 353 - DNA, 100 bp, Homo sapiens
  source 1..100: mol_type = other DNA
caaatcaatttagctgaaagcgatgaattacagaagtaaatctttaggtacaaagtagacagctgacacacatgtagcatatacacactagtgatctgcc

SEQ ID NO: 354 - DNA, 100 bp, Homo sapiens
  source 1..100: mol_type = other DNA
ttccttctttaccaacatagagtttcccatgagccctgaatccggggcacttttgctaacttcccctgcagcggcgacgctgccactcccagtgcccccg

SEQ ID NO: 355 - DNA, 100 bp, Homo sapiens
  source 1..100: mol_type = other DNA
cagtggaaggggctcgcgccacctccattgctcttggccccaaagccatagaggtgccccccggaaggggcctggctgccactgccattctggtggccct

SEQ ID NO: 356 - DNA, 100 bp, Homo sapiens
  source 1..100: mol_type = other DNA
gaagcaggtcgtgcttgtccttcctggatttccccgcatccttatcccgcttggcgcctcggctgctctggcttttacctggcttctcctctttgctttt

SEQ ID NO: 357 - DNA, 100 bp, Homo sapiens
  source 1..100: mol_type = other DNA
cccacaggagcctgcccccgcggtggcggcagaggtgctggtgctggtactattgctgtttgggttgccgctgccgccgctgctcacactttgacccagc

SEQ ID NO: 358 - DNA, 100 bp, Homo sapiens
  source 1..100: mol_type = other DNA
gctgaattcatgccagttgcctctccagggcgcccttggacttcctgcctcttgccagtgctgctgatctcgggaatcccatacaaggcagcagaaggca

SEQ ID NO: 359 - DNA, 100 bp, Homo sapiens
  source 1..100: mol_type = other DNA
gagatttattagcatccttagaagttttactccttttcacttttgatttgctggtctctttgtgtgaattcccctggggagcagaggcctgaacagaagc

SEQ ID NO: 360 - DNA, 100 bp, Homo sapiens
  source 1..100: mol_type = other DNA
aaattttaggccatcagctaaggctgcggtagcaccagccccactggaggccggacctccacaatccttggagttgctgctactagtggtggtggtggaa

SEQ ID NO: 361 - DNA, 100 bp, Homo sapiens
  source 1..100: mol_type = other DNA
ttattcatctcaaatttctgtctgtccttctccaaatcagcgtccaaatcaattattaaatttccaaccccgatttcccaatcatcgccactgtcataag

SEQ ID NO: 362 - DNA, 100 bp, Homo sapiens
  source 1..100: mol_type = other DNA
tatcaactgtatttggatccacaccttttcctgcagtagaaatgttcactgacatcctgaagatgagctctctagaataaaaatccgatgaacttttctt

SEQ ID NO: 363 - DNA, 100 bp, Homo sapiens
  source 1..100: mol_type = other DNA
ttcctcaggaatttgagctggggatctgcatcctggccattgcagtcctttagcatcctcgccgcgccctgagcgcgctggaggctcgcaggctgcgccc

SEQ ID NO: 364 - DNA, 100 bp, Homo sapiens
  source 1..100: mol_type = other DNA
tcccagggctgatgccgcgtcctgctccgccgttctgggacgtcggggacaaaagtggaggagacgggagagcccgggcagaaaaagcaggacgcgcgtc

SEQ ID NO: 365 - DNA, 100 bp, Homo sapiens
  source 1..100: mol_type = other DNA
ccaggtgcccacctcttcgctttgaggcgggggcggtgggatggaatatgggtgcgcgaggtcggggctggtaactctcggaggggcacggcctccacgc

SEQ ID NO: 366 - DNA, 100 bp, Homo sapiens
  source 1..100: mol_type = other DNA
tgggagggatgaatggacgctgggccccggcaaatgaggcgctgtgggtccccaggaagtggggtaccaggctctactcccaccccggcctctgaaacgc

SEQ ID NO: 367 - DNA, 100 bp, Homo sapiens
  source 1..100: mol_type = other DNA
ggccaggaggggtggcggctgggtggggagagagggtgcaagacgagcggcgcgtgtcgggagcctttgggctgcgggtgcgttacaggagagcaggcgg

SEQ ID NO: 368 - DNA, 100 bp, Homo sapiens
  source 1..100: mol_type = other DNA
gtaggagccttcgcgggggccgagctcggaaggcggacggctgtgcccgcccaggggatgcgcccgggccggccgcgaaggtgccttcttccgggggccc

SEQ ID NO: 369 - DNA, 100 bp, Homo sapiens
  source 1..100: mol_type = other DNA
ggacgaccctgacacggcacgcgcgcgcttcgcagcctcaaagactccggggcctcgtggtcactggcgcaggggatcggggcggggtgcccggagtgcg

SEQ ID NO: 370 - DNA, 100 bp, Homo sapiens
  source 1..100: mol_type = other DNA
cccgcagtgcagagcagagcgggcggaggaccccgggcgcgggcgcggacggcacgcggggcatgaacctggagggcggcggccgaggcggagagttcgg

SEQ ID NO: 371 - DNA, 100 bp, Homo sapiens
  source 1..100: mol_type = other DNA
catgagcgcggtgagctgcggcaacgggaagctccgccagtggctgatcgaccagatcgacagcggcaagtaccccgggctggtgtgggagaacgaggag

SEQ ID NO: 372 - DNA, 100 bp, Homo sapiens
  source 1..100: mol_type = other DNA
aagagcatcttccgcatcccctggaagcacgcgggcaagcaggactacaaccgcgaggaggacgccgcgctcttcaaggtctccggcctcgggagccggc

SEQ ID NO: 373 - DNA, 100 bp, Homo sapiens
  source 1..100: mol_type = other DNA
cccgcgcgccacagctctgcagctcgtggcagcggcgcagcgctccagccatgtcgcgcggcctccagcttctgctcctgagctgcggtagggctcgcga

SEQ ID NO: 374 - DNA, 100 bp, Homo sapiens
  source 1..100: mol_type = other DNA
gcgcctgtctcgcctgtcgccccccgcccctccacgacaccccctcccgtcggtcgcttgctcacgacgcgctctctctttcttgtagcctacagcctgg

SEQ ID NO: 375 - DNA, 100 bp, Homo sapiens
  source 1..100: mol_type = other DNA
ctcccgcgacgccggaggtgaaggtggcttgctccgaagatgtggacttgccctgcaccgccccctgggatccgcaggttccctacacggtctcctgggt

SEQ ID NO: 376 - DNA, 100 bp, Homo sapiens
  source 1..100: mol_type = other DNA
caaggtaggtgctgcgatacccacgggctggggtttggtgggctcatttgaagacagcaggaaccatctcccctaggctggcgaccctctgtggctgcca

SEQ ID NO: 377 - DNA, 100 bp, Homo sapiens
  source 1..100: mol_type = other DNA
ggtgggggcgaggggcgtctcccgcagctgaacttggagtacccagcctcccgtcgcgcctcccccaccccatccgcatccaggtacagggccgaattag

SEQ ID NO: 378 - DNA, 100 bp, Homo sapiens
  source 1..100: mol_type = other DNA
gttttgctctccgcagacctcaatccccttcctgtcactgaaggtggcctgagatgaatgatccacttaagatgttttggaagggcagagactctcattt

SEQ ID NO: 379 - DNA, 100 bp, Homo sapiens
  source 1..100: mol_type = other DNA
ggattaattctggaggccacctgtggttgtgggccagcaggtcaggaagaaagcaacagggacctagatttgggcattggacagggggaatgtctccaga

SEQ ID NO: 380 - DNA, 100 bp, Homo sapiens
  source 1..100: mol_type = other DNA
ctctccagttcctatattctaatacccctccgccgccaaataaaatttggcgtctggccacagctcttttagtgggtatctgggtggctcttaaaagagc

SEQ ID NO: 381 - DNA, 100 bp, Homo sapiens
  source 1..100: mol_type = other DNA
ctttggggttaggtgttaagacgcttacttggaatgtttacttggagctggtgtacttggtgacggccttggtgccctccgacacggcgtgcttggccag

SEQ ID NO: 382 - DNA, 100 bp, Homo sapiens
  source 1..100: mol_type = other DNA
ctccggcccctgccgagaagactcccgtgaagaagaaggcccgcaagtctgcaggtgcggccaagcgcaaagcgtctgggcccccggtgtccgagctcat

SEQ ID NO: 383 - DNA, 100 bp, Homo sapiens
  source 1..100: mol_type = other DNA
tactaaagctgttgccgcctccaaggagcgcagcggcgtatctttggccgctctcaagaaagcgctggcagccgctggctatgacgtggagaagaacaac

SEQ ID NO: 384 - DNA, 100 bp, Homo sapiens
  source 1..100: mol_type = other DNA
agccgcatcaagctgggtctcaagagcctggtgagcaagggcaccctggtgcagaccaagggcaccggcgcgtcgggttccttcaaactcaacaagaagg

SEQ ID NO: 385 - DNA, 100 bp, Homo sapiens
  source 1..100: mol_type = other DNA
cggcctctggggaagccaagcctaaggctaaaaaggcaggcgcggccaaggccaagaagccagcaggagcggcgaagaagcccaagaaggcgacgggggc

SEQ ID NO: 386 - DNA, 100 bp, Homo sapiens
  source 1..100: mol_type = other DNA
ggccacccccaagaagagcgccaagaagaccccaaagaaggcgaagaagccggctgcagctgctggagccaaaaaagcgaaaagcccgaaaaaggcgaaa

SEQ ID NO: 387 - DNA, 100 bp, Homo sapiens
  source 1..100: mol_type = other DNA
gcagccaagccaaaaaaggcgcccaagagcccagcgaaggccaaagcagttaaacccaaggcggctaaaccaaagaccgccaagcccaaggcagccaagc

SEQ ID NO: 388 - DNA, 100 bp, Homo sapiens
  source 1..100: mol_type = other DNA
caaagaaggcggcagccaagaaaaagtagaaagttcctttggccaactgcttagaagcccaacacaacccaaaggctcttttcagagccacccaccgctc

SEQ ID NO: 389 - DNA, 100 bp, Homo sapiens
  source 1..100: mol_type = other DNA
tcagtaaaagagctgttgcactattagggggcgtggctcgggaaaacgctgctaagcaggggcgggtctcccgggaacaaagtcggggagaggagtggga

SEQ ID NO: 390 - DNA, 100 bp, Homo sapiens
  source 1..100: mol_type = other DNA
ctccttagccagactcgattacaagcactgcatgcattactcagtgtgataagatcatgataatccctttaaaaagatcgcccgaatttaagcctggatt

SEQ ID NO: 391 - DNA, 100 bp, Homo sapiens
  source 1..100: mol_type = other DNA
aggaacacgtgtttacagctctaatatcgataatttaagtggctcttaaaagagcctttggggttgggctttaagacgcttacttggcaagtttacttag

SEQ ID NO: 392 - DNA, 100 bp, Homo sapiens
  source 1..100: mol_type = other DNA
cgctggtgtacttggtgacggccttggtgccctcggacacggcgtgcttggccaactccccgggcagcagcaggcgcacggccgtctggatctccctgga

SEQ ID NO: 393 - DNA, 100 bp, Homo sapiens
  source 1..100: mol_type = other DNA
ccccggctccggctcctgcggcagctcctctgggcaccgtccctgcgccgacatcctggaggttgggatgctcttgtccaaaatcaactcgcttgcccac

SEQ ID NO: 394 - DNA, 100 bp, Homo sapiens
  source 1..100: mol_type = other DNA
ctgcgcgccgcgccctgcaacgacctgcacgccaccaagctggcgcccggtgagagcaccccccgcctccggcccggggatgcggggcggcggcgggatc

SEQ ID NO: 395 - DNA, 100 bp, Homo sapiens
  source 1..100: mol_type = other DNA
tcctgggtggggagctggcggctcgcgggccggcactgagtccccgtgcttccccctttcctaggcaaggagaaggagcccctggagtcgcagtaccagg

SEQ ID NO: 396 - DNA, 100 bp, Homo sapiens
  source 1..100: mol_type = other DNA
tgggcccgctactgggcagcggcggcttcggctcggtctactcaggcatccgcgtctccgacaacttgccggtgagtgggcgccccgcggtggggagggc

SEQ ID NO: 397 - DNA, 100 bp, Homo sapiens
  source 1..100: mol_type = other DNA
gcgccgggcggggggcgcacgggcgtgctttagcccggacgagggaacctgacggagaccctgggcttccaggtggccatcaaacacgtggagaaggacc

SEQ ID NO: 398 - DNA, 100 bp, Homo sapiens
  source 1..100: mol_type = other DNA
ggatttccgactggggagagctggtgagtgccctgcaggagcgacccccaggatgagtgggtggggtgaggggcgcccccgactcccgccctaacgcggc

SEQ ID NO: 399 - DNA, 100 bp, Homo sapiens
  source 1..100: mol_type = other DNA
cccctcgcccctgcagcctaatggcactcgagtgcccatggaagtggtcctgctgaagaaggtgagctcgggtttctccggcgtcattaggctcctggac

SEQ ID NO: 400 - DNA, 100 bp, Homo sapiens
  source 1..100: mol_type = other DNA
tggttcgagaggcccgacagtttcgtcctgatcctggagaggcccgagccggtgcaagatctcttcgacttcatcacggaaaggggagccctgcaagagg

SEQ ID NO: 401 - DNA, 100 bp, Homo sapiens
  source 1..100: mol_type = other DNA
agctggcccgcagcttcttctggcaggtgctggaggccgtgcggcactgccacaactgcggggtgctccaccgcgacatcaaggacgaaaacatccttat

SEQ ID NO: 402 - DNA, 100 bp, Homo sapiens
  source 1..100: mol_type = other DNA
cgacctcaatcgcggcgagctcaagctcatcgacttcgggtcgggggcgctgctcaaggacaccgtctacacggacttcgatggtgagccaggcccggga

SEQ ID NO: 403 - DNA, 100 bp, Homo sapiens
  source 1..100: mol_type = other DNA
gggagctgcccaggtgactcggcccggcccggcccagtccggaggcctcggccagtctcccgcgccagccttttgtaaaggtcattgggccgcctggctc

SEQ ID NO: 404 - DNA, 100 bp, Homo sapiens
  source 1..100: mol_type = other DNA
gatgctagccggggtgggacgcaggagagcctcccagcgtagtaaagccggggattttcagccagctgaacctgtaatgtttctggcatgattttattct

SEQ ID NO: 405 - DNA, 100 bp, Homo sapiens
  source 1..100: mol_type = other DNA
tcaagtggaattcagttagttccaggctttcccgatgaataagaggttgtgggcaaccggcggtagcccagatttttctaaagtctgacccagtttcccc

SEQ ID NO: 406 - DNA, 100 bp, Homo sapiens
  source 1..100: mol_type = other DNA
ctctaaacagacaaaagcaaaatatctcattaggcatcatctccgccaaggttcccactaggcaggaaaggatttttatctaaagtaattacccttttta

SEQ ID NO: 407 - DNA, 100 bp, Homo sapiens
  source 1..100: mol_type = other DNA
gttaaatacactcaacagatgaaatttacagagagtgagagactgcagcactagacagcgaaggtgaaaaccaggaacgccgcgtctcgccgcccgcggg

SEQ ID NO: 408 - DNA, 100 bp, Homo sapiens
  source 1..100: mol_type = other DNA
cccgccgggagactgcgggtccgtctcgcgggtggggcgccccggtccctctcgtttcctggaggccacaggtcacggcgacggcggtgaccgggagagc

SEQ ID NO: 409 - DNA, 100 bp, Homo sapiens
  source 1..100: mol_type = other DNA
cgggtctgacagctgctgcggctcgcgcggacgcgcgcctcctgcagcccgccctccccatgcctgacttattactctctgctcctcctccctctgctgt

SEQ ID NO: 410 - DNA, 100 bp, Homo sapiens
  source 1..100: mol_type = other DNA
tccaaaacacccttcgacgccagcaaaatacaatgcgcctcggccgccgtaaacagccgggagggagagcacacattcggcgcggcgcggccgccggctc

SEQ ID NO: 411 - DNA, 100 bp, Homo sapiens
  source 1..100: mol_type = other DNA
ggctcccacccccttcccgttcctagaaaatgccataaaagcgggcagggcgcggggagggcggctgcgcgcccggcggccggggctcccttcccgcgcc

SEQ ID NO: 412 - DNA, 100 bp, Homo sapiens
  source 1..100: mol_type = other DNA
tatgaaacagccagtgctacgtctcctttataccaaaactggtagcctgaagagctctcaggcttacctataaacgatgttcagtgaatgcaggtagccc

SEQ ID NO: 413 - DNA, 100 bp, Homo sapiens
  source 1..100: mol_type = other DNA
aaggcactggctatttcagcagcatagaaacgagcccgtggttccaggaagcagcgttccctctggagatggtagaacaactgcaggagacagaacaaag

SEQ ID NO: 414 - DNA, 100 bp, Homo sapiens
  source 1..100: mol_type = other DNA
tcattctgggttgcaaatgaatttaattagttttgacatacacagcaaaagaacaactgcaggaagtggccccaagtaatctattaactataaacctgac

SEQ ID NO: 415 - DNA, 100 bp, Homo sapiens
  source 1..100: mol_type = other DNA
aggttgaaggaaatgctaattctggtaacattctccccaccaaaaatctttgaaaacttttttctcaaactaaaacaaagcaggctgtgcagagacacta

SEQ ID NO: 416 - DNA, 100 bp, Homo sapiens
  source 1..100: mol_type = other DNA
agagttgacttctatcccccctgctcacctctccaccattaatgtagtctaggacaaagtacaatttgtcagcagtctggaaagagaagtgaaggcccac

SEQ ID NO: 417 - DNA, 100 bp, Homo sapiens
  source 1..100: mol_type = other DNA
caggaaagggtgcttcacattcttcaacagaacattccgctccgacataatatgcttctcctaggaaaatgacgattcagatttagtggcatgtttcaac

SEQ ID NO: 418 - DNA, 100 bp, Homo sapiens
  source 1..100: mol_type = other DNA
gaggacatgaaggaagtgtaccaaaagatcttcagatttgaaattacctttccaaaactgccctttccgatcactttcaagaagtgaaagtcagatggtt

SEQ ID NO: 419 - DNA, 100 bp, Homo sapiens
  source 1..100: mol_type = other DNA
tagcatgaggattggacgacgggccaaggttgatttgctgagaaggacttggctagaaaaaaaaaaaaagaatttcttttaataccattgcttcaaagga

SEQ ID NO: 420 - DNA, 100 bp, Homo sapiens
  source 1..100: mol_type = other DNA
aatttcttttaataccattgcttcaaaggaagacatctataacataaacgatgtagaaaatgttacatctacaaatgactgatgcaaatgaccatacatc

SEQ ID NO: 421 - DNA, 100 bp, Homo sapiens
  source 1..100: mol_type = other DNA
aataaaataatactctgactcaatacttaaatatttatatcacttgttatgccataatgaagcattcctgccttgatactaatttctagaaatgctattt

SEQ ID NO: 422 - DNA, 100 bp, Homo sapiens
  source 1..100: mol_type = other DNA
taatccattaatgtaggaatactaactgactcccttacagttctccacagatgcacggcacatacaaaaacttactggaggagaagggttggcattcata

SEQ ID NO: 423 - DNA, 100 bp, Homo sapiens
  source 1..100: mol_type = other DNA
agctcaggctcctgaggttgggagatcttcaagatggactgaacttcagggctgcagggaataaagggcacgatttagaatccagctcgccactaggggg

SEQ ID NO: 424 - DNA, 100 bp, Homo sapiens
  source 1..100: mol_type = other DNA
cacaccaacatcaaaagtgagtttctggctctaccgacttctacccggataattcactgtttaaactgaaaataccccaatacattagtcagttaaagaa

SEQ ID NO: 425 - DNA, 100 bp, Homo sapiens
  source 1..100: mol_type = other DNA
aataataaaccccattaaatacagaaataaggattgttgctcatggagaaaggccgtgaattcggccaacacgaaccatttatcttacatctccagttca

SEQ ID NO: 426 - DNA, 100 bp, Homo sapiens
  source 1..100: mol_type = other DNA
agccaaatcagcaaattaactttaatgtttaaaatgtgtcaaatatattagaatttaaggagaaatgagatccccaccccagaagaagtcttcgccttcc

SEQ ID NO: 427 - DNA, 100 bp, Homo sapiens
  source 1..100: mol_type = other DNA
cgataaacgccgtgatgagaatgtttaccgctggcaaattcaaactatactagttatttcctcaaatccggtcaaacttactgtttgcatgcataggagt

SEQ ID NO: 428 - DNA, 100 bp, Homo sapiens
  source 1..100: mol_type = other DNA
tattggcaatcttctgaataaagtcgttcagacccatcctcctctgcttcatgaaagctgtggatgaaggaggagaaataaagaaacgtttagacggctt

SEQ ID NO: 429 - DNA, 100 bp, Homo sapiens
  source 1..100: mol_type = other DNA
cataacgtccggcgccacacacactaatctgatccgggactttcaaaaaatttccactttgcgtctcctggagcagaagtcccgcaagattcctgcactc

SEQ ID NO: 430 - DNA, 100 bp, Homo sapiens
  source 1..100: mol_type = other DNA
accgatgagaattgccaccatgcccctcatcctggagtaagtgagggtgcccttagcagcctcagttttcaccgtcatcaccaccgcggggagacagaaa

SEQ ID NO: 431 - DNA, 100 bp, Homo sapiens
  source 1..100: mol_type = other DNA
gacgttagcgctcaaagaccggctcggcgtatgctgcgccaggccgcgcgctcggccttataaaaaaggcaccgccgcgggggcggggcctgcgcgacag

SEQ ID NO: 432 - DNA, 100 bp, Homo sapiens
  source 1..100: mol_type = other DNA
agggtgagaggagtcaccaggtaaagatgggttggaaggacctggcaggcagagcagggagcaggaccccagtccagggcagcagggaagcgggagtctg

SEQ ID NO: 433 - DNA, 100 bp, Homo sapiens
  source 1..100: mol_type = other DNA
ggcagagctgattccaggcagctcagtattgctggcctgtgcatcctgagacttatccgagtcgcaggtgaagctggtgggaatcaggcagagtgcagag

SEQ ID NO: 434 - DNA, 100 bp, Homo sapiens
  source 1..100: mol_type = other DNA
ctttagctggggcagggttagccaagagcctgtcatggagctgctctctgggcactgggaaacataagtctggaggctttggctgcagctgcagataaag

SEQ ID NO: 435 - DNA, 100 bp, Homo sapiens
  source 1..100: mol_type = other DNA
atgcaggggcctctgacgatgggggccttagtcatctcagaggtggtgcagagggtagaagcctgactggggtcagagatgaggaaggagagggtcagaa

SEQ ID NO: 436 - DNA, 100 bp, Homo sapiens
  source 1..100: mol_type = other DNA
acagtgattctaaaccaatttggttgaggcagaagatactaatggccgaggggaggagagagggagcgtaggctctaaaggggaagcttgttaggaatga

SEQ ID NO: 437 - DNA, 100 bp, Homo sapiens
  source 1..100: mol_type = other DNA
agacagaggcgcaggcacagccctttcatcagctgaccaggagtgctcggcccggcctgccaggaacctcttatcaaactccaccggctgcctgcatcta

SEQ ID NO: 438 - DNA, 100 bp, Homo sapiens
  source 1..100: mol_type = other DNA
caattcaagtccatggctaaccttctgttagagacagaaattctgctgcagccagcaagtttgctggtgtacagggcaccgcttcatgggcctagtagga

SEQ ID NO: 439 - DNA, 100 bp, Homo sapiens
  source 1..100: mol_type = other DNA
agcgaagctgaaaggcaacttccgaaagccagtctcctctcccaaacgccctttaatatctccccagttggatctggggcgcctgtggtttcggaccctt

SEQ ID NO: 440 - DNA, 100 bp, Homo sapiens
  source 1..100: mol_type = other DNA
aggagctctgagaactggtgtgtgtggtcggaagccatctgagtctccctgtgatttggactttttaagaaacttctaagttgtattactatacccttta

SEQ ID NO: 441 - DNA, 100 bp, Homo sapiens
  source 1..100: mol_type = other DNA
ttcccttgtcatatgacttccatcctcagcactacaatattatcattaatgtttaaatcattgtcaagtctgtgattgccttagagatttattaagaata

SEQ ID NO: 442 - DNA, 100 bp, Homo sapiens
  source 1..100: mol_type = other DNA
acatgctaggattaggaaagtttaactttttaccatccttaaaattagatttttgaaaactgtcttatccccattaaagaaaaaaataaaaaggatgaat

SEQ ID NO: 443 - DNA, 100 bp, Homo sapiens
  source 1..100: mol_type = other DNA
tatacatacctgcacatatatacagcatatgtatatgtgtctgtattatatgtattaaatgaaagattatccacattttgttctttaggatcttcagcag

SEQ ID NO: 444 - DNA, 100 bp, Homo sapiens
  source 1..100: mol_type = other DNA
ctctcttcccatcacaatagaaaggcctgagctaacatttccatttctgcaaaaggcagattttgttcaattaaaaattataatgccttaaatttccaca

SEQ ID NO: 445 - DNA, 100 bp, Homo sapiens
  source 1..100: mol_type = other DNA
gacatttaagagacttcgttttcactgtgataaacaggtttgatttggacttataacttttttctaaaattatcaaattaataacgactataatgaaata

SEQ ID NO: 446 - DNA, 100 bp, Homo sapiens
  source 1..100: mol_type = other DNA
gaggcaaatattttagaggattcattccttggggtaacatttgttctataatttatagtctcataatgttgagagattaaagcatttaaataacattgtc

SEQ ID NO: 447 - DNA, 100 bp, Homo sapiens
  source 1..100: mol_type = other DNA
aactaactttcagcttacctttcttaaggaaaaaaaacaaaaaaatgttaaaaatagacatgtatttttcaaacatacaattcatgtttttatgtcatta

SEQ ID NO: 448 - DNA, 100 bp, Homo sapiens
  source 1..100: mol_type = other DNA
aagagatgtgagggacttataaataatattaagataacaggaattaaagtctcggtgtgtgaaaatactgtatatctaggatgcacataaaaactgccct

SEQ ID NO: 449 - DNA, 100 bp, Homo sapiens
  source 1..100: mol_type = other DNA
tacagatcttgcagggaaaagtacctgactatactgtataagacttctgctgtaccatttaatcataccaaaaaaaatggaatcaacacacaaatagatt

SEQ ID NO: 450 - DNA, 100 bp, Homo sapiens
  source 1..100: mol_type = other DNA
tcttttccactgttctcaatttaaaaataattggagaaatgtgtgctttgtttagaagagtaaaggaaaacattcattcaatagtaccatgcagaatgat

SEQ ID NO: 451 - DNA, 100 bp, Homo sapiens
  source 1..100: mol_type = other DNA
cagaaaaatagaaagattatcatcggatttgggaatcaaagacagctcagcaaaatactaggacatggctcatataagatggaataagcctggaaataca

SEQ ID NO: 452 - DNA, 100 bp, Homo sapiens
  source 1..100: mol_type = other DNA
ctttaggggatagctctgcaaggggagaggttcgggactgtggcgcgcactgcgcgctgcgccaggtttccgcaccaagacccctttaactcaagactgc

SEQ ID NO: 453 - DNA, 100 bp, Homo sapiens
  source 1..100: mol_type = other DNA
ctcccgctttgtgtgccccgctccagcagcctcccgcgacgatgcccctcaacgttagcttcaccaacaggaactatgacctcgactacgactcggtgca

SEQ ID NO: 454 - DNA, 100 bp, Homo sapiens
  source 1..100: mol_type = other DNA
gccgtatttctactgcgacgaggaggagaacttctaccagcagcagcagcagagcgagctgcagcccccggcgcccagcgaggatatctggaagaaattc

SEQ ID NO: 455 - DNA, 100 bp, Homo sapiens
  source 1..100: mol_type = other DNA
gagctgctgcccaccccgcccctgtcccctagccgccgctccgggctctgctcgccctcctacgttgcggtcacacccttctcccttcggggagacaacg

SEQ ID NO: 456 - DNA, 100 bp, Homo sapiens
  source 1..100: mol_type = other DNA
acggcggtggcgggagcttctccacggccgaccagctggagatggtgaccgagctgctgggaggagacatggtgaaccagagtttcatctgcgacccgga

SEQ ID NO: 457 - DNA, 100 bp, Homo sapiens
  source 1..100: mol_type = other DNA
cgacgagaccttcatcaaaaacatcatcatccaggactgtatgtggagcggcttctcggccgccgccaagctcgtctcagagaagctggcctcctaccag

SEQ ID NO: 458 - DNA, 100 bp, Homo sapiens
  source 1..100: mol_type = other DNA
gctgcgcgcaaagacagcggcagcccgaaccccgcccgcggccacagcgtctgctccacctccagcttgtacctgcaggatctgagcgccgccgcctcag

SEQ ID NO: 459 - DNA, 100 bp, Homo sapiens
  source 1..100: mol_type = other DNA
agtgcatcgacccctcggtggtcttcccctaccctctcaacgacagcagctcgcccaagtcctgcgcctcgcaagactccagcgccttctctccgtcctc

SEQ ID NO: 460 - DNA, 100 bp, Homo sapiens
  source 1..100: mol_type = other DNA
ggattctctgctctcctcgacggagtcctccccgcagggcagccccgagcccctggtgctccatgaggagacaccgcccaccaccagcagcgactctggt

SEQ ID NO: 461 - DNA, 100 bp, Homo sapiens
  source 1..100: mol_type = other DNA
gctccccatctgtccccacagttgctccttggctgagccaagggcttgctcacctctcagagcattgccctaactggtttgttttgggcttacattgcaa

SEQ ID NO: 462 - DNA, 100 bp, Homo sapiens
  source 1..100: mol_type = other DNA
gatcaggtcctccccagagccaggctggagtccgaggcagaaaaggctgtggagggcactggggtcaccacagactggaaaccggttgggcgcaggcccc

SEQ ID NO: 463 - DNA, 100 bp, Homo sapiens
  source 1..100: mol_type = other DNA
aaaccttgaggaatcgtttgggctgggaccagaacagggggctcctctgcacagagctccccaccgctttggtggattacttcagactcagaaaattgac

SEQ ID NO: 464 - DNA, 100 bp, Homo sapiens
  source 1..100: mol_type = other DNA
acaaagagaaactgacctgcccgcagccagccctggctgcctacacaagctttcccctgcttgccaggccactcagcactgcgtggcagacacggacatg

SEQ ID NO: 465 - DNA, 100 bp, Homo sapiens
  source 1..100: mol_type = other DNA
ctcgccccgggaagctcaccttcactccagccgggtctctgctgcctttgttaaataggggacctgcggctaggaaagctggatcccaggctgttgggat

SEQ ID NO: 466 - DNA, 100 bp, Homo sapiens
  source 1..100: mol_type = other DNA
gggggggagcggggtgggaggaccaggcatggggacggctcctagcccgggagcaactccctgacctgaagcccgcagagaccccgagcggcacccgagc

SEQ ID NO: 467 - DNA, 100 bp, Homo sapiens
  source 1..100: mol_type = other DNA
cgaggctgccgaagcctgtcaccttcctccagcctggctctgcagcaaacagaaaggaaacgcgattcgttccacttggaatttccttgaaatctccgaa

SEQ ID NO: 468 - DNA, 100 bp, Homo sapiens
  source 1..100: mol_type = other DNA
tctaatccggcgttaactcaccgtgagaggagcgctcatctcacaggaggctgtggtaatgggtgaattggcaggatccctgcgggccaggcagccaggc

SEQ ID NO: 469 - DNA, 100 bp, Homo sapiens
  source 1..100: mol_type = other DNA
ttttcgtttcttatcctctttttttaaaggggagaagccatgagaaaaggcgtcctgcagagaaggacccaatggggtctttaagggtctctgtatgaac

SEQ ID NO: 470 - DNA, 100 bp, Homo sapiens
  source 1..100: mol_type = other DNA
tggccggctcctaagcagaagctgaactcagaaaccgctacttccttgatttttcaaagccccctcctcaactccaggacgcctttggagccctagcccc

SEQ ID NO: 471 - DNA, 100 bp, Homo sapiens
  source 1..100: mol_type = other DNA
tgtcgccgccggagccttgaaaggctgcagctcgctgcccaagctacgcgttgccggaggcgggattcccaggtgcctcagcccgggcggccaagtgcgt

SEQ ID NO: 472 - DNA, 100 bp, Homo sapiens
  source 1..100: mol_type = other DNA
tgtttcaggtcccctgcctgggatccctgcactttgcaaagttagctgcgcggctgcagaggtccgagatccttccggccttagtacctgacccacggtc

SEQ ID NO: 473 - DNA, 100 bp, Homo sapiens
  source 1..100: mol_type = other DNA
cggcacccccaacccggtcccggcgggagagtgagagaagcgagctcgccgcctacttactatgcatggatgcaaacgggtcgtgcttacagtgtatttc

SEQ ID NO: 474 - DNA, 100 bp, Homo sapiens
  source 1..100: mol_type = other DNA
catcggggcgctccagactgcaggccggcccacgccgccgcctcccggcgccaaggggctgcccagggcggatagggagcctcgccaccaggccaggcac

SEQ ID NO: 475 - DNA, 100 bp, Homo sapiens
  source 1..100: mol_type = other DNA
tgtgcgagctgggctcagaaaacactgctggagcttcggggtctctctcagagcctccctgctggagaccgcccggagctgcgcggagaggcgggaaatg

SEQ ID NO: 476 - DNA, 100 bp, Homo sapiens
  source 1..100: mol_type = other DNA
gtgctagcgcacccgggctaggagcgggtgcccaactccggctggcttccctccctggctggctcaagcagcagctccgggcccagcccggggtagctgc

SEQ ID NO: 477 - DNA, 100 bp, Homo sapiens
  source 1..100: mol_type = other DNA
ggccaaggcgcccgcggcttcgggggcatagcgtaggggcccgcctccgggacagccagcagcccccggccccaggaaggagcagctttgaggaggccgc

SEQ ID NO: 478 - DNA, 100 bp, Homo sapiens
  source 1..100: mol_type = other DNA
cggaacaatcggcccttgacttcactcagggggcggagagacccgggggctgccaggctggttccgcggcctcgatgcttctgaggtccctcctcgaccc

SEQ ID NO: 479 - DNA, 100 bp, Homo sapiens
  source 1..100: mol_type = other DNA
cacacaggcaaacaacttttggacacaaactcatatatttttacatcttttaaaaatacatatactgtaatgaacacactgagtcccttatataaacaca

SEQ ID NO: 480 - DNA, 100 bp, Homo sapiens
  source 1..100: mol_type = other DNA
caggccctaacttgcagacccccggaaggacgccagcgtgaacattcagaaacagagaaaaacacagacaaactcacagatatttggactgatgcagaag

SEQ ID NO: 481 - DNA, 100 bp, Homo sapiens
  source 1..100: mol_type = other DNA
acagtttgaagtgtgagcctgaacatgtttgatctaaggtctggaggaagatgtgaagcaaatctgacctaaaaaaaattataggaaaaaagcaaattgt

SEQ ID NO: 482 - DNA, 100 bp, Homo sapiens
  source 1..100: mol_type = other DNA
tctggatttgtttcaccaaggaacaagtaagcagagaaccagacactggagaaaaaaaggagtcaggaagtagacaaggaaatgttaaaagaaataatag

SEQ ID NO: 483 - DNA, 100 bp, Homo sapiens
  source 1..100: mol_type = other DNA
gataactgaaagaatgtagcttccagattgctagctatcagcagatagatagaaacttttatacagcctttaaatcttccctagaaacctttttaaaagt

SEQ ID NO: 484 - DNA, 100 bp, Homo sapiens
  source 1..100: mol_type = other DNA
caagggcctgccaggatgagaacgggcaaacctggccaaggtgaccccattagggactaccctcctagggacagcactcagggccgttcccaatcacccc

SEQ ID NO: 485 - DNA, 100 bp, Homo sapiens
  source 1..100: mol_type = other DNA
ggatttcctgtcctgctcgtctcctgccacacctccttttgatctacccccaagacacccctacctttttattctgtgaaaatttactcatgctgtgggc

SEQ ID NO: 486 - DNA, 100 bp, Homo sapiens
  source 1..100: mol_type = other DNA
cctgctggaaatgccctcctactgtttccccaaaccccgtcagaaattccacggggaaactcccttcccttctgctgcaggcaccgtcactgtgtctctc

SEQ ID NO: 487 - DNA, 100 bp, Homo sapiens
  source 1..100: mol_type = other DNA
agctctgccccccagcctctgagtaccaccttatcctagcccttagctactggcttgtcattgtctctttacgttctcagcctcccacagaagcctggga

SEQ ID NO: 488 - DNA, 100 bp, Homo sapiens
  source 1..100: mol_type = other DNA
aggcacactcgcccctggtctccaaggctctgggtcctcagactggctgagtactggggaccaaggtcacccaagaagccctgagtggccctcttgaggg

SEQ ID NO: 489 - DNA, 100 bp, Homo sapiens
  source 1..100: mol_type = other DNA
ttagcagagcttctctctgtccaagacaggtcaggctctctcccctggccccagctccaccgtcactcagaggagtggcctaaacaaacgctgcaggtga

SEQ ID NO: 490 - DNA, 100 bp, Homo sapiens
  source 1..100: mol_type = other DNA
ggctcccgagcccctgacatggatgtttatggaagaggactcttggcatcagcacctgggcaaggtgggtagaggcaggagtgggcaaatgggaaagtct

SEQ ID NO: 491 - DNA, 100 bp, Homo sapiens
  source 1..100: mol_type = other DNA
ggagagccgtttgagattcaccaggtgaatgaaccccggtttttttctgggtaacaggtcgaatgtgaattacttattttcacaagctcttgacatgttc

SEQ ID NO: 492 - DNA, 100 bp, Homo sapiens
  source 1..100: mol_type = other DNA
cgtcaaattgctgttccccaaagagtggactctggtgacatataagtgtgtgggaccattgcatcttaccccagagatccactcctgatctggcattatt

SEQ ID NO: 493 - DNA, 100 bp, Homo sapiens
  source 1..100: mol_type = other DNA
caaaatctgctgaattcaaaacgatcctgtacttcctgctcaccaggtctgaaaagaaaaaagaaaaaagaagaaggaaagactacacctgacaaaagac

SEQ ID NO: 494 - DNA, 100 bp, Homo sapiens
  source 1..100: mol_type = other DNA
ttcacggtttctctttagttttatctgaaatacatttgtaagcttagggtgcaatttggattaaaacagttttctttagtgtcaataatggcctttacta

SEQ ID NO: 495 - DNA, 100 bp, Homo sapiens
  source 1..100: mol_type = other DNA
gagtgaatggatatttttccattctggattatcgtttaatcgaaactttgtttcctgtggaaatttttctggtttaagttatttgatttgggagataaat

SEQ ID NO: 496 - DNA, 100 bp, Homo sapiens
  source 1..100: mol_type = other DNA
catgtaacttaataaactttggcatcctggttaactgaaattgcttcattcaatatttgaagactgaaatctgtattgttgcctgtacctaaattatggg

SEQ ID NO: 497 - DNA, 100 bp, Homo sapiens
  source 1..100: mol_type = other DNA
ggacagacagggagagatgactgagttagatgagacgagggggcgggctgggggtgcgagaaggaagcttggcaaggagactaggtctagggggaccaca

SEQ ID NO: 498 - DNA, 100 bp, Homo sapiens
  source 1..100: mol_type = other DNA
gtggggcaggctgcatggaaaatatccgcagggtcccccaggcagaacagccacgctccaggccaggctgtccctactgcctggtggagggggaacttga

SEQ ID NO: 499 - DNA, 100 bp, Homo sapiens
  source 1..100: mol_type = other DNA
cctctgggagggcgccgctcttgcatagctgagcgagcccgggtgcgctggtctgtgtggaaggaggaaggcagggagaggtagaaggggtggaggagtc

SEQ ID NO: 500 - DNA, 100 bp, Homo sapiens
  source 1..100: mol_type = other DNA
ggggcaggcggagcttgaggaaaccgcagataagtttttttctctttgaaagatagagattaatacaactacttaaaaaatatagtcaataggttactaa

SEQ ID NO: 501 - DNA, 100 bp, Homo sapiens
  source 1..100: mol_type = other DNA
gatattgcttagcgttaagtttttaacgtaattttaatagcttaagattttaagagaaaatatgaagacttagaagagtagcatgaggaaggaaaagata

SEQ ID NO: 502 - DNA, 100 bp, Homo sapiens
  source 1..100: mol_type = other DNA
aaaggtttctaaaacatgacggaggttgagatgaagcttcttcatggagtaaaaaatgtatttaaaagaaaattgagagaaaggactacagagccccgaa

SEQ ID NO: 503 - DNA, 100 bp, Homo sapiens
  source 1..100: mol_type = other DNA
ttaataccaatagaagggcaatgcttttagattaaaatgaaggtgacttaaacagcttaaagtttagtttaaaagttgtaggtgattaaaataatttgaa

SEQ ID NO: 504 - DNA, 100 bp, Homo sapiens
  source 1..100: mol_type = other DNA
ttggagaagtatagaagatagaaaaatataaagccaaaaattggataaaatagcactgaaaaaatgaggaaattattggtaaccaatttattttaaaagc

SEQ ID NO: 505 - DNA, 100 bp, Homo sapiens
  source 1..100: mol_type = other DNA
ccatcaatttaatttctggtggtgcagaagttagaaggtaaagcttgagaagatgagggtgtttacgtagaccagaaccaatttagaagaatacttgaag

SEQ ID NO: 506 - DNA, 100 bp, Homo sapiens
  source 1..100: mol_type = other DNA
ctagaaggggaagttggttaaaaatcacatcaaaaagctactaaaaggactggtgtaatttaaaaaaaactaaggcagaaggcttttggaagagttagaa

SEQ ID NO: 507 - DNA, 100 bp, Homo sapiens
  source 1..100: mol_type = other DNA
tggtgtaagagatgtgccagcggctggccgaggggcgcttagggctagagcccggggcgctgcagaggttgagagtcagtgggtggggcgcagttatcaa

SEQ ID NO: 508 - DNA, 100 bp, Homo sapiens
  source 1..100: mol_type = other DNA
acaccagggcccaaaagcaggctctagataggttccaggtgctcaatttctatttcacgtttggagtgagccagtggaattgtgaagttgtggcattttg

SEQ ID NO: 509 - DNA, 100 bp, Homo sapiens
  source 1..100: mol_type = other DNA
attcggttgccaagagttatcactgggcctttgcaggtgccaaataaatttcaggacagagcctaaggcagagctctggcacaggaaggaagtaaaacgt

SEQ ID NO: 510 - DNA, 100 bp, Homo sapiens
  source 1..100: mol_type = other DNA
ttaatgagcaaatggacgcatgtttccaagcggtggtaggaagacagcagtttttggttgtcttcctggtgatcagcatggaaacctagtagtgctctta

SEQ ID NO: 511 - DNA, 100 bp, Homo sapiens
  source 1..100: mol_type = other DNA
ctctgatcaatacattgtcgaaggcatgtacctgatgctaacgtaacaataatattaaatattgactttatttgctattatttattgctaacattaagta

SEQ ID NO: 512 - DNA, 100 bp, Homo sapiens
  source 1..100: mol_type = other DNA
ctgctacctgctatgtgctaggtttgtctctgaagactttacatgtatttttcacgtttaattatcataatcttaagaagcaggtaccataattatctcc

SEQ ID NO: 513 - DNA, 100 bp, Homo sapiens
  source 1..100: mol_type = other DNA
gggaaaaagaatgacgaaaggcaagacagtggagcaagtgaggacacgcttcaccgagccagatctccactcctcccagggtatccacagggacaagtca

SEQ ID NO: 514 - DNA, 100 bp, Homo sapiens
  source 1..100: mol_type = other DNA
cacctggcagaaagctaagtcactcagctagaaacaggcccagggaattcaacagaaggctgaagagccactgcttatggaaataaagcccctcctgtaa

SEQ ID NO: 515 - DNA, 100 bp, Homo sapiens
  source 1..100: mol_type = other DNA
agaactgcatggcttttccctcccaaccccaaacccatcccacatctggcttttgttgtgtgaatcataaactgccctttcttcaccacagtgattcatg

SEQ ID NO: 516 - DNA, 100 bp, Homo sapiens
  source 1..100: mol_type = other DNA
aatcctctcccactgtggatctgtaaaatctagacaggtcagtcagctcccgccctttaagagtttattttccattctgtggaagaagcagataaggaga

SEQ ID NO: 517 - DNA, 100 bp, Homo sapiens
  source 1..100: mol_type = other DNA
gctgctgtccttaggagacatcctttagaggaagctggaagacacgggttcaggccctgcatcctcctctgagttgctatgtgactgggaacaggatact

SEQ ID NO: 518 - DNA, 100 bp, Homo sapiens
  source 1..100: mol_type = other DNA
tcacctctccattctttctctccttttctcttagggtcggaatatggaactagacaggaaagtactttggaggttttcttaccgtaaggaggctggcatt

SEQ ID NO: 519 - DNA, 100 bp, Homo sapiens
  source 1..100: mol_type = other DNA
gggccctccacccagcctcagttctatgggggacgtggagtcaggcgatgatgtcctctgaggcagcgtccatctccccttaacattaaggaataaggcc

SEQ ID NO: 520 - DNA, 100 bp, Homo sapiens
  source 1..100: mol_type = other DNA
agagggttctcgctcatttgggaaaataaaaaaagcaggaatggggcgctggaaattctataagcttttccccaccactcacaaaaacacagctgtgaaa

SEQ ID NO: 521 - DNA, 100 bp, Homo sapiens
  source 1..100: mol_type = other DNA
ataaataccaccccccaaaccaagggtctagggccaccaacagtcctcctcctcctcctcctcctccttctcctcctcgtcctccagatccagctgccaa

SEQ ID NO: 522 - DNA, 100 bp, Homo sapiens
  source 1..100: mol_type = other DNA
ccttctcctcctcgtcctccagatccagctgccaacagcatcccccgctcctgaagaaatgcaccgcccagaagggaacggcgaaagggggaagaagtcc

SEQ ID NO: 523 - DNA, 100 bp, Homo sapiens
  source 1..100: mol_type = other DNA
aggggacccccggcctctggccgagagcttgggtgggggcctcggccgtcgccactcacccggggaggggaaaagctccagatcgactttttccgtcttg

SEQ ID NO: 524 - DNA, 100 bp, Homo sapiens
  source 1..100: mol_type = other DNA
atgatggtgagagtcggcttgagatcgacggccgccttcatggtgccaggagtgggggacgtacgggatggtagcaagtttgcagttactgttgtttttc

SEQ ID NO: 525 - DNA, 100 bp, Homo sapiens
  source 1..100: mol_type = other DNA
tttttaatgaggattagtaacagggggaaggggacgggggaaatccgactttcttcccaaaaatctcaaattcccgctgcctttctttcccccgcgcccg

SEQ ID NO: 526 - DNA, 100 bp, Homo sapiens
  source 1..100: mol_type = other DNA
gacggtgcgcgcccggcactccaggggaagttggcactttgcggcgaagtgagcgcgctcgggtcccagcctcgcccgcgccgcgcccgctcctcctgcc

SEQ ID NO: 527 - DNA, 100 bp, Homo sapiens
  source 1..100: mol_type = other DNA
gagtgagtagcaaatattcatttatgacccagtttttgtccaccctcaggcggggcataggactacagacatttttctagattacagctaggatattatt

SEQ ID NO: 528 - DNA, 100 bp, Homo sapiens
  source 1..100: mol_type = other DNA
cctgagtttatgacaatgaaatggtttgagaaggcaatattgtggggctttcagagaggtttgctgagtggctaggtgcatgcatgggtttaaccattaa

SEQ ID NO: 529 - DNA, 100 bp, Homo sapiens
  source 1..100: mol_type = other DNA
cttccctttttgcctttttattataagctggttttgtctgtggctgtttttttcttttaaaattaattaaaacttctcaaaatttctaaaagtaaacaag

SEQ ID NO: 530 - DNA, 100 bp, Homo sapiens
  source 1..100: mol_type = other DNA
gcattctctacatacatctacatacatattttgcattttaaaaattggaatatttgtcatttttctgtattacccaaaagtatataaacagttaccagag

SEQ ID NO: 531 - DNA, 100 bp, Homo sapiens
  source 1..100: mol_type = other DNA
atttatgtgagaagacagttgtcacattacagatgtcagattagctataaaattgtttcattctagaaacctaatatggtaaaaataaaccttacttatt

SEQ ID NO: 532 - DNA, 100 bp, Homo sapiens
  source 1..100: mol_type = other DNA
tagccatttatcagacaattgcttttgttcagccagtttcttgttctagcagtataaatattctttttatagaaagttacttggtttgagaaataaacat

SEQ ID NO: 533 - DNA, 100 bp, Homo sapiens
  source 1..100: mol_type = other DNA
ataagcttaaggtaggctagagatgaaaaatttcagacttgtgtttgttttggatttattgtaccctttctactattatctgagaaagctatttaggagt

SEQ ID NO: 534 - DNA, 100 bp, Homo sapiens
  source 1..100: mol_type = other DNA
ttaagaaatagtctagttttaaaatagcaatggtttgccggacacagtggctcacccctgtaatcccagcattttgggaggccgaggtgggcagattgct

SEQ ID NO: 535 - DNA, 100 bp, Homo sapiens
  source 1..100: mol_type = other DNA
gaatttgccagttttcaatattctgattcactctgttaagctagtaaggcagtctttaaattacacagtctgtgtgttattttactactgctcagagggc

SEQ ID NO: 536 - DNA, 100 bp, Homo sapiens
  source 1..100: mol_type = other DNA
attggagaaggttcccttgtgattagaactgttcatgttgagacatgaatcataaggcattccaaagttggtttaaggtgtgtctgctttagacactgtg

SEQ ID NO: 537 - DNA, 100 bp, Homo sapiens
  source 1..100: mol_type = other DNA
cccaggactattcttttgctccagttttgccttttgattaaatcaatattatacctgagttttataaactactaagaatttgttccccttcctcactgtg

SEQ ID NO: 538 - DNA, 100 bp, Homo sapiens
  source 1..100: mol_type = other DNA
attttcttgcagtattttcttagaagagtcaactttaataacttaccccaaagtgcacgttcttgatattatgaacttgctattgttgtcttcccagttt

SEQ ID NO: 539 - DNA, 100 bp, Homo sapiens
  source 1..100: mol_type = other DNA
tattgtagtttttggaagggctcgttctgcccaagagaagttcctccttacagctgattcggctgtctaccatttgcacgttggtgctgttttgagtgct

SEQ ID NO: 540 - DNA, 100 bp, Homo sapiens
  source 1..100: mol_type = other DNA
acctcctgctggtgaggcttcatacagcacacagatggagccatcctctccaattctgtaggacacttcataggggtcaacccagagtgtgagttcactt

SEQ ID NO: 541 - DNA, 100 bp, Homo sapiens
  source 1..100: mol_type = other DNA
gggagaagcctgaacagctcctgactgctcagtccaatccgctgtgctgcctgtccaatcagaggatccattttatggttgatgcgaatacaacggtaac

SEQ ID NO: 542 - DNA, 100 bp, Homo sapiens
  source 1..100: mol_type = other DNA
ccgatcccttgcatggcttttctgggaaccagtgatgtttataatgttctatagaagaaaagaagaacagagaaacaacgcttaggatcgttagctccca

SEQ ID NO: 543 - DNA, 100 bp, Homo sapiens
  source 1..100: mol_type = other DNA
ctgcggattcctcctaccccaggctcctttgaggagcgaaaatgaaaactatcaactttttaaaatgtccaggattgcatccgttgttgtgcatgtgcgg

SEQ ID NO: 544 - DNA, 100 bp, Homo sapiens
  source 1..100: mol_type = other DNA
ggatggaaaaagcgggcagggttttagaaataacacagtagtaccggacaaaacaatctccaggaaccaaccggttgagccgccaaaacaggaatcaggc

SEQ ID NO: 545 - DNA, 100 bp, Homo sapiens
  source 1..100: mol_type = other DNA
gcgcagcctcggccagtcgggaagccactggcacctatggccaggcgagaaactgtttactttctccaccccaccccagatgcacacaatggagttgatg

SEQ ID NO: 546 - DNA, 100 bp, Homo sapiens
  source 1..100: mol_type = other DNA
gctttggagatgagaagcgccaccggactgttaaccccgaagggaagaaaaacaagcaaccctaaaccacgctctgggcagggctgttaattgtgccggt

SEQ ID NO: 547 - DNA, 100 bp, Homo sapiens
  source 1..100: mol_type = other DNA
acgcaacggttggagggggctgaggaaaggggacgtcgaacccaccccagccccacggctcctttgtccccaaatccgccgacggtcctcggaccgcagc

SEQ ID NO: 548 - DNA, 100 bp, Homo sapiens
  source 1..100: mol_type = other DNA
tcccgcctcggtgggcttaagtttctttgttgtgcgtgttgtcttctcctctccgttttgccagctggggggaagggggcgccctccgtccagcccctaa

SEQ ID NO: 549 - DNA, 100 bp, Homo sapiens
  source 1..100: mol_type = other DNA
agcctcgcggggaaccgctgttagcggccacccagcgcaaccacaccggtcccgcggcggggcccaagcgcgaccggccccggggcgctgccgaggttcc

SEQ ID NO: 550 - DNA, 100 bp, Homo sapiens
  source 1..100: mol_type = other DNA
cgcagccccgacggccggactctgacccagggatgtggggcccgcgtccctccgacgccctcgccctgctcacctgccagcagctcctgcaggctctggc

SEQ ID NO: 551 - DNA, 100 bp, Homo sapiens
  source 1..100: mol_type = other DNA
tgaaggtctgcagctgtcgctcgctcgtgagccccttggtgcggagaaacttggagatgaaggacacggcggcggcgatctcgcctatcatggtggcggc

SEQ ID NO: 552 - DNA, 100 bp, Homo sapiens
  source 1..100: mol_type = other DNA
ccgggtgtagaagggatgcatgggggcggcgtgcgggggcggcccggggcggctggggctcggcggcgcggccccgacggcggagcagccaccccgggct

SEQ ID NO: 553 - DNA, 100 bp, Homo sapiens
  source 1..100: mol_type = other DNA
acgccgcacccctcccccgtgcgttctgcggccacccaggccttccaggacaccgtggagagggaacaagggggcagggacgcccccttcggcaggagcc

SEQ ID NO: 554 - DNA, 100 bp, Homo sapiens
  source 1..100: mol_type = other DNA
gtcggagaagggggcccagaccggagggaggcgagaagccccactgaagccgggcgcagggtctgggacgcagttgggagtgcaaagggctggctgagag

SEQ ID NO: 555 - DNA, 100 bp, Homo sapiens
  source 1..100: mol_type = other DNA
ccgcaggagcagcaggctgtggcccaggcctcctgggtgacaggccctgtctggcggggaagagggaccaagagacaacacggaagaggctggacctcga

SEQ ID NO: 556 - DNA, 100 bp, Homo sapiens
  source 1..100: mol_type = other DNA
acaggggcggctgcctcactccctacctgagccagccgagggggccaaggactttagagctgtttcctccggcataagagagacacttgctttccagggc

SEQ ID NO: 557 - DNA, 100 bp, Homo sapiens
  source 1..100: mol_type = other DNA
agcaccctttatcggagaaggctctacagggaaggggtctttgcagcctggatggccatcccacattcctttaacggaggtctctaggcctcagagagaa

SEQ ID NO: 558 - DNA, 100 bp, Homo sapiens
  source 1..100: mol_type = other DNA
cccagagttagaaaggaggccagacggtccttgctgtccccctggggagagaggaagttgccgcctgctgccaggcccaggaggagctgggcctgcaata

SEQ ID NO: 559 - DNA, 100 bp, Homo sapiens
  source 1..100: mol_type = other DNA
gtgggggacctggcccctgaggcagtggcggccatgtcacggccaggccacggtgggctgatgcctgtgaatggtctgggcttcccaccgcagaacgtgg

SEQ ID NO: 560 - DNA, 100 bp, Homo sapiens
  source 1..100: mol_type = other DNA
cccgggtggtggtgtgggagtggctgaatgagcacagccgctggcggccctacacggccaccgtgtgccaccacattgagaacgtgctgaaggaggacgc

SEQ ID NO: 561 - DNA, 100 bp, Homo sapiens
  source 1..100: mol_type = other DNA
tcgcggttccgtggtcctggggcaggtggacgcccagcttgtgccctacatcatcgacctgcagtccatgcaccagtttcgccaggacacaggtgagcag

SEQ ID NO: 562 - DNA, 100 bp, Homo sapiens
  source 1..100: mol_type = other DNA
acacccaccccatgccacccgccccgccgagccatcactaccttgcagcgtaggatgctgaaaatcccagtaaatctgctgatgccaaatcccttcccca

SEQ ID NO: 563 - DNA, 100 bp, Homo sapiens
  source 1..100: mol_type = other DNA
tctccctgcctcacctccagaaaaacagggcagtctaaccttgtccagtttaagacttggattccaatgcagcctctgagcaagctgtagggccttgagc

SEQ ID NO: 564 - DNA, 100 bp, Homo sapiens
  source 1..100: mol_type = other DNA
gggtagatcaatatctctcacagctgagtgaggattaaataaaattgtgctcactgagcacagaacctagaacagcagtagcatgggattgtagaataag

SEQ ID NO: 565 - DNA, 100 bp, Homo sapiens
  source 1..100: mol_type = other DNA
ggctttacatgcacttcctcatttgatttttcccaagaatcacaggcagtaagtctgtgtattgttgtattattatgagtcccattttatagatgaagaa

SEQ ID NO: 566 - DNA, 100 bp, Homo sapiens
  source 1..100: mol_type = other DNA
tttatagatgaagaaaccgagtctcccagaagctgagtgatttaaactcagagctgggatttaaacccaggcggttgagttccagaaccaaagttcttaa

SEQ ID NO: 567 - DNA, 100 bp, Homo sapiens
  source 1..100: mol_type = other DNA
ctggtatcctatactggctccaagtgttggtttgtggggtggagtcgtgctggtggtaattaattggggatggggggcgttggtggtgttgatggtgggg

SEQ ID NO: 568 - DNA, 100 bp, Homo sapiens
  source 1..100: mol_type = other DNA
tgaggtggcaatgatggaggagacagtgttagcggttgtgttggtggtgactcagtgatagtattgatggtggtggggtcttggtgacaatggagggatg

SEQ ID NO: 569 - DNA, 100 bp, Homo sapiens
  source 1..100: mol_type = other DNA
tgttggtgacattgatagttgtgttggtggtggtgctggaagtggtgtgatggggtggtgatgatggagaaaatgagagaatgatgttggtggcagtctt

SEQ ID NO: 570 - DNA, 100 bp, Homo sapiens
  source 1..100: mol_type = other DNA
cgtggccatgtggtgtggctggtagccctgtgtgtggctgttacttagtggtattggtgatcctgttgtggttgtaatgatggtgatgttgatggttgcg

SEQ ID NO: 571 - DNA, 100 bp, Homo sapiens
  source 1..100: mol_type = other DNA
ttggtggtaatgtgatggctgatgatggagataaaatcgatgaggtcccactctcaggcctactctcttttgttctggagatttgtcatcgttggggaga

SEQ ID NO: 572 - DNA, 100 bp, Homo sapiens
  source 1..100: mol_type = other DNA
tgaaatggctgctgtcgggctgtcatctccaggcccggggcgctgacatttgggccactctcggtctccctcttcattctgggcgcgcattagctctggt

SEQ ID NO: 573 - DNA, 100 bp, Homo sapiens
  source 1..100: mol_type = other DNA
ccggccggttccgctgcagctgaacagcaagatgcggcacccaggttaccctgatcatcgcagatttctccccggggctctgttctgaggcctcaaaagt

SEQ ID NO: 574 - DNA, 100 bp, Homo sapiens
  source 1..100: mol_type = other DNA
gctccttgtagatgggaccaggggtcatttgggcagtagcagcgcctggtctcagtctggtactgaagtcaggaatggcttaaggtgaaatcgtggtcct

SEQ ID NO: 575 - DNA, 100 bp, Homo sapiens
  source 1..100: mol_type = other DNA
ctggtgaagctcagcgaagaccccctcgccttgtttatgacaagagaacttctgggggcgggaggaagagtccctgttacgatgctgatcatcattgagc

SEQ ID NO: 576 - DNA, 100 bp, Homo sapiens
  source 1..100: mol_type = other DNA
ttttgctgagcagaaaactctttagtactcaaggtcgagagtctctggtggtctgcctggcaccaggcaccttcctacaaccctagttttccaaaaggac

SEQ ID NO: 577 - DNA, 100 bp, Homo sapiens
  source 1..100: mol_type = other DNA
aaagcctggggcaggcgacgtcctagctcgcatttgaacagggccgcgggccagcagagatgcgcgatgcccaactctttccaagagcacctcgcgtccc

SEQ ID NO: 578 - DNA, 100 bp, Homo sapiens
  source 1..100: mol_type = other DNA
gaaccggtgccttcaactcggagaagtcaagagacccgcaagaaacttgcacgactgcacccgccgccgcgctctgggggctgggcaggggcagctgggc

SEQ ID NO: 579 - DNA, 100 bp, Homo sapiens
  source 1..100: mol_type = other DNA
tggctcccggggaacgcgacccccccgcgccccgcagaccggctgtctcccatggacccctcggcacctgcagcctccgaggaagggtcagcgcgcgtgt

SEQ ID NO: 580 - DNA, 100 bp, Homo sapiens
  source 1..100: mol_type = other DNA
ggggggctcgggccagccgatgtttttggccagaagccgttcgtcctgggccgcggctgcctctccacaccgggagctcgtgtttgttttgcggagggag

SEQ ID NO: 581 - DNA, 100 bp, Homo sapiens
  source 1..100: mol_type = other DNA
ctgttgtttttgttctctgcaccggggagagggggacttggtggcggccgcgcgtggttttcgggatcacattagcgtccgcccggcgtggcccggtcga

SEQ ID NO: 582 - DNA, 100 bp, Homo sapiens
  source 1..100: mol_type = other DNA
cattaaggggatcgaacctttccgcggcctcgtcggggtctgctcggaatcggcccctgggccaggcccgaggcgcaagcagatcgccaggttgggtcag

SEQ ID NO: 583 - DNA, 100 bp, Homo sapiens
  source 1..100: mol_type = other DNA
agttgttgaaaactccccgctgcctgatttcaactttattatttttttcccacgccttcactggggtcccggagggagaggagccgccgcaacgctggct

SEQ ID NO: 584 - DNA, 100 bp, Homo sapiens
  source 1..100: mol_type = other DNA
agtagcgcctcggtctctaaaagccactgggggcgagcctccggtgtggcggtgtcacaagttagctgtcctttctgagtcaaacccaacaaaaaaggca

SEQ ID NO: 585 - DNA, 100 bp, Homo sapiens
  source 1..100: mol_type = other DNA
agaggaaaatcaataaagtccacgtgctccccggcctcctatggaaagggctggctgcgatggccggatgcccggccgtgggctgggtttggctccagtg

SEQ ID NO: 586 - DNA, 100 bp, Homo sapiens
  source 1..100: mol_type = other DNA
ggacaaagaattttcagaaccgtgagaaggggaggctttccaaagttgagatccaagtcgtcggtgtctcgggagctcccctggtacacagggtgcccgg

SEQ ID NO: 587 - DNA, 100 bp, Homo sapiens
  source 1..100: mol_type = other DNA
tgcccgactggagccatttaaaaatggcagaaacagctgcaggccaacacacacacgctggaaaacaacccgcagccccctctactgtgggattccccgc

SEQ ID NO: 588 - DNA, 100 bp, Homo sapiens
  source 1..100: mol_type = other DNA
gggaagcccggagttgctcccctccttgcctcagcccctgtgcaaagaaagaactggtgtctgtgcctgggtcccttctgtcgccggcctggaggttggg

SEQ ID NO: 589 - DNA, 100 bp, Homo sapiens
  source 1..100: mol_type = other DNA
aaacagccggcaagccgcctttctctgctcgaggaggcgtggtggggcctcctactccaggttcccggctggacagaggctcctgcaccctgacagctgc

SEQ ID NO: 590 - DNA, 100 bp, Homo sapiens
  source 1..100: mol_type = other DNA
ggaggccttccagcccgctgaccccgcggggaccaggcctgtagttggagcttgaggggctgtacctctgcgcctccctgggtttggggaaacaacacat

SEQ ID NO: 591 - DNA, 100 bp, Homo sapiens
  source 1..100: mol_type = other DNA
cgtgtcctctgaagacctcaggctttgggatctcatggtccagcttccagttcacttcgttgccgcgaccttgggcatatcattgtcacttctctaacca

SEQ ID NO: 592 - DNA, 100 bp, Homo sapiens
  source 1..100: mol_type = other DNA
tggtgacccggggttttgtgcttggcttccaggtcccctcgggttattgaggacgattgaggtcatgcctccgagagcaccgcgccctgggcgcaggagg

SEQ ID NO: 593 - DNA, 100 bp, Homo sapiens
  source 1..100: mol_type = other DNA
aatgcaaatttaacagggcaccctgtattttacccagagggaagccgaagtgtttggcagatcatttggccccatgagccttgggtgggtttctcctcag

SEQ ID NO: 594 - DNA, 100 bp, Homo sapiens
  source 1..100: mol_type = other DNA
ccctagtgacccctaaaattacccccccgacccacccactgtcccctgatgcttcccccacccccggaaaaagctgtggcctccctctcatttggggcag

SEQ ID NO: 595 - DNA, 100 bp, Homo sapiens
  source 1..100: mol_type = other DNA
gctgcctcctgttctctttttctggtgtttcagcaaggcaggccagtggaggtgaggtgaccagaagatggctaaagggaaaacaaaatggtgggcctct

SEQ ID NO: 596 - DNA, 100 bp, Homo sapiens
  source 1..100: mol_type = other DNA
ccagggtttgggggccctgtgctggtggaggagagaagaccccagggcgatggtaggagacgaaagcttgggctgcagcgtaagcttggaggcccgctgc

SEQ ID NO: 597 - DNA, 100 bp, Homo sapiens
  source 1..100: mol_type = other DNA
ggtggctcacgcctgtaatcccagagctttgggaggctgagacaggaggattgcttgagcccaggagtttgagaccagcctgggtctcaaaccaaaaaaa

SEQ ID NO: 598 - DNA, 100 bp, Homo sapiens
  source 1..100: mol_type = other DNA
taaatataattttaacgccaatctgagaaaaatgacttattagctgtgtgattttgagcaatgctcttaacctcccccatgaaggatggtgtgagaacga

SEQ ID NO: 599 - DNA, 100 bp, Homo sapiens
  source 1..100: mol_type = other DNA
acagaattgtagcacgtgtatcagtctggtacacaatgtcctatgaaggttagctttattatcaccatcattattattgcagaaagactttcagttcaga

SEQ ID NO: 600 - DNA, 100 bp, Homo sapiens
  source 1..100: mol_type = other DNA
ataagacagcacagttacagagacctggttttattttccagcttcttaactgagtcatctttcagctccttttaattaaaaagaaaaaacaatcagagat

SEQ ID NO: 601 - DNA, 100 bp, Homo sapiens
  source 1..100: mol_type = other DNA
tcaaagacctggcagaaatgacttcccaaccccagatgcccccagcagcagtatttagcagtcatacaattgcctgaaatgaagaatgagtaatctggat

SEQ ID NO: 602 - DNA, 100 bp, Homo sapiens
  source 1..100: mol_type = other DNA
gagtcggccctgaaatcgacctgcaacttacccggaacgtgagctgtctctctctgacctctgctggctgcttcacctggagtctgagtccgactcatgt

SEQ ID NO: 603 - DNA, 100 bp, Homo sapiens
  source 1..100: mol_type = other DNA
agcacttcactgtccgcgttagtttagccttcactgtcagcaactcgtcaccttgtcctcttgcagcgaaggtttggaatcccatcacgggtgtgcagtg

SEQ ID NO: 604 - DNA, 100 bp, Homo sapiens
  source 1..100: mol_type = other DNA
gttagtcctgagatcatggtggtgctaggagaacctgccaaccaatacagaaagttgtcacgaatagaaacctaagctctggccgggtgcggtggttcaa

SEQ ID NO: 605 - DNA, 100 bp, Homo sapiens
  source 1..100: mol_type = other DNA
agatatactgttctagacatgtgtctgaaaggaatcctgcaaattctgtcttattgaacaggcataaggtgtcacgtcaggcgtaaggtgtcacagcagg

SEQ ID NO: 606 - DNA, 100 bp, Homo sapiens
  source 1..100: mol_type = other DNA
cgtaaggcgtcacgtcaggcgtaaggtgtcacagcaggcgtaaggcatcacgtcaggcgtaaggcgtcacgtcaggcgtaaggtgtcacaagctcggtga

SEQ ID NO: 607 - DNA, 100 bp, Homo sapiens
  source 1..100: mol_type = other DNA
acgtcaggggtgtgccttgtgttctctgttcgttgctttcagaagcagcagcatgtggcagcatctctgtgcctatgacgatattgcagtgaatatgaga

SEQ ID NO: 608 - DNA, 100 bp, Homo sapiens
  source 1..100: mol_type = other DNA
aattgtacatttcaacaacataaataagctgttcaagactgtctcccatgcctccaaaacaaataaaaaccccccacaactcaaatgcatataagctgtt

SEQ ID NO: 609 - DNA, 100 bp, Homo sapiens
  source 1..100: mol_type = other DNA
actatagtataatggtgagttatagccagtgtatgatgggattgttgatagaataatgcatattagagcttttagttcaaaaatttgagatagtgattca

SEQ ID NO: 610 - DNA, 100 bp, Homo sapiens
  source 1..100: mol_type = other DNA
gaaagaaaaaaaggaatgattatcatgaattctgtttattagaattctgtttattaaagagttaaagatatgttttatttttttatctttattatcatta

SEQ ID NO: 611 - DNA, 100 bp, Homo sapiens
  source 1..100: mol_type = other DNA
aattctaatgttggtcccttaggatcagcagggggggaccgggaatctgtaactgcaaccaccccaccgagaggattacaggaacccagtcgagagctgg

SEQ ID NO: 612 - DNA, 100 bp, Homo sapiens
  source 1..100: mol_type = other DNA
ttcccaacaatgaggttcatttaaaaagtcgtgaggggggaggggggccaaagaaagaaatagatcaaagagcgggagagtcgagaaaagaaggaagaaa

SEQ ID NO: 613 - DNA, 100 bp, Homo sapiens
  source 1..100: mol_type = other DNA
tgttggggagcgctggcagccgggctggcaagtggagtttgggaatgtgcagggagggaaggaagctgaaaaattcaaactttttaaatgctactcttca

SEQ ID NO: 614 - DNA, 100 bp, Homo sapiens
  source 1..100: mol_type = other DNA
gctcctcggcgtccctgcaccccaaccctgcagccctggggcgttggcagctgcaccaacaggagcagcaagctgggaaaacagagcaacatgacccgac

SEQ ID NO: 615 - DNA, 100 bp, Homo sapiens
  source 1..100: mol_type = other DNA
gtgttaagagaaggcaaaacacttcagcaattaaaaagtagcccagcagcttcaccctttcaaattgggagggggaggttggaaagaaatttaacaacat

SEQ ID NO: 616 - DNA, 100 bp, Homo sapiens
  source 1..100: mol_type = other DNA
ccatagacttttgctatgtacatttaaaccgcagtcctggaacattccgagtttaaaacttgctttttcaacactggctgacaagcaacatgttttaagg

SEQ ID NO: 617 - DNA, 100 bp, Homo sapiens
  source 1..100: mol_type = other DNA
agccccccattaaatccttactcgcgggactctcgagttcaagccagcattttgtcgccacctccccccccaaccccgcccgcaatcgatgagccgcaat

SEQ ID NO: 618 - DNA, 100 bp, Homo sapiens
  source 1..100: mol_type = other DNA
gcctcggcaacacaggtaagcgggtcaacctgaatgcctctttcaccccaaagtttgctgcacgatcggctatcgcgggaagaagcccaacggagctagg

SEQ ID NO: 619 - DNA, 100 bp, Homo sapiens
  source 1..100: mol_type = other DNA
gcggactcaagccccactgcaaacttgttctgcaacatctttttgaatcacaacttggcctttcttcctcgcatatccccagctccccccaaagagtgga

SEQ ID NO: 620 - DNA, 100 bp, Homo sapiens
  source 1..100: mol_type = other DNA
ggaaaacattgtcccgagactcacttccccgagggacctcccactcccaaccccacgggtgggtaatgccgctggacagacctagggcgcagactgggaa

SEQ ID NO: 621 - DNA, 100 bp, Homo sapiens
  source 1..100: mol_type = other DNA
cccgatcagaccagcaaacctgggatccagcagcacgttacgtaaaacaggatcgcccaaaacttgtcccaatcccagccctccccccgaagcccccggg

SEQ ID NO: 622 - DNA, 100 bp, Homo sapiens
  source 1..100: mol_type = other DNA
ctgccctgccaggcaaacttcgcccctcaaaaccctggcctccagattcacatgtaatccccgccagcaactgttgaaactcaaagggtgggaaggacgg

SEQ ID NO: 623 - DNA, 100 bp, Homo sapiens
  source 1..100: mol_type = other DNA
ggccaaattccttcaaacttgggagaaatgccggaggagaaaagaatcatctcgctgcaccactttccccattgccttccaagacccaaacttttggggg

SEQ ID NO: 624 - DNA, 100 bp, Homo sapiens
  source 1..100: mol_type = other DNA
ttctttcttaaggcaaaagaaaaagactttttgaaaagcaaatgctccgcccccctttaccttgcataaaacttcgctcaagtcgaagatggtggcagac

SEQ ID NO: 625 - DNA, 100 bp, Homo sapiens
  source 1..100: mol_type = other DNA
acgagggtggtggtcatcctgtgcgttcgcgcgagccaggggcgaggatctggtgtgtcgcgaaggtcccggtgcggggaaggcgcagcctctcctgtct

SEQ ID NO: 626 - DNA, 100 bp, Homo sapiens
  source 1..100: mol_type = other DNA
ttatttttttatattaagatttattctaaattttgattcttctaaatatagtatatatttagtatatatataatgcacctctcttacctaatgatcattt

SEQ ID NO: 627 - DNA, 100 bp, Homo sapiens
  source 1..100: mol_type = other DNA
ctaaataatcataacaacatcgagtaaaactatgtaataacacatattattattaagataagtataagaaatataataataaattgtccctgttctaaaa

SEQ ID NO: 628 - DNA, 100 bp, Homo sapiens
  source 1..100: mol_type = other DNA
ggtaattatataatgctgaatgtgtcagaggcattcgaaccagagtgactccattttgagtgagggctaggaaaatgaggctgagacttgctgggatgca

SEQ ID NO: 629 - DNA, 100 bp, Homo sapiens
  source 1..100: mol_type = other DNA
tttaatttttatgctttcttcagtgtatgtttggagagagtttgaacattttttgactctttttcattgagtaaatccaaatacttgtaaaagacttatc

SEQ ID NO: 630 - DNA, 100 bp, Homo sapiens
  source 1..100: mol_type = other DNA
tatttctttaacaaaaacttaacatggattaaggacccatcttaaggcatcacacattaaaaaagtcaatattgattcaataccggcgcttatactacga

SEQ ID NO: 631 - DNA, 100 bp, Homo sapiens
  source 1..100: mol_type = other DNA
catcacttgttaaatttgttttctaaataaagcccagaggtagtggaaaatacttcacactctaggccagtgtttgctatgcctggttgaccctaaactg

SEQ ID NO: 632 - DNA, 100 bp, Homo sapiens
  source 1..100: mol_type = other DNA
ttgagggttctttttaaaaatacagatttctgggacccacctgagatgattccgataatcggccatatggatgagtcacttagagatacccatttttaag

SEQ ID NO: 633 - DNA, 100 bp, Homo sapiens
  source 1..100: mol_type = other DNA
gattaggaccccgaagcccagaaaatgcctgctgtagtcaacattatagtcacactccacaggcactgggtccacccctttgaccgacattcctttgcgg

SEQ ID NO: 634 - DNA, 100 bp, Homo sapiens
  source 1..100: mol_type = other DNA
ttttcccacccttcttccctgcctggagaactcctattcatcctccagagcccggctcaaagtggcttcatctgtggggatcctccctgccccatagtga

SEQ ID NO: 635 - DNA, 100 bp, Homo sapiens
  source 1..100: mol_type = other DNA
gtgctccttgagtcctcgcccttcctagggcatcccaagctcccaggggctgcccctgctgcctcgccatccgctccaaagctggctgtacctcgatggt

SEQ ID NO: 636 - DNA, 100 bp, Homo sapiens
  source 1..100: mol_type = other DNA
taagggcagccaggcgtgctgcttctcgtccaaatacacgaacttctcccaggcccacaggcggtccgggtggtcggtgactgcctccccgagtgtcggg

SEQ ID NO: 637 - DNA, 100 bp, Homo sapiens
  source 1..100: mol_type = other DNA
aggaatcagatttcaaaatgaatatgtataagaaaagaaccggggatcagtgatcaggaacagggatccatgatctggtccagggctcagcggtcaggaa

SEQ ID NO: 638 - DNA, 100 bp, Homo sapiens
  source 1..100: mol_type = other DNA
ccctggcctggagtcccaagtccccagcccatcctgcccctggagcccagtttagcttggtcttgaagtctgctctaggtacccccaaaatcacagtatc

SEQ ID NO: 639 - DNA, 100 bp, Homo sapiens
  source 1..100: mol_type = other DNA
cagccccgctctgcccaccgggacagccaagttcagctgagactggcctaccgggggagtcgccctctgaagttcactctaagccagcctggttcagcct

SEQ ID NO: 640 - DNA, 100 bp, Homo sapiens
  source 1..100: mol_type = other DNA
ggcccaggtcagcccaggacctccccttgcaggcagcaaactcttatttcagtccagccagctcaaccagcttgcttctgactcagctcctcttagccag

SEQ ID NO: 641 - DNA, 100 bp, Homo sapiens
  source 1..100: mol_type = other DNA
ttagctcagcaaagctggacctaaagtagccacctcaccccagcttcatccagatgaatacagtccagatcagcttagtcagttaagcctagcctagcta

SEQ ID NO: 642 - DNA, 100 bp, Homo sapiens
  source 1..100: mol_type = other DNA
gttaaatccagttacgaccagctcaactaatcctgctcaggcctgctcagcccagcccagctgaacccagtttagccgaggccaggccagcccagctgaa

SEQ ID NO: 643 - DNA, 100 bp, Homo sapiens
  source 1..100: mol_type = other DNA
tacagttgcccagtctagctcagcccagtccagcactgcccagtttagctgagctcagcctggcccagcccagctcatatcagcccatctcagctgaacc

SEQ ID NO: 644 - DNA, 100 bp, Homo sapiens
  source 1..100: mol_type = other DNA
agtttgacccagtctaacccaaccccgctcagctgaacccagcccagcccagcccagcccagccaaacccagtttagcctagctcagctcagcccatttc

SEQ ID NO: 645 - DNA, 100 bp, Homo sapiens
  source 1..100: mol_type = other DNA
cctgtcctaggggtggcaggcagtctgcacccagcctagccctgcccagcgtggggtctctgaccttcttggtcttgggcccagccaagattcccagccc

SEQ ID NO: 646 - DNA, 100 bp, Homo sapiens
  source 1..100: mol_type = other DNA
ttctagctttcctgtgtccccatgcagggaagggatgcctagagtccacgcagtgaccaagaagcttggttgatgctgtgagggtggcccaggagtcccc

SEQ ID NO: 647 - DNA, 100 bp, Homo sapiens
  source 1..100: mol_type = other DNA
cacctgctgtccttggtcctggctgagaggagggccctacggccagctctgctgaccctgccctgggctctggtgatgctgccggcctggacaagcccct

SEQ ID NO: 648 - DNA, 100 bp, Homo sapiens
  source 1..100: mol_type = other DNA
gagctcaggtcggtcgtgcccatcctggcatcaccccacagccggttctgccgcatcccgtcatgttcctcgtgctcccagcccggtcgtcctggaggcc

SEQ ID NO: 649 - DNA, 100 bp, Homo sapiens
  source 1..100: mol_type = other DNA
tgagcatgagtggggcgggcagaggcctccgggtgaggagacagatggggcctgccttgctgccctgggctggggctgcacagccggggtgcgtccaggc

SEQ ID NO: 650 - DNA, 100 bp, Homo sapiens
  source 1..100: mol_type = other DNA
aggagggctgagcctggcttccagcagacaccctccctccctgagctggcctctcaccaactgtcttgtccaccttggtgttgctgggcttgtgatctac

SEQ ID NO: 651 - DNA, 100 bp, Homo sapiens
  source 1..100: mol_type = other DNA
accaactgtcttgtccaccttggtgttgctgggcttgtgatctacgttgcaggtgtaggtctgggtgccgaagttgctggagggcacggtcaccacgctg

SEQ ID NO: 652 - DNA, 100 bp, Homo sapiens
  source 1..100: mol_type = other DNA
ggactgtaggacagccgggaaggtgtgcacgccgctggtcagagcgcctgagttccacgacaccgtcaccggttcggggaagtagtccttgaccaggcag

SEQ ID NO: 653 - DNA, 100 bp, Homo sapiens
  source 1..100: mol_type = other DNA
tgctacactgccctgcaccacctccactcagcttcattgtgctggtggccctggctcctggcagcccatcttgctccttctggggcgccagcctcagagg

SEQ ID NO: 654 - DNA, 100 bp, Homo sapiens
  source 1..100: mol_type = other DNA
ccttcctgcctagggtccgctggggccagccctgggaccctcctggtctcaagcacacattccccctgcagccacacctgcccctgcctgagagctcagc

SEQ ID NO: 655 - DNA, 100 bp, Homo sapiens
  source 1..100: mol_type = other DNA
cccgagccctggaatgccttcccttctccatcccagctcacccttgccaactgctcagtgggatgggctcacactcccttcctggcaccaggaggctgca

SEQ ID NO: 656 - DNA, 100 bp, Homo sapiens
  source 1..100: mol_type = other DNA
ctgcactttcaccagccctcagctgtctgctgccagcaactacccagctcctgccaaaatctaggagctgagtgatgcctcccaccggccctgctcacct

SEQ ID NO: 657 - DNA, 100 bp, Homo sapiens
  source 1..100: mol_type = other DNA
gtggttgccttgccctgagctctagtgcctgtcccctgctcgtcctgcctcccaccggccctgctcacctgtggctgctctgctctgattccctgaggct

SEQ ID NO: 658 - DNA, 100 bp, Homo sapiens
  source 1..100: mol_type = other DNA
aagcctcagtcctgctcaccttctgatgctctcctctgtcccctgagctccaggggctgtcccctgctcgtcctgcctcctacctgcccctgcttacctg

SEQ ID NO: 659 - DNA, 100 bp, Homo sapiens
  source 1..100: mol_type = other DNA
agggtgctctgccctggtgctctgagctccaggggctgtcccctgctcctcctgcttcctaccagcccctgctcacctgtggctgctctgccctggtccc

SEQ ID NO: 660 - DNA, 100 bp, Homo sapiens
  source 1..100: mol_type = other DNA
ctctgccctggtcccctgagctccaggggcttccccctgctcttcctgcccccaccagcccctgttcaccttcagatgccctcccctggtcccctgaagt

SEQ ID NO: 661 - DNA, 100 bp, Homo sapiens
  source 1..100: mol_type = other DNA
cccagagctgccccctgttcctcctgcctcccaccagcccgtgctcacctgccgctgctctgccctggtcccgagttccaggggctgcaccctgttcgcc

SEQ ID NO: 662 - DNA, 100 bp, Homo sapiens
  source 1..100: mol_type = other DNA
cacctcccactagccatgctcagctcttgatgctctgtcctggtcccctgagctccaggagctgtcccctactcgtcctgccacccaccagcccctgctc

SEQ ID NO: 663 - DNA, 100 bp, Homo sapiens
  source 1..100: mol_type = other DNA
acctgaggcacctgaggctgctctgccctggtcccctgagctccagggtcttccccctgctcatcctgcctcccacctgcccttgttcaccttcagttgc

SEQ ID NO: 664 - DNA, 100 bp, Homo sapiens
  source 1..100: mol_type = other DNA
tctgccctggtctgctgagctccaggaggtgccccctgctccttctgcccccacctgccctgctcacctgtggctgctcggtcctggtaccctgaactcc

SEQ ID NO: 665 - DNA, 100 bp, Homo sapiens
  source 1..100: mol_type = other DNA
gccccctgctccttctgcccccacctgccctgctcacctgtggctgctcggtcctggtaccctgaactccaatgcctgccccctgctcactctgccctcc

SEQ ID NO: 666 - DNA, 100 bp, Homo sapiens
  source 1..100: mol_type = other DNA
ctcaacccgggcagcaatgtcactcaggtcactgttgcccccctgcctgtcctggcaccctctgtccaggtttgggctgtttttctggcctcatttttgt

SEQ ID NO: 667 - DNA, 100 bp, Homo sapiens
  source 1..100: mol_type = other DNA
tgtccagtcaggtctccccaacagagccccttgcccttgcccatgtgcccctcctgggtgagctcccagatcctcccgtccctgcactgctcctgctctg

SEQ ID NO: 668 - DNA, 100 bp, Homo sapiens
  source 1..100: mol_type = other DNA
gaagcctctccagaacctcagctcctcagtggcctctgctctgctgggtcagctccctgaacgcacggagcctcacccctcccctcgccccaggcctgct

SEQ ID NO: 669 - DNA, 100 bp, Homo sapiens
  source 1..100: mol_type = other DNA
gcactctgggcctttctgggcctccctggactcttccctcctcccatctgtgcactcagcacagctctcccctccactccgctgctgaccacagccctgc

SEQ ID NO: 670 - DNA, 100 bp, Homo sapiens
  source 1..100: mol_type = other DNA
cctttctgggcctccctggactcttccctcctcccatctgtgcactcagcacagctctcccctccactccgctgctgaccacagccctgctccccgccag

SEQ ID NO: 671 - DNA, 100 bp, Homo sapiens
  source 1..100: mol_type = other DNA
cccacggccagcactgctgaccctgccctgggctccagtgatgctgctggcctggacaagcccctccgttcacctggggcctctcctcctccctcgttct

SEQ ID NO: 672 - DNA, 100 bp, Homo sapiens
  source 1..100: mol_type = other DNA
actgcctcctcagctcaggtgggtcctgcccatgctggcatcaccccacggccggctctgccgcatcccgtcaggttcctcgtgctcccagcctggtcgt

SEQ ID NO: 673 - DNA, 100 bp, Homo sapiens
  source 1..100: mol_type = other DNA
catggaggcctcagtcagcctctggtgtgtcctgccctgttggcttggaagcccctgcccacggtccccgtcatcttgcactgggtgggcgttggtgcct

SEQ ID NO: 674 - DNA, 100 bp, Homo sapiens
  source 1..100: mol_type = other DNA
agctcagcccagcctagtccagcccagcccagcacaggtcagcccagcttagcttagcccaggtcagtccagctcagctcagtccacttaagctcaccca

SEQ ID NO: 675 - DNA, 100 bp, Homo sapiens
  source 1..100: mol_type = other DNA
ggtcagctccgtccagctcagcccagcctagcccagcttagcccagcccagcccaacacaggtcagcccagctcagcctagcccagcccagctcagcaca

SEQ ID NO: 676 - DNA, 100 bp, Homo sapiens
  source 1..100: mol_type = other DNA
ggtcagaccagctcagtacagctcaggtcagcccagaccagtccaacccagcccagcgcagtccaacccagcccagctcagctcatccaagcctagctca

SEQ ID NO: 677 - DNA, 100 bp, Homo sapiens
  source 1..100: mol_type = other DNA
gctcagcccagcccaggtcagcctagcccagccgaacccagctcagcccaggtcaacccaattcagctcagctcagcccaggtcaacccaaccaagctca

SEQ ID NO: 678 - DNA, 100 bp, Homo sapiens
  source 1..100: mol_type = other DNA
gctcagcctagcccagtccagctcagcccagctcagctcagcccagtccagctcaatccacctaagctcacccagctcagcccagtctggctcagcttag

SEQ ID NO: 679 - DNA, 100 bp, Homo sapiens
  source 1..100: mol_type = other DNA
gtcagcccagcccagcctagcccagatcagtccagcttagcccagcccaggtcagcccagcccaggtcagcccagctcagctcagcccagcccagctcag

SEQ ID NO: 680 - DNA, 100 bp, Homo sapiens
  source 1..100: mol_type = other DNA
cccagcccagctcagcgcagcccagcctagctcaccccagccaggtccagcttagcccagctcagcccagcccaactcagctcagcccagctcagcccaa

SEQ ID NO: 681 - DNA, 100 bp, Homo sapiens
  source 1..100: mol_type = other DNA
tctgagctccaggggctgcccacctgctcctcctgcttcccaccggccctgctcacctgcagctgctctgccctggctccctgaggctgagcctcagtcc

SEQ ID NO: 682 - DNA, 100 bp, Homo sapiens
  source 1..100: mol_type = other DNA
tgctcaccttctgatgctctccccttgtcccctgagctccaggggctgacccctgatctttctgcttcctacctgcccctgctcacctgtggctgctctg

SEQ ID NO: 683 - DNA, 100 bp, Homo sapiens
  source 1..100: mol_type = other DNA
ccctgatcccctgagctccaggagctgcctcctgctcttcctgcctcccacctgcccctgctcacctgcagatctgccctggctctctgaggtccagggg

SEQ ID NO: 684 - DNA, 100 bp, Homo sapiens
  source 1..100: mol_type = other DNA
ctgccccctgctcgcccacctcccaccagccatgctgacgttgtgatgctctgccctggtctcctgaggtccaggggctgtcccctgcttattctgcctc

SEQ ID NO: 685 - DNA, 100 bp, Homo sapiens
  source 1..100: mol_type = other DNA
ccacctgccccttctcacctgaggctcttctgccctggtgctctgagctccaaaagctgcccacttgctcctcctgcttcctaccagcccctgctctcct

SEQ ID NO: 686 - DNA, 100 bp, Homo sapiens
  source 1..100: mol_type = other DNA
gtggatgatctgccctggctctctgagctccaggggctgcccacctgctccccatgcttcccacctgcccctgctgacctgcggctgctctgccttggct

SEQ ID NO: 687 - DNA, 100 bp, Homo sapiens
  source 1..100: mol_type = other DNA
ccctgagctccaggagcttccccctgctcatcctgccccccactggcccctgttcaccttcagatgccctccctggtcccctgaagtccaggagctgccc

SEQ ID NO: 688 - DNA, 100 bp, Homo sapiens
  source 1..100: mol_type = other DNA
cctgttcctcccgcctcccaccagcccgtgctcacctgcggctgctctgccctggtcccctgagttccaggggctgccccctgctcgcccacctcccact

SEQ ID NO: 689 - DNA, 100 bp, Homo sapiens
  source 1..100: mol_type = other DNA
agccatgctcacctcctgatgctctgtcctggtcccctgagctccaggggctgccccctgcttgcccatctcccactagccatgctcaccttctgatgct

SEQ ID NO: 690 - DNA, 100 bp, Homo sapiens
  source 1..100: mol_type = other DNA
ctgccctggtcccctgagctccagggtcttccccctgctcatcctgccgcccaccagcccctgctcacctgaggctgctctgccctggtcccctgagctc

SEQ ID NO: 691 - DNA, 100 bp, Homo sapiens
  source 1..100: mol_type = other DNA
cccctgagctccagggtcttccccctgctcatcctgccgcccaccagcccctgctcacctgaggctgctctgccctggtcccctgagctccaggaggtgc

SEQ ID NO: 692 - DNA, 100 bp, Homo sapiens
  source 1..100: mol_type = other DNA
ttctgcccccacctgccctgctcacctgtggctgcttggtcctggtccctgagctccaatgcctgctccctgctcactctgccctccctcaacccgggca

SEQ ID NO: 693 - DNA, 100 bp, Homo sapiens
  source 1..100: mol_type = other DNA
gcaatgtcactcaggtcactgttgcccccctgcctgtcctggcaccctctgtccaggtttgggctgtttttctgccctcatttttgattttgcagcactt

SEQ ID NO: 694 - DNA, 100 bp, Homo sapiens
  source 1..100: mol_type = other DNA
cctctgtccaggtttgggctgtttttctgccctcatttttgattttgcagcacttggcgtgttccctatgctgtggagcagccccagtgtccagtcaggt

SEQ ID NO: 695 - DNA, 100 bp, Homo sapiens
  source 1..100: mol_type = other DNA
agtgtccagtcaggtctccccaacagagccccttgcccttgcccatgtgcccctcctgaatgagctcccggatcctcctgtccctgcactgctcctgctc

SEQ ID NO: 696 - DNA, 100 bp, Homo sapiens
  source 1..100: mol_type = other DNA
tggaagcctctctggaacctcagctcctcagtggcctctgctctgctgggtcagttccctgaacgcacggagcctcagcccttcccctcgccccaggcct

SEQ ID NO: 697 - DNA, 100 bp, Homo sapiens
  source 1..100: mol_type = other DNA
gctgcactctgggcctttctgggcctccctggactcttcccttctcccgcccgtgcactcagcacagctctcccctcctctccactgctgaccacagccc

SEQ ID NO: 698 - DNA, 100 bp, Homo sapiens
  source 1..100: mol_type = other DNA
tgctccccgccagcaggtgccccaaccccatcagctggctctgagcccagcccctgtgcctcccctgtccctgcctctgcctctgggctccttggcttcc

SEQ ID NO: 699 - DNA, 100 bp, Homo sapiens
  source 1..100: mol_type = other DNA
acctgctgtccttggtcctggctgagaggagggccccacggccagcactgctgaccctgccctgggctccggtgatgctgccggcctggacaagcccctc

SEQ ID NO: 700 - DNA, 100 bp, Homo sapiens
  source 1..100: mol_type = other DNA
cgttcacctggggcctctcctcctccctcgctctgctgcctcctgagctcaggtcggtcgtgcccatcctggcatcaccccacggccggctctgccgcat

SEQ ID NO: 701 - DNA, 100 bp, Homo sapiens
  source 1..100: mol_type = other DNA
ccagtcatgttcctcgtgctcccagcccggtcgtcctggaggcctcagtcagcctctggtgtgtcctgccctgttggcttggaagcccctgcccacggtc

SEQ ID NO: 702 - DNA, 100 bp, Homo sapiens
  source 1..100: mol_type = other DNA
cccgtcgtctcgcactgggtgggcatcggtgcctgaaggctgcccacctcccccgtgctggctccgcttgggcctccatgtggggccggcctcgacccca

SEQ ID NO: 703 - DNA, 100 bp, Homo sapiens
  source 1..100: mol_type = other DNA
cactgcactttcaccagccctcagctgtctgctgccggcaactacccagctcctgccaaagtctaggagctgcgtgctgcctcccaccgtccctgctcac

SEQ ID NO: 704 - DNA, 100 bp, Homo sapiens
  source 1..100: mol_type = other DNA
ctgtggctgctctgccctggtgctctgagctccaggagatgccccctgctcctcctgccccccacctgcccctgctcacctgcagcggctctgccctggt

SEQ ID NO: 705 - DNA, 100 bp, Homo sapiens
  source 1..100: mol_type = other DNA
gagctccaagagctgccccctgctcctcctgtcccctgaccctgctcctgtttgcctatggctgctctgcccttgtcccctgagctccaggagctgcccc

SEQ ID NO: 706 - DNA, 100 bp, Homo sapiens
  source 1..100: mol_type = other DNA
tgctcattctgccgcccacctgcccctgttcacctgtggctgctcttccctggtcctctgagctccatgagctgccccttgctcctcctgctttccacca

SEQ ID NO: 707 - DNA, 100 bp, Homo sapiens
  source 1..100: mol_type = other DNA
gcccctgctcacctaccgatgatcttccccggctctctgagctccaggggctgcccacctgctacccctgcttcccaccagccctgcttacctgcagctg

SEQ ID NO: 708 - DNA, 100 bp, Homo sapiens
  source 1..100: mol_type = other DNA
ctctgccctggctggcagagctgcagaagctgccccctgctctgcaacctcccaccggcccttctcatcttctgatgttctcccctgttccctgagctcc

SEQ ID NO: 709 - DNA, 100 bp, Homo sapiens
  source 1..100: mol_type = other DNA
aggagctgccccctactcgttctacctcccaccaacccgtgctcacctgcgactgctctgccctggtcccctgagctccaggggctgccccctgctcgcc

SEQ ID NO: 710 - DNA, 100 bp, Homo sapiens
  source 1..100: mol_type = other DNA
tgccctgatcccctgagctccaggactgccccctgctcgtcctgcccctcacctgcccctgctcacctgaggctgctctgccctggtcccctgagctaaa

SEQ ID NO: 711 - DNA, 100 bp, Homo sapiens
  source 1..100: mol_type = other DNA
ggggctgccccttactcatcctgcctcccaccagcccctgctcaccttctgatgccctcccctggtcccctgagctccaggggctgccccctgctcgtcc

SEQ ID NO: 712 - DNA, 100 bp, Homo sapiens
  source 1..100: mol_type = other DNA
gggctgccccctgctcgtcctgcctcccaccagcccctgctcacctgcagctacactgccctggttccctgagctccaggagctgccacctgcttgtcct

SEQ ID NO: 713 - DNA, 100 bp, Homo sapiens
  source 1..100: mol_type = other DNA
gccttccaccagcccctgctcacctgcagctacactgccctggttccctgagctccgggagctgccgcctgcttgtcctgcctcccaccagcccctgctc

SEQ ID NO: 714 - DNA, 100 bp, Homo sapiens
  source 1..100: mol_type = other DNA
acctgtggctacactgccctggtgccctgagctccaggagctgccccctgcttgcccatcttccactgagccctgctcacctgcaactgctctgccctgg

SEQ ID NO: 715 - DNA, 100 bp, Homo sapiens
  source 1..100: mol_type = other DNA
ctctatgagctccaggggctgccccctgctggtcctgcctcccacctgccctgcgcacctgtggctgcctcctcacctgtggctgctctgccctggtccc

SEQ ID NO: 716 - DNA, 100 bp, Homo sapiens
  source 1..100: mol_type = other DNA
ctgagctccagggtcttcctcctgctcatcctgcccctccaccggctcctgttcaccttcagatgctctcccgtggtcccctgagctccaggagctgccc

SEQ ID NO: 717 - DNA, 100 bp, Homo sapiens
  source 1..100: mol_type = other DNA
cctgttcttcctgcctcccacctgccctgtgcacctgtggctgcttggtcctggtcccctgaactccaatgcctgccccctgctcactctgccctccctc

SEQ ID NO: 718 - DNA, 100 bp, Homo sapiens
  source 1..100: mol_type = other DNA
aacctggggcagcaacgtcactcggtccactgttgcccccctgcctgtcctggcaccctctgtccaggtttaggctgtttttcttgcctcatttttgttt

SEQ ID NO: 719 - DNA, 100 bp, Homo sapiens
  source 1..100: mol_type = other DNA
tggcaccctctgtccaggtttaggctgtttttcttgcctcatttttgtttttgcagcacttggcgtgttccctatgctgtggagcagccccagtgtccag

SEQ ID NO: 720 - DNA, 100 bp, Homo sapiens
  source 1..100: mol_type = other DNA
tccagtcaggtctccccaacagagccccttgcccttgcccatgtgcccctcctggatgagctcccggatcctcccgtccctgcactgctcctgctctgga

SEQ ID NO: 721 - DNA, 100 bp, Homo sapiens
  source 1..100: mol_type = other DNA
agcctctccagaacctcagctcctcagtggcctctgctctgctgggtcagttccctgaacgcacggagcctcagcccctcccctcgccccaggcctgctg

SEQ ID NO: 722 - DNA, 100 bp, Homo sapiens
  source 1..100: mol_type = other DNA
cactctgggcctttctgggcctccctggactcttccctcctcccgcccgtgcactcagcacagctctcccctcctctccgctgctgaccacagccctgct

SEQ ID NO: 723 - DNA, 100 bp, Homo sapiens
  source 1..100: mol_type = other DNA
gaccacagccctgctcccggccagcaggtgccccaaccccatcagctggctctgagcccagcccctgtgcctcccctgtccctgcctctgcctctgggct

SEQ ID NO: 724 - DNA, 100 bp, Homo sapiens
  source 1..100: mol_type = other DNA
gctctgctcccagctcacctgctgtccttggtcctggctgagaggagggccctacggccagctctgctgaccctgccctgggctccggtgatgctgccgg

SEQ ID NO: 725 - DNA, 100 bp, Homo sapiens
  source 1..100: mol_type = other DNA
cctggacaagcccctcggttcacctggggcctctcctcctccctctctctgctgcctcctgagctcaggtcggtcatgcccatcctggcatcaccccatg

SEQ ID NO: 726 - DNA, 100 bp, Homo sapiens
  source 1..100: mol_type = other DNA
gctggctctgccccatcccgtcatgttcctcacactcccagcccggtcgtcctggaggcctcagtcagcctctggtgtgtcctgccctgttggcttggaa

SEQ ID NO: 727 - DNA, 100 bp, Homo sapiens
  source 1..100: mol_type = other DNA
gggtagagcccacctcgtggcctgcaagccagccagcccctgccggtcgagaaggaagcctgtgtgagagcacacaactggaggccgggcggggaagaga

SEQ ID NO: 728 - DNA, 100 bp, Homo sapiens
  source 1..100: mol_type = other DNA
aacacgtgccaacaggccacgcaggccaggaccccagacccggaggcagcgcccctttgagttcctctctctggtctccgatgttcttctgttgggatca

SEQ ID NO: 729 - DNA, 100 bp, Homo sapiens
  source 1..100: mol_type = other DNA
tttcacctacaggcaacagagacagtgtgaaatgctttccctgtggtcgggaagggagccggggcagagatgacccagtggggtggtgtgggggcctccg

SEQ ID NO: 730 - DNA, 100 bp, Homo sapiens
  source 1..100: mol_type = other DNA
ctttgcacaccacgtgttcgtctgtgccctgcatgacgtccttggaaggcagcagcacctgtgaggtggctgcgtacttgccccctctcaggactgatgg

SEQ ID NO: 731 - DNA, 100 bp, Homo sapiens
  source 1..100: mol_type = other DNA
gaagccccgggtgctgctgatgtcagagttgttcttgtatttccaggagaaagtgatggagtcgggaaggaagtcctgtgcgaggcagccaacggccacg

SEQ ID NO: 732 - DNA, 100 bp, Homo sapiens
  source 1..100: mol_type = other DNA
ctgctcgtatccgacggggaattctcacaggagacgagggggaaaagggttggggcggatgcactccctgaggacccgcaggacaaaagagaaagggagg

SEQ ID NO: 733 - DNA, 100 bp, Homo sapiens
  source 1..100: mol_type = other DNA
actccagctaccctgaagtctccccaggcagacaacccaggcctgggagtgagtatagggagggtgggtgtgatggggaacgcagtgtagactcagctga

SEQ ID NO: 734 - DNA, 100 bp, Homo sapiens
  source 1..100: mol_type = other DNA
ggctatccatctatgtccaacaagatcatgaagattggcccagtgccatgtcctccagttcatcccagcccaggccagctcaatccagttcatcccagcc

SEQ ID NO: 735 - DNA, 100 bp, Homo sapiens
  source 1..100: mol_type = other DNA
caggccagctcaatccagcccagcccaccccaccccagctcagcaaagccaagctcagctcagcccaactcagatgagctcagaccagctcagcccagcc

SEQ ID NO: 736 - DNA, 100 bp, Homo sapiens
  source 1..100: mol_type = other DNA
cagctcagctcagcccaacccagcccagctcgctcaaccttgctcggctcagcttagcccagcccagcccagctcaatccagcctggctcagcccagccc

SEQ ID NO: 737 - DNA, 100 bp, Homo sapiens
  source 1..100: mol_type = other DNA
agcccagtttggctcaacccagcttggctcagcccaggtcagcctggctcaactcagcccagcccagcccagctctgctcaacccagctctgctcaactc

SEQ ID NO: 738 - DNA, 100 bp, Homo sapiens
  source 1..100: mol_type = other DNA
agcccagctcatcccagctcagcccagcccagcctagcttagctcaacccagctcagctcagttcagctcagccctgctcagcacagcacagcagagccc

SEQ ID NO: 739 - DNA, 100 bp, Homo sapiens
  source 1..100: mol_type = other DNA
agcccggatcggctcaacccagcttagctcagcccaggtcagcccagcttaactcagcccaggtcagcccagcttaactcagcccagcccagcccagctc

SEQ ID NO: 740 - DNA, 100 bp, Homo sapiens
  source 1..100: mol_type = other DNA
tcagcccagttcagcccagctcagcccagcccagcctagcttggctcaacacagctcagctcagccagcccagaccagctcagctcagcccagtccagct

SEQ ID NO: 741 - DNA, 100 bp, Homo sapiens
  source 1..100: mol_type = other DNA
caacccagcccagcccaacccagctcggcttaacccagctcggctcagcccagatcagcctggctcaactcagcccagcccagctcaacccagcccagtt

SEQ ID NO: 742 - DNA, 100 bp, Homo sapiens
  source 1..100: mol_type = other DNA
cagctcagctgagcccagcccagcccagtccggctcagctcagccccgccccactcagcccagctcagctcagcccagctcagcccagctcagcttagcc

SEQ ID NO: 743 - DNA, 100 bp, Homo sapiens
  source 1..100: mol_type = other DNA
cagcccagatcatcccagctcagctcagctcagctcggcttagcccagctcaacctggcccagcctggtccaggtcagcccagcctggaccacccagccc

SEQ ID NO: 744 - DNA, 100 bp, Homo sapiens
  source 1..100: mol_type = other DNA
agctcagctcagcccagctcatcctggttcagctcagctcaacccggctcagcccaggtctgctcaacccagcccaaatcagctcagcccagcccaggtc

SEQ ID NO: 745 - DNA, 100 bp, Homo sapiens
  source 1..100: mol_type = other DNA
atcccagctcagcccagcacagcctacttcagctcagctcagctcagcctaggtcagctcagttgaggtcagctcaactcagcccaatccagcctggctc

SEQ ID NO: 746 - DNA, 100 bp, Homo sapiens
  source 1..100: mol_type = other DNA
agcccagctcaccctagctcagcttagctcagcccaactcaacccagcccagccttgcccaacccagctcagctcagcccagcccaggttagcccagccc

SEQ ID NO: 747 - DNA, 100 bp, Homo sapiens
  source 1..100: mol_type = other DNA
agcctcggcttagctctgctcagctcggccctgctcgcctcagcccgttcagcccagttcagctcagctcagctcagcccagctcagcccagccctggtt

SEQ ID NO: 748 - DNA, 100 bp, Homo sapiens
  source 1..100: mol_type = other DNA
agctcagcccagctaagctcagctcggcttggctctgctgagcttggcccagcttggcttagcctgatacaacctgctcagcccagttcagctcggctca

SEQ ID NO: 749 - DNA, 100 bp, Homo sapiens
  source 1..100: mol_type = other DNA
gcccagcgtagctcagctcagctgagcccagcccaggttagctcagccccagtccaggtcagctcaactcagcccaaaccagcctggctcggcccagctc

SEQ ID NO: 750 - DNA, 100 bp, Homo sapiens
  source 1..100: mol_type = other DNA
accctagttcagcttagctcagcccagcccagccctgcccaacccagctcagctcagcccagcccaggttagcccagcccagcctcggcttagctctgct

SEQ ID NO: 751 - DNA, 100 bp, Homo sapiens
  source 1..100: mol_type = other DNA
agcccagcccaggttagcccagcccagcctcggcttagctctgctcagctcggcccagcccaggttagcccagcccagcctcggcttagctctgctcagc

SEQ ID NO: 752 - DNA, 100 bp, Homo sapiens
  source 1..100: mol_type = other DNA
tcggccctgctcgcctcagcccgttcagcccagttcagctcagctcagctcagcccagctcagcccagccctggttagctcagcccagctaagctcagct

SEQ ID NO: 753 - DNA, 100 bp, Homo sapiens
  source 1..100: mol_type = other DNA
cggctcagctctgctgagctcggcccagcttggctcagcccgacacagcctgctcagcccagttcagctcggctcagcccagcccagcccagcgtagctc

SEQ ID NO: 754 - DNA, 100 bp, Homo sapiens
  source 1..100: mol_type = other DNA
agctgagcccagcccaggttagctcagccccagcccaggttagctcagcccagctcagctctgcccaggttagctcagccccagtccaggttagctcagc

SEQ ID NO: 755 - DNA, 100 bp, Homo sapiens
  source 1..100: mol_type = other DNA
ccagctcagctctgcccaggttagctcagccccagtccaggttagctcagcccagctcagccttgcccaggttagctcagcccagctaagctcaacttgg

SEQ ID NO: 756 - DNA, 100 bp, Homo sapiens
  source 1..100: mol_type = other DNA
ctcagctcagcctagcttggctcagcccagcacagcacgctcaacccggttcagcttggctcagcccagcccagcccagcctagctcagctcagccccgc

SEQ ID NO: 757 - DNA, 100 bp, Homo sapiens
  source 1..100: mol_type = other DNA
ccagctcagcgcagcccagctcagctcagctcagcctagccttgctcggcccagctcagctcagcccagctcagcctagccttgctcagcccagctcagc

SEQ ID NO: 758 - DNA, 100 bp, Homo sapiens
  source 1..100: mol_type = other DNA
tcagcccagccctgcccagctcagcccagcttagtgcagccaagcccagctcagctcagctcacctggtgcaacttagcccagctcagctcagctcagct

SEQ ID NO: 759 - DNA, 100 bp, Homo sapiens
  source 1..100: mol_type = other DNA
caacccagttcaactcagcccagttcagctcagctcagcccagttcagccttgtttagtctaggtcagcttaggtcagttttgcccatctgagtccattt

SEQ ID NO: 760 - DNA, 100 bp, Homo sapiens
  source 1..100: mol_type = other DNA
ctgaaagctggatggagttgtcatggccagaaatggtcagcccaccagacctgcttgtctcagctaaagccatctcattgccaggttcctgcacagccag

SEQ ID NO: 761 - DNA, 100 bp, Homo sapiens
  source 1..100: mol_type = other DNA
gctggcttccatcttttgtctccctctacttgataccccagttccctgcagtcctgccccagcgccacctgggttttggttccaaagcattaccaatcat

SEQ ID NO: 762 - DNA, 100 bp, Homo sapiens
  source 1..100: mol_type = other DNA
taccaccctccactacctgggtggaatatttctttgctgctttaaagtcattaaaacatcttgagaatgagaccaagaatttaggagcctgtgctgtgat

SEQ ID NO: 763 - DNA, 100 bp, Homo sapiens
  source 1..100: mol_type = other DNA
aaaaatgagcaggtccccttgctctagaagtggcagcatatcttctgcaccaagaggagggtattgagatgctcagagcctccaccttcccggagcatcc

SEQ ID NO: 764 - DNA, 100 bp, Homo sapiens
  source 1..100: mol_type = other DNA
cctcccttctgagtctgcagtaaacccctgcctttaaattccctctagataacagtcatcattggaaacaaccaagaaatgcattttatctgaatttgcc

SEQ ID NO: 765 - DNA, 100 bp, Homo sapiens
  source 1..100: mol_type = other DNA
acttaaaattctgccatttaccataaatcgctttggaaggcatgggctactttcaagggtgcgatgatgacctacagtcaatgacttagacaagggcgat

SEQ ID NO: 766 - DNA, 100 bp, Homo sapiens
  source 1..100: mol_type = other DNA
gccagtggggcttggtatgttctcaagcatcattacccatgccatccccattcagaggttgtggagcagctcgtgcgacctctccttcaaatgggcttta

SEQ ID NO: 767 - DNA, 100 bp, Homo sapiens
  source 1..100: mol_type = other DNA
gggaaagttaaatgggagtgacccagacaatggtcactcaaaagactcacataaatgagtctcctgctcttcatcaagcaattaagaccagttccccttc

SEQ ID NO: 768 - DNA, 100 bp, Homo sapiens
  source 1..100: mol_type = other DNA
tagtggaaataagacgtcaaatacaaagttttaagagaagcaaatgcagcagcggcggctgcctgtctcttaccatgtcgggcgcctggtcactgcgagc

SEQ ID NO: 769 - DNA, 100 bp, Homo sapiens
  source 1..100: mol_type = other DNA
cttgcaaagctttggcatggaatcattcctccaagtccattaacaagggctggggcctgagcagccagtcggcccggcagcagaagccacgcatcccagc

SEQ ID NO: 770 - DNA, 100 bp, Homo sapiens
  source 1..100: mol_type = other DNA
tctgggtagtccggggagacccaaagcccaggccgggcctggcagccaccctcccagagcctccgctaggccagtcctgctgacgccgcatcggtgattc

SEQ ID NO: 771 - DNA, 100 bp, Homo sapiens
  source 1..100: mol_type = other DNA
ggaacagaatctgtccttctaaggtgtctccacagtcctgtcttcagcactatctgattgagttttctcttatgccaccaactaacatgcttaactgaaa

SEQ ID NO: 772 - DNA, 100 bp, Homo sapiens
  source 1..100: mol_type = other DNA
taattcaggataatgatgcacattttacctaaaacttatcctaaagtgagtagttgaaaagtggtcttgaaaaatactaaaatgaaggccactctatcag

SEQ ID NO: 773 - DNA, 100 bp, Homo sapiens
  source 1..100: mol_type = other DNA
aatatcaaagtgtttctccttaatcacaaagagaaaacgagttaacctaaaaagattgtgaacacagtcattatgaaaataatgctctgaggtatcgaaa

SEQ ID NO: 774 - DNA, 100 bp, Homo sapiens
  source 1..100: mol_type = other DNA
aagtatttgagattagttatcacatgaagggataacaagctaatttaaaaaactttttgaatacagtcataaactctccctaagactgtttaatttctta

SEQ ID NO: 775 - DNA, 100 bp, Homo sapiens
  source 1..100: mol_type = other DNA
aacatcttactttaaaaatgaatgcagtttagaagttgatatgctgtttgcacaaactagcagttgataagctaagattggaaatgaaattcagatagtt

SEQ ID NO: 776 - DNA, 100 bp, Homo sapiens
  source 1..100: mol_type = other DNA
aaaaaaagccttttcagtttcggtcagcctcgccttattttagaaacgcaaattgtccaggtgttgttttgctcagtagagcactttcagatctgggcct

SEQ ID NO: 777 - DNA, 100 bp, Homo sapiens
  source 1..100: mol_type = other DNA
gggcaaaaccacctcttcacaaccagaagtgataaatttaccaattgtgtttttttgcttcctaaaatagactctcgcggtgacctgcttcctgccacct

SEQ ID NO: 778 - DNA, 100 bp, Homo sapiens
  source 1..100: mol_type = other DNA
gctgtgggtgccggagacccccatgcagccatcttgactctaattcatcatctgcttccagcttcgctcaattaattaaaaaaataaacttgatttatga

SEQ ID NO: 779 - DNA, 100 bp, Homo sapiens
  source 1..100: mol_type = other DNA
tggtcaaaacgcagtcccgcatcggggccgacagcactgtgctagtatttcttagctgagcttgctttggcctcaattccagacacatatcactcatggg

SEQ ID NO: 780 - DNA, 100 bp, Homo sapiens
  source 1..100: mol_type = other DNA
tgttaatcaaatgataagaatttcaaatacttggacagttaaaaaaattaatatacttgaaaatctctcacatttttaagtcataattttcttaaccatt

SEQ ID NO: 781 - DNA, 100 bp, Homo sapiens
  source 1..100: mol_type = other DNA
tttctcagaagccacttcaaacatatcctgtcttttaacagtaagcatgcctcctaagataaacaatccttttctcttggaaaccagcttcaaggcactg

SEQ ID NO: 782 - DNA, 100 bp, Homo sapiens
  source 1..100: mol_type = other DNA
aggtcctggagcctccctaagcccctgtcaggacggcagccaccgtttctgggctacccctgcccccaaccctgctctcatcaagaccggggctacgcgt

SEQ ID NO: 783 - DNA, 100 bp, Homo sapiens
  source 1..100: mol_type = other DNA
ccctcctggctggattcacccactccgacagttctctttccagccaataaagaatttaagatgcaggttgacacacagcgcacctcataattctaaagaa

SEQ ID NO: 784 - DNA, 100 bp, Homo sapiens
  source 1..100: mol_type = other DNA
aatatttcacgattcgctgctgtgcagcgatcttgcagtcctacagacaccgctcctgagacacattcctcagccatcactaagacccctggtttgttca

SEQ ID NO: 785 - DNA, 100 bp, Homo sapiens
  source 1..100: mol_type = other DNA
ggcatctcgtccaaatgtggctccccaagcccccaggctcagttactccatcagacgcacccaacctgagtcccattttccaaaggcatcggaaaatcca

SEQ ID NO: 786 - DNA, 100 bp, Homo sapiens
  source 1..100: mol_type = other DNA
cagaggctcccagatcctcaaggcaccccagtgcccgtcccctcctggccagtccgcccaggtcccctcggaacatgccccgaggaccaacctgcaatgc

SEQ ID NO: 787 - DNA, 100 bp, Homo sapiens
  source 1..100: mol_type = other DNA
tcaggaaaccccacaggcagtagcagaaaacaaaggccctagagtggccattcttacctgaggagacggtgaccgtggtccctttgccccagacgtccat

SEQ ID NO: 788 - DNA, 100 bp, Homo sapiens
  source 1..100: mol_type = other DNA
gtagtagtagtagtagtaatcacaatggcagaatgtccatcctcaccccacaaaaacccagccacccagagaccttctgtctccgggcgtcacatggaag

SEQ ID NO: 789 - DNA, 100 bp, Homo sapiens
  source 1..100: mol_type = other DNA
ctgactgtccgtggccctgtcctgcccttctcatggaaccctctgctggcctcccacgtaccccacattctggcctgacccctcagaagccagaccactg

SEQ ID NO: 790 - DNA, 100 bp, Homo sapiens
  source 1..100: mol_type = other DNA
tcggcctgggaagtccaactgcaagcagacggctgctaagtcacccccaggagtccaaaaaccccggggggcacccgtcccagagagcgggtgccttgga

SEQ ID NO: 791 - DNA, 100 bp, Homo sapiens
  source 1..100: mol_type = other DNA
gcgggacagagtcccaccacgcaatcatcacgacagcccctgagaatgctccaggtgaagcggagagaggtcaccccagaccagccgaaggagcccccca

SEQ ID NO: 792 - DNA, 100 bp, Homo sapiens
  source 1..100: mol_type = other DNA
gctgccgacatctgtggccggacttggggaggacaggctgggttcccattcgaagggtccctctccccggctttctttcctgacctccaaaatgcctcca

SEQ ID NO: 793 - DNA, 100 bp, Homo sapiens
  source 1..100: mol_type = other DNA
agactctgaccctgagaccctggcaagctgagtctccctaagtggactcagagagggggtggtgaggactcacctgaggagacggtgaccagggttccct

SEQ ID NO: 794 - DNA, 100 bp, Homo sapiens
  source 1..100: mol_type = other DNA
ggccccaggggtcgaaccagttgtcacattgtgacaacaatgccaggaccccaggcaagaactggcgccccgctacgtccctgggaccctctcagactga

SEQ ID NO: 795 - DNA, 100 bp, Homo sapiens
  source 1..100: mol_type = other DNA
gcccggggagggcccgggggttgttgggcattggaccccagaggcctagggtggccctggccacagagagacccgtgctgctgggctcaggaggaaggag

SEQ ID NO: 796 - DNA, 100 bp, Homo sapiens
  source 1..100: mol_type = other DNA
catctggagcccttgcccctcgtctgtgtggccgctgttgcctcagggcatcctcctgagccccccaggatgctccggggctctcttggcaggagaccca

SEQ ID NO: 797 - DNA, 100 bp, Homo sapiens
  source 1..100: mol_type = other DNA
gcacccttatttccccccagaaatgcagcaaaacccttcagagttaaagcaggagagaggttgtgaggactcacctgaggagacggtgaccagggttccc

SEQ ID NO: 798 - DNA, 100 bp, Homo sapiens
  source 1..100: mol_type = other DNA
tggccccagtagtcaaagtagtcacattgtgggaggccccattaaggggtgcacaaaaacctgactctccgactgtcccgggccggccgtggcagccagc

SEQ ID NO: 799 - DNA, 100 bp, Homo sapiens
  source 1..100: mol_type = other DNA
cccgtgtcccaaggtcattttgtccccagcacaagcatgactctgcccaccctttgccccagcagcagagtcccagttcccaaagaaaggccttctgctg

SEQ ID NO: 800 - DNA, 100 bp, Homo sapiens
  source 1..100: mol_type = other DNA
aacgtggtcccaaacagccggagaaggagccccggagggccccacatggcccagcgcagaccaaggagcccccggacattatctcccagctccaggacag

SEQ ID NO: 801 - DNA, 100 bp, Homo sapiens
  source 1..100: mol_type = other DNA
aggacgctgggcccagagaaaggaggcagaaggaaagccatcttacctgaagagacggtgaccattgtcccttggccccagatatcaaaagcatcacaca

SEQ ID NO: 802 - DNA, 100 bp, Homo sapiens
  source 1..100: mol_type = other DNA
gggacacagtccctgttcctgcccagacacaaacctgtgcccgtgcaggacactcgaatgggtcacatggcccaagcacagagcagaggcagccggcgtc

SEQ ID NO: 803 - DNA, 100 bp, Homo sapiens
  source 1..100: mol_type = other DNA
cctgtccccagccacacagacccccgggctgagacccaggcagggaggggtgacgttcccagggagacggtggccgggctgccctggccccagtgctcca

SEQ ID NO: 804 - DNA, 100 bp, Homo sapiens
  source 1..100: mol_type = other DNA
agcacttgtagccacactaaagcgcaggcctggtccccggcacatgaacagccagcgcccagccccagcccaggctctgcccacaacttctccttcccgt

SEQ ID NO: 805 - DNA, 100 bp, Homo sapiens
  source 1..100: mol_type = other DNA
ccctgccctcggcctgcttgctacctgtggagggtccctgacggggctgaagcccagcggggtccctgcctgtccttgggggctccagctggccccaggg

SEQ ID NO: 806 - DNA, 100 bp, Homo sapiens
  source 1..100: mol_type = other DNA
ctaagtgacagcagggctctggcatgcagcccatggcggagaccccagggatggcagctggtgtggcctcaggccagacccaggccggctgcagacccca

SEQ ID NO: 807 - DNA, 100 bp, Homo sapiens
  source 1..100: mol_type = other DNA
gatacctggcctggtgcctggacagagaagactgggagggggctgcagtgggactcacctgaggagacagtgaccagggtgccacggccccagagatcga

SEQ ID NO: 808 - DNA, 100 bp, Homo sapiens
  source 1..100: mol_type = other DNA
agtaccagtagcacagcctctgccctcctgcttctcccatacaaaaacacaccctccgccctcctgccgacctcctttgctgagcacctgtccccaagtc

SEQ ID NO: 809 - DNA, 100 bp, Homo sapiens
  source 1..100: mol_type = other DNA
tgaagccaaagcccttgcctggcccagtacacctggctccccgctatccccagacagcagactcacctgaggagacggtgaccagggtgccctggcccca

SEQ ID NO: 810 - DNA, 100 bp, Homo sapiens
  source 1..100: mol_type = other DNA
gtgctggaagtattcagccacggtgagtcagccctgagccaggggctacagaaacccacagcccggggtcccgggggagcatggtttttgtagagctgcc

SEQ ID NO: 811 - DNA, 100 bp, Homo sapiens
  source 1..100: mol_type = other DNA
aatcactgtgtccccagttagcacagtggttctcagctcagccaaaaccctgcggctggtagggggcctgtggggctgggggctgatgtggctgcggtct

SEQ ID NO: 812 - DNA, 100 bp, Homo sapiens
  source 1..100: mol_type = other DNA
tgctgggtctgtcctctgtgggaggggctgctacccaggcccaggactgcagtggagggctcactgaggggcttttgggtctggcctgagccgctgtggg

SEQ ID NO: 813 - DNA, 100 bp, Homo sapiens
  source 1..100: mol_type = other DNA
gctctcaggtctactgcggggacactcgggtctgcccctggcttaggtggacagtgtccgtgcccacctgtgccctgaggctccatttcaggctgatatc

SEQ ID NO: 814 - DNA, 100 bp, Homo sapiens
  source 1..100: mol_type = other DNA
tgtctgtattgtccctacccgctgcatggccatgtccttttgggtttataaattgcccccaaatcacgcaggcatcattcaggctttttatattccctgg

SEQ ID NO: 815 - DNA, 100 bp, Homo sapiens
  source 1..100: mol_type = other DNA
tattccctgggccaccaggtgcctccacccagaaagctgagatgtgggaggttctagagtcattctgcaaccctggatgagcccctgcagcctcagtgct

SEQ ID NO: 816 - DNA, 100 bp, Homo sapiens
  source 1..100: mol_type = other DNA
actgaggttccagcaagacctggagcaggtgcagatgaggcctgaggccaggtgaagcccaggccaggtgaggtccaggccagtgaggcccaggtcagat

SEQ ID NO: 817 - DNA, 100 bp, Homo sapiens
  source 1..100: mol_type = other DNA
gaggcccaggtcaggtgaagcccaggtcaggtgaaacccaggtcaggtgaggcccagatcatgtgagctcaggacaggcaaggtccaagtcaggtgaggc

SEQ ID NO: 818 - DNA, 100 bp, Homo sapiens
  source 1..100: mol_type = other DNA
cgagctcaggtgaagcccagaggtgaggtctaggccaggtgaggtccaggccaggtgaggtccaggtcaggtgaggcccaggtcaggcaaggctgaggta

SEQ ID NO: 819 - DNA, 100 bp, Homo sapiens
  source 1..100: mol_type = other DNA
tccaggtcaggtgaggcccaggtcaggcaaggctgaggtagatgtatgagacttctgtaattttcagttggtgccaaccctgcctggtgtccctgcccct

SEQ ID NO: 820 - DNA, 100 bp, Homo sapiens
  source 1..100: mol_type = other DNA
cctcccagcccatgctctgtgcctgccagatggcggcccctgcacaggtgctgctggctgtggaggagctgggctctgcctccctgtgcatgggcgtccc

SEQ ID NO: 821 - DNA, 100 bp, Homo sapiens
  source 1..100: mol_type = other DNA
gcctgcagcctgtccggggatgcccagggaggtgagtgccaccacatatcaggccttttctctttaaagtcatttctttggggatacatcatcaatgtct

SEQ ID NO: 822 - DNA, 100 bp, Homo sapiens
  source 1..100: mol_type = other DNA
tctaaacacagctgtgtgcattttcctcttcttgcaatttagaattttaactgctgttttcaaggtactgtaatgtatttgttctcttcttgttaggaga

SEQ ID NO: 823 - DNA, 100 bp, Homo sapiens
  source 1..100: mol_type = other DNA
cttgccaaccctgtgtgtctcagttcataccctcttccttccccagtagaagtaacgaccactgtgtttatgtgatcatccttttcttgattttccttat

SEQ ID NO: 824 - DNA, 100 bp, Homo sapiens
  source 1..100: mol_type = other DNA
tgtgatcatccttttcttgattttccttatagttttcctagtggaaagtttatcccttaagaagatagttcattttgccggctgtaaattttatttagaa

SEQ ID NO: 825 - DNA, 100 bp, Homo sapiens
  source 1..100: mol_type = other DNA
ctgccatcgtttatttgcctgttttccttcagatggctgtttgcttcattctcagtttggggctatgacaaacatatgttctgcacatctttgcccatga

SEQ ID NO: 826 - DNA, 100 bp, Homo sapiens
  source 1..100: mol_type = other DNA
ggctctcagggagggctctggagctggcattgcctgcagggctctgctttgttgcagggagttcctgccaaggcttttcagagtgtctgtgcccagcctg

SEQ ID NO: 827 - DNA, 100 bp, Homo sapiens
  source 1..100: mol_type = other DNA
aaggtacacactgtactttgcccttgcatcaggcactttccttgtgcttgcttctgtgtggctccacattctggagaatttattcagatctgtgctgcaa

SEQ ID NO: 828 - DNA, 100 bp, Homo sapiens
  source 1..100: mol_type = other DNA
cttcccacactgtcctcctgggctcactcccagccatcgatcttgaacaccagtttatggaactatctgcacaggaaagcagaaacagcaaaaggccctg

SEQ ID NO: 829 - DNA, 100 bp, Homo sapiens
  source 1..100: mol_type = other DNA
ttgcgtggaccctgtttttggtcaagggaagtacttgctggtgaaggagacctcccctcctttctttctcaggagccccctctgatgccgttgcctggtg

SEQ ID NO: 830 - DNA, 100 bp, Homo sapiens
  source 1..100: mol_type = other DNA
tttctcagggctggtgctgggggctcagcagtgtctgccctgttccaggtgggaatgtgggtctgttctgtttccacgcggtgttctggggccgccagtg

SEQ ID NO: 831 - DNA, 100 bp, Homo sapiens
  source 1..100: mol_type = other DNA
cagcagtgtctgccctgttccaggtgggaatgtgggtctgttctgtttccacgcggtgttctggggccgccagtgaggggctcgggatgtcagcggctgg

SEQ ID NO: 832 - DNA, 100 bp, Homo sapiens
  source 1..100: mol_type = other DNA
tctctgtccctatggtctgggctccggttcactgctcccctgccctccaggtcggtcactgactcagttactatccagcgggctccgtggctgttcagtg

SEQ ID NO: 833 - DNA, 100 bp, Homo sapiens
  source 1..100: mol_type = other DNA
gggagcaaatggagagggaagtggcagcggcccgagtgccaggcggtcccggtttggggttgatctttgtggaacagctccctggcccgtgtgtaagtgg

SEQ ID NO: 834 - DNA, 100 bp, Homo sapiens
  source 1..100: mol_type = other DNA
tcgggggaggcacggaggtctggagctacaagcggtggcaggaaggcaggtcccagtcttgggggtctggagcttatcttcttcctgtgaactgagtgtg

SEQ ID NO: 835 - DNA, 100 bp, Homo sapiens
  source 1..100: mol_type = other DNA
atggaggacctgcctcggatgacacccctatcttaagaaggtcatggtgggttccagctgggaggaagggaagtgggccacctcctgggggtcttccacc

SEQ ID NO: 836 - DNA, 100 bp, Homo sapiens
  source 1..100: mol_type = other DNA
gtcttccacccccaccacctcagcctggggcctctgtgattcctctctgcacagaccccaaagtctgtgctgccgcagggcaggaaggaagggcctgtgg

SEQ ID NO: 837 - DNA, 100 bp, Homo sapiens
  source 1..100: mol_type = other DNA
tcgaggttggggccacagtggtgttccctaagcccgagtctggtctcatggcccgccccgcagcaggtcctgagtgagggacagagaccggggcggggtc

SEQ ID NO: 838 - DNA, 100 bp, Homo sapiens
  source 1..100: mol_type = other DNA
tttggtcctggtggactctggggtggattccagtggggagtcatcagggtcggtgtcccccagggtactggggtgtctctgctcctggagtcggctctgg

SEQ ID NO: 839 - DNA, 100 bp, Homo sapiens
  source 1..100: mol_type = other DNA
cctgggtttttgtacaggaggtgccctgggctgtgtctttgtggtctgtgtgcacagtaatatgtggctgtgtccacagggtccatgttggtcattgtaa

SEQ ID NO: 840 - DNA, 100 bp, Homo sapiens
  source 1..100: mol_type = other DNA
gtgtccttggtgatggtgagcctgctcttcagagatgggctgtagcgcttatcatcattccaataaatgagtgcaagccactccagggcctttcctgggg

SEQ ID NO: 841 - DNA, 100 bp, Homo sapiens
  source 1..100: mol_type = other DNA
gctgacggatccagcccacacccactccactagtgctgagtgagaacccagagaaggtgcaggtcagcgtgagggtctgtgtgggtttcaccagcgtagg

SEQ ID NO: 842 - DNA, 100 bp, Homo sapiens
  source 1..100: mol_type = other DNA
ctgtggagaaagcataagaagatgaagcccacaaacaagaaaactgatgtttcacccgtgaaggagtccctgaccacagcactcacatgaagggatggtc

SEQ ID NO: 843 - DNA, 100 bp, Homo sapiens
  source 1..100: mol_type = other DNA
agcagcaggagcgtggagcaaagtgtgtccatggtggggcacaggagtcactgagctgggacctgtgctcggctttttcaacccagaggagggtggagct

SEQ ID NO: 844 - DNA, 100 bp, Homo sapiens
  source 1..100: mol_type = other DNA
aagtgtgtccatggtggggcacaggagtcactgagctgggacctgtgctcggctttttcaacccagaggagggtggagctggtggagatttgcattcccc

SEQ ID NO: 845 - DNA, 100 bp, Homo sapiens
  source 1..100: mol_type = other DNA
agatttgcattcccctcatctgtgccctactctatgggatggagtcaggtttcaggactcaggagggtgttgcatctgtggtgaggaccagtgatagtaa

SEQ ID NO: 846 - DNA, 100 bp, Homo sapiens
  source 1..100: mol_type = other DNA
catgatcagtgtaattcagatggcattaatctaaggctgggcaagtagattctgagtagaagtctttgcagaagtcatgattatgaggtcatgttggtct

SEQ ID NO: 847 - DNA, 100 bp, Homo sapiens
  source 1..100: mol_type = other DNA
gcccttcacagagtccacatagtatttctcacttccatcttgctttatgttggccacccactccagccccttccctggagcctggcggacccagctcatc

SEQ ID NO: 848 - DNA, 100 bp, Homo sapiens
  source 1..100: mol_type = other DNA
tgagtcctctgtgctcagtgctgatcaccaagtggaaaggccttggagtccagggctaaggctcctctctgagacctgcagggtcagggttgggttggtt

SEQ ID NO: 849 - DNA, 100 bp, Homo sapiens
  source 1..100: mol_type = other DNA
ttcatcagtagagggagggccctatttgcatgtctcctactatataagaagctctagtgggatgctggaggaataggctgtacccatataagaagacggt

SEQ ID NO: 850 - DNA, 100 bp, Homo sapiens
  source 1..100: mol_type = other DNA
agggccctatttgcatgtctcctactatataagaagctctagtgggatgctggaggaataggctgtacccatataagaagacggtgctctgcagaagttt

SEQ ID NO: 851 - DNA, 100 bp, Homo sapiens
  source 1..100: mol_type = other DNA
gctgacaatgatggtatttggaaaatatgctgtcttatgaaattgtgctgtgataaacactttgccctgatcaccctattacattttttaaaaaatgtgt

SEQ ID NO: 852 - DNA, 100 bp, Homo sapiens
  source 1..100: mol_type = other DNA
caaacacagagacaacctagtcagaaactgccacatatattcactgcttatctcactcacgtccactcaatgtctctagttctccataaatcacctttta

SEQ ID NO: 853 - DNA, 100 bp, Homo sapiens
  source 1..100: mol_type = other DNA
taatagcaacaaggaaaacccagctcagcccaaactccatggtgagtcctctgtgttcagtgctgatcaccgaatggaaactcctgggaattctggggct

SEQ ID NO: 854 - DNA, 100 bp, Homo sapiens
  source 1..100: mol_type = other DNA
gtcctctgtgttcagtgctgatcaccgaatggaaactcctgggaattctggggctggggctcttctcccagagctgcagggtctgggctcggctggtttt

SEQ ID NO: 855 - DNA, 100 bp, Homo sapiens
  source 1..100: mol_type = other DNA
tatcagcagagggagggccctatttgcatgtctcctactatatagcaagctctagtgggacgctggaggagagggcagtgcccagagcagatgagagggt

SEQ ID NO: 856 - DNA, 100 bp, Homo sapiens
  source 1..100: mol_type = other DNA
cccggaaaacactggaggtaatcctatctctcaggaaaatataacttcagattatgtgattgtgacttgatgatcaattagcagtcatcatcttatttaa

SEQ ID NO: 857 - DNA, 100 bp, Homo sapiens
  source 1..100: mol_type = other DNA
tgtttacatatttgcagaatatattcagtgcaagtgtcaatgttacatttttagagaagatgaattacatacataacagagcagttgtgcaatgtgtcca

SEQ ID NO: 858 - DNA, 100 bp, Homo sapiens
  source 1..100: mol_type = other DNA
actcacacttaatctctctagttctccataaatcaccttttaaaatagcagcaaggaaaatccagctcagcccaaactccatggtgagtcctctgtgttc

SEQ ID NO: 859 - DNA, 100 bp, Homo sapiens
  source 1..100: mol_type = other DNA
gatgctatttaatagcccaattcctgacccaggatgagaaagagcaaatacatgacacatggacgacacaattgtagaagctgagggttcaagccgtaat

SEQ ID NO: 860 - DNA, 100 bp, Homo sapiens
  source 1..100: mol_type = other DNA
cctgttagaggccacgcatcccctacccatccctgaactctgtgttgacagagcttcccccactggagaacaagctcccccaggacacgcacctcactta

SEQ ID NO: 861 - DNA, 100 bp, Homo sapiens
  source 1..100: mol_type = other DNA
ggcccttcacggagtctgcgtagtatgtgctaccaccactaccactaatagctgagacccactccagccccttccctggagcctggcggacccagctcat

SEQ ID NO: 862 - DNA, 100 bp, Homo sapiens
  source 1..100: mol_type = other DNA
ggcatagctgctaaaggtgaatccagaggctgcacaggagagtctcagggaccccccaggctgtaccaagcctcccccagactccaacagctgcacctca

SEQ ID NO: 863 - DNA, 100 bp, Homo sapiens
  source 1..100: mol_type = other DNA
actgtttctctcactcttatccattcacactcaatttttctatttctccatgaattaccttttaaaatagccacaagaaaaagccagctcagcccaaact

SEQ ID NO: 864 - DNA, 100 bp, Homo sapiens
  source 1..100: mol_type = other DNA
ccatggtgagttctctctgttcagtcctgatcaccaaatgaaaacacctgaaaatcccagggctgggctcctctctcagagctgcagggtcagggctggg

SEQ ID NO: 865 - DNA, 100 bp, Homo sapiens
  source 1..100: mol_type = other DNA
tttgcatatctcctactatatagtaagctctggggtgagaggcctttggagatagtggggctcagagcatgtcagaatgtcctcggggagatctgtgata

SEQ ID NO: 866 - DNA, 100 bp, Homo sapiens
  source 1..100: mol_type = other DNA
ttgaaagcattgggaaattgtgctttcctattgtcagtttgttttgtgataaacttaaaccttaaaacctaaaaatcttataattttgtaatttttattt

SEQ ID NO: 867 - DNA, 100 bp, Homo sapiens
  source 1..100: mol_type = other DNA
gaggtaccatagatctacataaactgcatatttttaaagttagcaccaatcatcttttatttttacatacgcagagaaaccatggtatatagtatcaata

SEQ ID NO: 868 - DNA, 100 bp, Homo sapiens
  source 1..100: mol_type = other DNA
ttatttccatgttaaagatgaaaaattatcagcaaaagcacaggtgggttttacaatgtccccagtgctcacttttggtcagagtgagcctgggcatctg

SEQ ID NO: 869 - DNA, 100 bp, Homo sapiens
  source 1..100: mol_type = other DNA
tcctacataatgacagtgtacacatctttccattgctgttttactcaattactcaacccattttctaaacagatttaaacttcataaatcctgtcatctc

SEQ ID NO: 870 - DNA, 100 bp, Homo sapiens
  source 1..100: mol_type = other DNA
ctcagcctcagcacagctgcctcattcctcagggtttctgacgctctcaggatgtgggttttcacactgtgtctgttgcacagtaatacacggccgtgtc

SEQ ID NO: 871 - DNA, 100 bp, Homo sapiens
  source 1..100: mol_type = other DNA
gctcagctccatgtaggctgtgtctgtagatgtgtcctcggtcatggtgactctgccctggaacttctgtgcgtagattgtttcaccatcttcaggatca

SEQ ID NO: 872 - DNA, 100 bp, Homo sapiens
  source 1..100: mol_type = other DNA
ttcaggatcaaaacctcccatccactcaagcccttttccaggagcctgtcgcacccagtgcatggataattcagtgagggtgtatccggaaaccttgcag

SEQ ID NO: 873 - DNA, 100 bp, Homo sapiens
  source 1..100: mol_type = other DNA
gagaccttcactgaggccccaggcttcttcacctcagccccagactgtaccagctggacctgggcgtgggtgcctgtggagaggacagaggagtggatga

SEQ ID NO: 874 - DNA, 100 bp, Homo sapiens
  source 1..100: mol_type = other DNA
gacaccacttaactggacccagtcccctcatcagccctggaactcaggattctcttgcctgtagctgctgccaccaagaagaggatcctccaggtgcagt

SEQ ID NO: 875 - DNA, 100 bp, Homo sapiens
  source 1..100: mol_type = other DNA
gagggtgggaatctgggagagcaaggggcttcccataagtgttctgataaaaatcctctttgtttagggggaaagtgatgatttttttgaatgatagaga

SEQ ID NO: 876 - DNA, 100 bp, Homo sapiens
  source 1..100: mol_type = other DNA
atacatcacccaaacatttaaaaatgtattgtgtaaagaagtgtaaatggcatctcagccatttacacactgcaagacacacagcttattagtgtgcctg

SEQ ID NO: 877 - DNA, 100 bp, Homo sapiens
  source 1..100: mol_type = other DNA
tggtgaatcggcccttcacggagtctgcatagtatttattacttccatcatatgatataactgccacccactccagccccttgcctggagcctggcggac

SEQ ID NO: 878 - DNA, 100 bp, Homo sapiens
  source 1..100: mol_type = other DNA
acaatcacttgagttcagacacaccaggattcacttaatgttatttttagttcagaacctctatcaggtttagagggaatcgctctgtcccagggagtgg

SEQ ID NO: 879 - DNA, 100 bp, Homo sapiens
  source 1..100: mol_type = other DNA
atcttacaatagcaaaacggtcttagaaaacccaacataatctacagcgagacctcagcatggcaagcaaggaatcactaaagccaccagggagatccgg

SEQ ID NO: 880 - DNA, 100 bp, Homo sapiens
  source 1..100: mol_type = other DNA
cactaaagccaccagggagatccggatgcactgatacgatccagaaacatagcgagtccgggaactgatgcggactttgaggcagcctcttttttttttt

SEQ ID NO: 881 - DNA, 100 bp, Homo sapiens
  source 1..100: mol_type = other DNA
gatggtgaatcggcccttcacggagtctgcatagtatttattacttccatcataccatataactgccacccactccagccccttgcctggagcctggcgg

SEQ ID NO: 882 - DNA, 100 bp, Homo sapiens
  source 1..100: mol_type = other DNA
acccagtgcatgccatagctactgaaggtgaatccagacgctgcacaggagagtctcagggacctcccaggctggaccacgcctcccccagactccacca

SEQ ID NO: 883 - DNA, 100 bp, Homo sapiens
  source 1..100: mol_type = other DNA
ctcgactcttgagggacgggttgtagttggtgcttccactatgattgatttccccaatccactccagccccttccctgggggctggcggatccagctcca

SEQ ID NO: 884 - DNA, 100 bp, Homo sapiens
  source 1..100: mol_type = other DNA
ggctggcggatccagctccagtagtaaccactgaaggacccaccatagacagcgcaggtgagggacagggtctccgaaggcttcaacagtcctgcgcccc

SEQ ID NO: 885 - DNA, 100 bp, Homo sapiens
  source 1..100: mol_type = other DNA
actgctgtagctgcacctgggacaggacccctgtgaacagagaaacccacagtgagccctgggatcagaggcagcatctcatatcttcatatccgcattc

SEQ ID NO: 886 - DNA, 100 bp, Homo sapiens
  source 1..100: mol_type = other DNA
ctgagacactcacatctgggagctgccaccaggaggaggaagaaccacaggtgtttcatgttcttgtgcaggaggtccatgactctcagaaagcacttcc

SEQ ID NO: 887 - DNA, 100 bp, Homo sapiens
  source 1..100: mol_type = other DNA
gaggatttgcatgtgggtggtgcctttgtatggataggtaaaaagggatgagggaggccccagtcttttgggctcaccctgggaggtgtatgctggctgt

SEQ ID NO: 888 - DNA, 100 bp, Homo sapiens
  source 1..100: mol_type = other DNA
agttctcttcctgtggcctcccctcaccaaacccagagtcctcttcttccaggtaggaaatgtgctgaaggagctggtctgggagacaagtgtgatcatg

SEQ ID NO: 889 - DNA, 100 bp, Homo sapiens
  source 1..100: mol_type = other DNA
ggtctgggagacaagtgtgatcatggatcaaagacagattttggaatacagttaatactgttctacatttaaagattcatataacaccaaccatacaccc

SEQ ID NO: 890 - DNA, 100 bp, Homo sapiens
  source 1..100: mol_type = other DNA
aggtcacctaaattgtcatttaccccttcagacatattgaaacagctgctgagtgtaataatcacagtgaattgagacaaacctggatccatgcaatgtg

SEQ ID NO: 891 - DNA, 100 bp, Homo sapiens
  source 1..100: mol_type = other DNA
tactgtagttcagaacatccatcatggttagaaggatgctacctgtcccaggaagtgggttatttttaaatagtacctgagagctgcccttctgagacct

SEQ ID NO: 892 - DNA, 100 bp, Homo sapiens
  source 1..100: mol_type = other DNA
tttgaaatttgagattgtgtgtgagatctcaggagaaggtagtagaatatatctccatccttctcaatgtgtaaccctgagaatatggcctgacctctaa

SEQ ID NO: 893 - DNA, 100 bp, Homo sapiens
  source 1..100: mol_type = other DNA
acatttctgtgtgaaaagatgtacattggggatagcagtgacagcttcagatgaaaactctatagtacatcagcactggaggatagtctcatcaccaaga

SEQ ID NO: 894 - DNA, 100 bp, Homo sapiens
  source 1..100: mol_type = other DNA
ttagtgaaattacctttcctgggaaccagagaggacctctgtgagctctaccctctgagagaacaaggaactctggttcttccctgacaggtcacacctg

SEQ ID NO: 895 - DNA, 100 bp, Homo sapiens
  source 1..100: mol_type = other DNA
aacaagtgggctggccttctatgagacgacagagggaaagagacagactcaatatccagagcgaggtgagctccttacctacctaccaggtggtctctgg

SEQ ID NO: 896 - DNA, 100 bp, Homo sapiens
  source 1..100: mol_type = other DNA
gccatttgtttgagcagacccagaagtaccttcctcaccctcaggagaattatgaacattgagagaaactgagatactttttttatttacagggaatatt

SEQ ID NO: 897 - DNA, 100 bp, Homo sapiens
  source 1..100: mol_type = other DNA
tcatcggcgtgtttacatctacctgggtgtgtacagggatgctaggatgtgctcatacacagaagagcaagaattatatttcgtggaaagaaaaccaaag

SEQ ID NO: 898 - DNA, 100 bp, Homo sapiens
  source 1..100: mol_type = other DNA
agcttctgaatttgtaggtattgtttgctgcaaatgtgtcaggtcactagatcatgttatgctgctagaagaaaaacttcccaacattgtcatggagaca

SEQ ID NO: 899 - DNA, 100 bp, Homo sapiens
  source 1..100: mol_type = other DNA
aaatgcaaaacagtaaagattcaactgagattcccttgaaaatcaccagtaatgaacaggccaaaagaaatcaaccattgtggaaagagtggtcattaag

SEQ ID NO: 900 - DNA, 100 bp, Homo sapiens
  source 1..100: mol_type = other DNA
cccagtgtcaccttacacatcctgcaggtcacctcacacatccaccaggtcaccgcacatataccccacatcacctcagacacaccctggtcacctcata

SEQ ID NO: 901 - DNA, 100 bp, Homo sapiens
  source 1..100: mol_type = other DNA
catacgtcaggtcacctcacgctcacccaaggtcacctcacacatcccgcaggtcacctcgtaaatcccccaggtcaccacatacatgcaccagttcacc

SEQ ID NO: 902 - DNA, 100 bp, Homo sapiens
  source 1..100: mol_type = other DNA
ctcttgagggacgggttgtagtaggtgctcccactataatagatactcccaatccactccagccccttccctgggggctggcggatccagccccagtagt

SEQ ID NO: 903 - DNA, 100 bp, Homo sapiens
  source 1..100: mol_type = other DNA
aactactactgctgatggagccaccagagacagtgcaggtgagggacagggtctccgaaggcttcaccagtcctgggcccgactcctgcagctgcagctg

SEQ ID NO: 904 - DNA, 100 bp, Homo sapiens
  source 1..100: mol_type = other DNA
gaacagaaaaacccacagtgagccctgggatcagaggcagcctcccatatctccatgtctgcatcctagaaacactcacatctgggagccgccaccagca

SEQ ID NO: 905 - DNA, 100 bp, Homo sapiens
  source 1..100: mol_type = other DNA
ggaggaagaaccacaggtgcttcattttcttgcacatgagatccatgactctcagaaagcatttcccttatgagttggacctgaatttaaggaaatgtgt

SEQ ID NO: 906 - DNA, 100 bp, Homo sapiens
  source 1..100: mol_type = other DNA
ggtggcttcctgtgggcgcctaagtgaggatttgcatgggggtggtgcgtttgtacggagcagtgaaaagggatgagagaggcgccagtcttttgagctc

SEQ ID NO: 907 - DNA, 100 bp, Homo sapiens
  source 1..100: mol_type = other DNA
accctgggaggagaatgctggctgtgccctttgagaactcagttctcttcttgggcctcccctctccaagcccagagtcctcttcttccaggtaaagaga

SEQ ID NO: 908 - DNA, 100 bp, Homo sapiens
  source 1..100: mol_type = other DNA
tgtgctgaaggagctggtctgagagatgagtgtgatcctggatcaaggacagattttggaatagggtcagtactgttcaacccttaaagattcatataaa

SEQ ID NO: 909 - DNA, 100 bp, Homo sapiens
  source 1..100: mol_type = other DNA
acccaccacacacccaggccatctaaatagtcatttaccctttcagacacattgaaacaacagctgaatgtaataatgacagtgacttcaaacaatactg

SEQ ID NO: 910 - DNA, 100 bp, Homo sapiens
  source 1..100: mol_type = other DNA
atgtttattgtagttcagaacatccaccatggttacagggaagctcactgtccctggaagtgggtcattttttaaaagcacctgagagctgtccttctgt

SEQ ID NO: 911 - DNA, 100 bp, Homo sapiens
  source 1..100: mol_type = other DNA
aaggtagtgggacatatctccatacttctcaatgtgtgaccttgaagatgtgtcctgccctctaaacacttctgattgaaaatatgtagattggggatta

SEQ ID NO: 912 - DNA, 100 bp, Homo sapiens
  source 1..100: mol_type = other DNA
gtggaaatgccttggaatccagggctaaggcacctctctgagagctgcagggtcagggttgggttggttttcatcagtagagggagggccctatttgcat

SEQ ID NO: 913 - DNA, 100 bp, Homo sapiens
  source 1..100: mol_type = other DNA
ggacccttgaggagtaggctgtacccagataagacgacggtgccctgtagaagtttgctggcaatgattgcatttggaaaatatgctgtcttattatgaa

SEQ ID NO: 914 - DNA, 100 bp, Homo sapiens
  source 1..100: mol_type = other DNA
attgtgctgtgataaacactttgcactaatcaccctatttcattttaaatattcatgtaaactatgttctgtaggagacaatattttctccatttacaga

SEQ ID NO: 915 - DNA, 100 bp, Homo sapiens
  source 1..100: mol_type = other DNA
acactttgcactaatcaccctatttcattttaaatattcatgtaaactatgttctgtaggagacaatattttctccatttacagaagtggaagtaaaccc

SEQ ID NO: 916 - DNA, 100 bp, Homo sapiens
  source 1..100: mol_type = other DNA
ctgtatgcatctaggagctcatgtctgggatgagtgaaccccggtatctggccctgtgctcttcatcactgtctctgacatccccctaaaccaactccag

SEQ ID NO: 917 - DNA, 100 bp, Homo sapiens
  source 1..100: mol_type = other DNA
gacaaagctggatgtgtctagtgtttttatcagaacccactttccgtaataagagcatgtgtggttttgctgccctccagcactcttctgaaaatatgga

SEQ ID NO: 918 - DNA, 100 bp, Homo sapiens
  source 1..100: mol_type = other DNA
gagaactaggatccaggcacattaattttcaggtacttctgacattgaacttattttttctatctttctattactctttccttgtctaagtttccatttg

SEQ ID NO: 919 - DNA, 100 bp, Homo sapiens
  source 1..100: mol_type = other DNA
agagagacccacagtgagccctgggatcagaggcacctcccatatccccatgtctggatccctgagatactcacatctgggagctgccaccaggagaagg

SEQ ID NO: 920 - DNA, 100 bp, Homo sapiens
  source 1..100: mol_type = other DNA
aagaaccacagatgtttcatgttcttgcacaggaggtccaggactctcagaaagtatttcccatgtgagctggaacctgaatttaaggaaatgtgtggtg

SEQ ID NO: 921 - DNA, 100 bp, Homo sapiens
  source 1..100: mol_type = other DNA
atttgcatgtgggtggtgcctttgtatggagaggtgaaaaaggaggagggaggccccagtcttttgggctcgccctgggagtaggatgctggctgtgccc

SEQ ID NO: 922 - DNA, 100 bp, Homo sapiens
  source 1..100: mol_type = other DNA
tttgagaactcagttgtcttcttggggtctcccctctccaagcccagagtcctcttctttcaggtaaagagacgtgctgaaggacctggtctgggagatg

SEQ ID NO: 923 - DNA, 100 bp, Homo sapiens
  source 1..100: mol_type = other DNA
ctgacagtggtgaccatggttgagaacttttcatctcctctgtgaggatcaatctgcattttctgcataggagaataggttttcatattaaaacaatcat

SEQ ID NO: 924 - DNA, 100 bp, Homo sapiens
  source 1..100: mol_type = other DNA
tttaaaaatatgtagaaatgaccctagtaatcacagaattccgaacttaggttcagtagagaaactttaagaagatgaagtcccacatcgtgacaggaaa

SEQ ID NO: 925 - DNA, 100 bp, Homo sapiens
  source 1..100: mol_type = other DNA
tggagatggtgaatctgcccttcacagagtctgcataatatgtgctacccccattactactaatagctgaaacatattccagtcccttccctggagcctg

SEQ ID NO: 926 - DNA, 100 bp, Homo sapiens
  source 1..100: mol_type = other DNA
gcggacccagtgcatagcatagctactgaaggtgaatccagaggctgcacaggagagtctcagggaccccccaggctggaccaagccttccccagactcc

SEQ ID NO: 927 - DNA, 100 bp, Homo sapiens
  source 1..100: mol_type = other DNA
ttctctcactcatgtccactcacactcaatatctctatttcctcatgaatcacctttaaaaatagcaacaaggaaaacccagctcagcccaaactccatc

SEQ ID NO: 928 - DNA, 100 bp, Homo sapiens
  source 1..100: mol_type = other DNA
atgactcttctgtgttcagtgctgatcaccaaatgaaaacacctgggaatcccagggcgggggctcctctcccagagctgcggagtcagggctgggctgg

SEQ ID NO: 929 - DNA, 100 bp, Homo sapiens
  source 1..100: mol_type = other DNA
tagggcacatccttcccatccactcaagcccttgtgcatgggcctggcgcacctagtgcatagagtaactggtgaaggtaggtgtatccacaagtcttgc

SEQ ID NO: 930 - DNA, 100 bp, Homo sapiens
  source 1..100: mol_type = other DNA
aggagactttcactgatgccccagccttcttcatctcatccccagactgcaccagctgcacctgggactgggcacctgtggagaggacacgggagtggat

SEQ ID NO: 931 - DNA, 100 bp, Homo sapiens
  source 1..100: mol_type = other DNA
gaaaacttgttcacagtagcaccttcatggaatgtttgtatcaacgttatagagtgtggccttttccactctgtgaatttggcttatattacgactcttg

SEQ ID NO: 932 - DNA, 100 bp, Homo sapiens
  source 1..100: mol_type = other DNA
aatggaatatttatcttaaaattagagtatgtacttgtttctactgttctttttttctcaaatatataacccattttgtaaacagccttaaacctaataa

SEQ ID NO: 933 - DNA, 100 bp, Homo sapiens
  source 1..100: mol_type = other DNA
ctgctcagctccatgtaggctgtgctcgtggatttgtccgcggtaatcgtgactctgccctggaacttctgtgcgtagtttgctgtaccaaagataggga

SEQ ID NO: 934 - DNA, 100 bp, Homo sapiens
  source 1..100: mol_type = other DNA
tgatccctcccatccactcaagcccttgtccaggggcctgtcgcacccagctgatagcatagctgctgaaggtgcctccagaagccttgcaggagacctt

SEQ ID NO: 935 - DNA, 100 bp, Homo sapiens
  source 1..100: mol_type = other DNA
caccgaggacccaggcttcttcacctcagccccagactgcaccagctgcacctgggactggacacctgtggagaggacacaggggtgaataaaatcctct

SEQ ID NO: 936 - DNA, 100 bp, Homo sapiens
  source 1..100: mol_type = other DNA
cctgggactggacacctgtggagaggacacaggggtgaataaaatcctctttaactaaaccaggatcccttcctcagccttaggactaggaagcccctta

SEQ ID NO: 937 - DNA, 100 bp, Homo sapiens
  source 1..100: mol_type = other DNA
cctgtagctgctgccaccacaaagaggaacctccaggtccagtccatggtgatgagctgtgctcccaggggcttcttcagaggaggaatgtggttgttat

SEQ ID NO: 938 - DNA, 100 bp, Homo sapiens
  source 1..100: mol_type = other DNA
gtgatgctctcagggcaccaatatatctatatttatctcagaagacctcaggttatttgcatatgcatgaggcagggtatttcacagctcaaagcctgat

SEQ ID NO: 939 - DNA, 100 bp, Homo sapiens
  source 1..100: mol_type = other DNA
tttgcatatgcatgaggcagggtatttcacagctcaaagcctgatctaggatgagaaagaaaacacagatgccacatcagctgtacaagtgtgggatgct

SEQ ID NO: 940 - DNA, 100 bp, Homo sapiens
  source 1..100: mol_type = other DNA
cagaacaaaccccaaccccaggatgcactcctcactgtgaacccacattttattggcctaaagattacctgggttttttgtgggaccattgctgtctctg

SEQ ID NO: 941 - DNA, 100 bp, Homo sapiens
  source 1..100: mol_type = other DNA
acattgagcaggcacctagacccatcctggtcccattaggaacactcagagctcactggtaacactgaaaaggtggccactcgttaccctacatgagtgt

SEQ ID NO: 942 - DNA, 100 bp, Homo sapiens
  source 1..100: mol_type = other DNA
ccagcaggacccatggagagttctgagatctgctgggcactcccaagacagggtccccagcactttcctgagggtcctgacctcccaggtccttcagtgg

SEQ ID NO: 943 - DNA, 100 bp, Homo sapiens
  source 1..100: mol_type = other DNA
ttatccatttctatgtgttcttttgaaaatgtctactcatgtcctttgctcattttaacggagttatttggttcttgttgctgttgttgttgtagagttg

SEQ ID NO: 944 - DNA, 100 bp, Homo sapiens
  source 1..100: mol_type = other DNA
ttgcaaattcttcatattagttccctgtcacaggcaaagtgtgcaaaagttttctgtcattctgtaaattgcgtattcactctgttgttgtgaaaaaaat

SEQ ID NO: 945 - DNA, 100 bp, Homo sapiens
  source 1..100: mol_type = other DNA
tatttaggttaattaaatctcatctgtctatttttttttaggtagcaggacctttcatgctgaatctttgtcaaacaggatacagcttctgcttgcatga

SEQ ID NO: 946 - DNA, 100 bp, Homo sapiens
  source 1..100: mol_type = other DNA
accactaacaggggacatgccatttattagtaaagaaaaaggaggaaaacaaggctctgagtcagatggggatgggaaacgcacgccctgggcaggaaat

SEQ ID NO: 947 - DNA, 100 bp, Homo sapiens
  source 1..100: mol_type = other DNA
ggcatctcagccacactatcctgttctgcagaagtggggagggagcaccactgaaaaacacctgggttcttgtacaggaagcgccctgggctgtgtctct

SEQ ID NO: 948 - DNA, 100 bp, Homo sapiens
  source 1..100: mol_type = other DNA
gtggtatccgtgcacaataatacgtggctgtgtccacagggtccatgttggtcattgtaaggaccacctggtttttggaggtgtccttggagatggtgag

SEQ ID NO: 949 - DNA, 100 bp, Homo sapiens
  source 1..100: mol_type = other DNA
acctggtttttggaggtgtccttggagatggtgagcctggtcttcagagatgtgctgtagtatttatcatcatcccaatcaatgagtgcaagccactcca

SEQ ID NO: 950 - DNA, 100 bp, Homo sapiens
  source 1..100: mol_type = other DNA
gggccttccctgggggctgacggatccagctcacacacattccactagtgctgagtgagaacccagagaaggtgcaggtcagtgtgagggtctgtgtggg

SEQ ID NO: 951 - DNA, 100 bp, Homo sapiens
  source 1..100: mol_type = other DNA
tttcaccagcgcaggaccagactccctcaaggtgacctgggataagacccctgtggagaagacataagaagatgaagcccacaaaggagagaatagattt

SEQ ID NO: 952 - DNA, 100 bp, Homo sapiens
  source 1..100: mol_type = other DNA
ctgtggagaagacataagaagatgaagcccacaaaggagagaatagattttttgcttctgaagtactacctgaccacagcactcacaggacgggacagtc

SEQ ID NO: 953 - DNA, 100 bp, Homo sapiens
  source 1..100: mol_type = other DNA
agtagcaggagcgtggaacaaagtatgtccatggtggagagcaggattcactgagcgaggccctgtcctcgtcttttgaacccaggggagggtggagctg

SEQ ID NO: 954 - DNA, 100 bp, Homo sapiens
  source 1..100: mol_type = other DNA
gtggagatttgcatcccctcatctgagccctactctatggggtgcactcaggtctcaggactcagtaggggagtgcatctgtggtgaggagcagtgagcc

SEQ ID NO: 955 - DNA, 100 bp, Homo sapiens
  source 1..100: mol_type = other DNA
tactctatggggtgcactcaggtctcaggactcagtaggggagtgcatctgtggtgaggagcagtgagccctcaggtgtgggggtccacgtgtgctctcc

SEQ ID NO: 956 - DNA, 100 bp, Homo sapiens
  source 1..100: mol_type = other DNA
atcagggaatctatctcatttcagcaccatggctctcagtcaagtcttgacgctcctgcttctacagacaggatcttcttcgatgctcccgcaccggaca

SEQ ID NO: 957 - DNA, 100 bp, Homo sapiens
  source 1..100: mol_type = other DNA
tgcaaccttctggttttagtcctagaggattagagtagaaatcaagagagctgccgttcctcctcccttcaagaataatgatggtgggcatctggggggc

SEQ ID NO: 958 - DNA, 100 bp, Homo sapiens
  source 1..100: mol_type = other DNA
aaggggctccccacaagcattctgatcaaaatcctctttgattatggggaaaagtgatgaatttgtgtaaaaaaattggagagaataaataagaaaatac

SEQ ID NO: 959 - DNA, 100 bp, Homo sapiens
  source 1..100: mol_type = other DNA
agttacaagtaattatgtaaagaagtgtgtgcttagcagtgtgtgtgcacacagctgcattcctagaggcatgttccatgaaaaatcgatgttgtccttg

SEQ ID NO: 960 - DNA, 100 bp, Homo sapiens
  source 1..100: mol_type = other DNA
tgccccgtcagttctgtggagagagtagactgcatgaatgacttcccttttctcagcccatgaatgagcggatgctttggacaagggaattggaagactc

SEQ ID NO: 961 - DNA, 100 bp, Homo sapiens
  source 1..100: mol_type = other DNA
ctgagggagcagcaggctgactgttgcagccttgctctgcacctgcactggatgtggtctctgtgctcataaggccgtggaaactcatcaatccaggttc

SEQ ID NO: 962 - DNA, 100 bp, Homo sapiens
  source 1..100: mol_type = other DNA
caaaaaggggttaaatgattttggaaaagtaagtagaaaataaaagaaggagggagtaagagcggacagaagggaggaaggcaagcaagcaatgatgaac

SEQ ID NO: 963 - DNA, 100 bp, Homo sapiens
  source 1..100: mol_type = other DNA
tgtgtaaaattttcactaattaaaagactattatattgaagaggtgcctattaggcagccttttgatgttaaccatgtaatatacaccatgaacaacctt

SEQ ID NO: 964 - DNA, 100 bp, Homo sapiens
  source 1..100: mol_type = other DNA
gaacaaccttgtagaacacacaagagccccctcagagaactggatgggtcaggtctcccatccagttgccttaggggttaggaacgctcccatgttgttc

SEQ ID NO: 965 - DNA, 100 bp, Homo sapiens
  source 1..100: mol_type = other DNA
tctggtttttgctcctgaggacacaaacagccagtgtttcctccccggatgaatagagaggcccctggggagggtgtgtctggcagctcactctgcacct

SEQ ID NO: 966 - DNA, 100 bp, Homo sapiens
  source 1..100: mol_type = other DNA
gtttcctccccggatgaatagagaggcccctggggagggtgtgtctggcagctcactctgcacctgcaccgcggaaggttttagatggtccctctcacac

SEQ ID NO: 967 - DNA, 100 bp, Homo sapiens
  source 1..100: mol_type = other DNA
aataatacatggcggcgtccgaggccttcaggctgctccactgcaggtaggcggtgctgctggagctgtcggctgagatggtgacgtggccttggaagga

SEQ ID NO: 968 - DNA, 100 bp, Homo sapiens
  source 1..100: mol_type = other DNA
tgggctgtatctggtatcagagttcccaggatagatgctccccatccactccagttctttcccgggcatctggcgcacccagtggatccagtagctggta

SEQ ID NO: 969 - DNA, 100 bp, Homo sapiens
  source 1..100: mol_type = other DNA
acaggagatcctcagagactccccgggtcttttcacctctgctgcagactgcaacagctgcacctcggcaaagacacctgtgtgggagacacaaaatttg

SEQ ID NO: 970 - DNA, 100 bp, Homo sapiens
  source 1..100: mol_type = other DNA
gtgtctggagtatgaaccatgtatcagcaccgaaaggttctagaagtcagactttcgggcagtgtgtcactaactctcagcatgctggcctggctcggcc

SEQ ID NO: 971 - DNA, 100 bp, Homo sapiens
  source 1..100: mol_type = other DNA
cacagcaaggtcttctcgcctccctttgggtaaatactgaggggtgcctctgcaggacgggacctctgccagactccactccatacccagagaagcaggg

SEQ ID NO: 972 - DNA, 100 bp, Homo sapiens
  source 1..100: mol_type = other DNA
aaaccaaaattggagtcagccttgaggtgtagctgttgagccctcagcagctggggagagctggcggatgctgccctccccccagtttcctaatggtgtt

SEQ ID NO: 973 - DNA, 100 bp, Homo sapiens
  source 1..100: mol_type = other DNA
gtttaaaaagggtcaggggacgggggaacagatggtgggaagagcacagtgcagacacctggcaccggctctgaaggcagcatggcagctacaccgttgg

SEQ ID NO: 974 - DNA, 100 bp, Homo sapiens
  source 1..100: mol_type = other DNA
ctgggaagggtgtgcccctgaagaagtcgtttacattctcgagtcaattttcctggagtgtacaatggacctgtgggaaagcctgtatgaaagggtaatg

SEQ ID NO: 975 - DNA, 100 bp, Homo sapiens
  source 1..100: mol_type = other DNA
atgagggacctagcacagtgtccaatattttataggaactggaattgagctcataggagctcaattttattggcattgctgttgttggatggttaaaggg

SEQ ID NO: 976 - DNA, 100 bp, Homo sapiens
  source 1..100: mol_type = other DNA
gtggtatcccttttctcagactcccctgaaatgtatggtttgctttgaacccagagactgatgacaggtctgccggtgtggttgggtgcagccttaagtt

SEQ ID NO: 977 - DNA, 100 bp, Homo sapiens
  source 1..100: mol_type = other DNA
gctacgggaaagtgttggagggggagaagtcagaggtaaccttgccccctccctcaattccagatgaggaaattcaggcctgaaaagggaaagtgaccac

SEQ ID NO: 978 - DNA, 100 bp, Homo sapiens
  source 1..100: mol_type = other DNA
ctcaaagtctcatgccttggaggacccagcaggaatccaagacctctgaaaaggaccggcagggctcttgccacggctgggggtgtggtcatggtaacac

SEQ ID NO: 979 - DNA, 100 bp, Homo sapiens
  source 1..100: mol_type = other DNA
aggttttccatccatggaaggtacctgagggattttctcttcctccctagggccagcatcagaggagtgaatagctcagttagctcatctcaggggccat

SEQ ID NO: 980 - DNA, 100 bp, Homo sapiens
  source 1..100: mol_type = other DNA
gtgccctcggaggtggtttgccactttcacggttggactgagttggagagaaacagagacccacccaggggtggggacaagctccctgcaactcaggact

SEQ ID NO: 981 - DNA, 100 bp, Homo sapiens
  source 1..100: mol_type = other DNA
tgcagatcacttgcccaagtggctccctagctcctggctcctggcccggggcctgggactctccccgaagtggggctggccactgtgaggaaccgactgg

SEQ ID NO: 982 - DNA, 100 bp, Homo sapiens
  source 1..100: mol_type = other DNA
aggcagggacctcttggatgccccaggcagttgggatgccacttctgataaagcacgtggtggccacagtaggtgcttggttgctccacagcctggcccg

SEQ ID NO: 983 - DNA, 100 bp, Homo sapiens
  source 1..100: mol_type = other DNA
agctcagcgctgcagaaagaaagtgaaagggaaaaagaactgcggggaggcggggaggtaggatgaccagcggacgagctgccacagacttgccgcggcc

SEQ ID NO: 984 - DNA, 100 bp, Homo sapiens
  source 1..100: mol_type = other DNA
ccagagctggcgggagggagaggccaccagcagcgcgcgcgggagcccggggaacagcggtaggtgaccaaagtctcctctgtaacccctaaggtcgggc

SEQ ID NO: 985 - DNA, 100 bp, Homo sapiens
  source 1..100: mol_type = other DNA
tgagaatcgaggctccgagactgtcagctacttgctcaaggtcacacagcaagtctgggaggatggggggatggaatatgcaaaatgtagggccgggaaa

SEQ ID NO: 986 - DNA, 100 bp, Homo sapiens
  source 1..100: mol_type = other DNA
cacctcgtttccagcatccccgcaacgactctgcgcgggaaccaggagccgggaacccggagcttggcttgctgtgcccagagctccggggccgtgggcg

SEQ ID NO: 987 - DNA, 100 bp, Homo sapiens
  source 1..100: mol_type = other DNA
ggtggcaggaaagcctggcggcagcttctgcagagaagccggagcgcagactgggagcgcggagcagacacactcccccggccacccttggccgactccg

SEQ ID NO: 988 - DNA, 100 bp, Homo sapiens
  source 1..100: mol_type = other DNA
cgcgcccgggatcctgcagaggtgcgcgcccttcttgtacgccagactttggaccagggccgccgttccctgagcttcactttccctgttgggtcatatt

SEQ ID NO: 989 - DNA, 100 bp, Homo sapiens
  source 1..100: mol_type = other DNA
ccatctctaactctggaatcttgggtattgggctctccaggcggggggccctgctcagggaggcagtagggagccaaacctttaaccagaggatgggata

SEQ ID NO: 990 - DNA, 100 bp, Homo sapiens
  source 1..100: mol_type = other DNA
agtcctcaactctcgttgaacatcttggcgaaggtgtgtgttgttgggaggggtgggggagggatccccccggactgaaccgatctcttgatctctcact

SEQ ID NO: 991 - DNA, 100 bp, Homo sapiens
  source 1..100: mol_type = other DNA
tctctacctcgctttggggccctgagtcacaccctctaaggagagaggctaaagcgccccggaaagccagcgtgcgaatgccggggtgggagtgggagat

SEQ ID NO: 992 - DNA, 100 bp, Homo sapiens
  source 1..100: mol_type = other DNA
tggatctccctggggtccaggaaagccggaatcggagccaccatgcttagcttagtctggaactcttaaaagccgcggtcctcctgagtcccacagcccc

SEQ ID NO: 993 - DNA, 100 bp, Homo sapiens
  source 1..100: mol_type = other DNA
tctccaccctaggtggcacaggagaggtggcaaaagcctagaagttcaaggcatggctccctccccagccgcagcctggagtgtctaactttggcaggaa

SEQ ID NO: 994 - DNA, 100 bp, Homo sapiens
  source 1..100: mol_type = other DNA
gtcttccgtttctgctccccactccagagaaaaaataaataaatacttctccggagtgagattaaggaaacaggtacttcttcctcttggagaaagagga

SEQ ID NO: 995 - DNA, 100 bp, Homo sapiens
  source 1..100: mol_type = other DNA
cttctccggagtgagattaaggaaacaggtacttcttcctcttggagaaagaggagccaaaggaacttgactccaacaaatgatcaccttgcaaaccccc

SEQ ID NO: 996 - DNA, 100 bp, Homo sapiens
  source 1..100: mol_type = other DNA
ggctcccttaggggatgacctggtctccaacaatctcagagcgtttggaggcagggtctttggagatgactgagtggggaatcccaggctccccacacat

SEQ ID NO: 997 - DNA, 100 bp, Homo sapiens
  source 1..100: mol_type = other DNA
gaacatcacctgggatgatcaacctgttcaggatgtaggttcccgggctcacccccaggcccggttggctaggcctggggtgaggctgagatcctgcagg

SEQ ID NO: 998 - DNA, 100 bp, Homo sapiens
  source 1..100: mol_type = other DNA
ttaaaccatctatcccaggtgactccaatgttcgtttgtggggcaaaagtccctcaagtcagagacactgggaggcgctgatgtggtctcatctctttac

SEQ ID NO: 999 - DNA, 100 bp, Homo sapiens
  source 1..100: mol_type = other DNA
caagaggtgagaaggggtctgcggcctcgtctccagccgagggcgggaggcgcctcgcccctacacccatccgctccctccaacccaggccggggagggt

SEQ ID NO: 1000 - DNA, 100 bp, Homo sapiens
  source 1..100: mol_type = other DNA
acccacatggttccaggcaagtaataacaaaataacacggcatcccagttaatgctgcgtgcacggcgggcgctgccggtcaaatctggaaggggaagga

SEQ ID NO: 1001 - DNA, 100 bp, Homo sapiens
  source 1..100: mol_type = other DNA
gctcaggtagtcgcggaggacggggttgagggggatgcgagccaggttctcgcggcccacggtggccacgatgcgctggcggcacagctcctgcagcggc

SEQ ID NO: 1002 - DNA, 100 bp, Homo sapiens
  source 1..100: mol_type = other DNA
cgcacgcggcgctggcgcagcggggcccccagcatgcggcgcggcgccgccacgtagtgctccagcagctcgaagaggcagtcgaagctctcgcggctgc

SEQ ID NO: 1003 - DNA, 100 bp, Homo sapiens
  source 1..100: mol_type = other DNA
catccaggtgaaagcggccggcctgaaagtgcacgcggatgctcgtgggtcccgaggccatcttcacgctaagggcgaaaaagcagttccgctggcggct

SEQ ID NO: 1004 - DNA, 100 bp, Homo sapiens
  source 1..100: mol_type = other DNA
gtcgcgcaccaggaaggtgcccacgggctcggcgcgcagccgctcgtgcgccccgtgcacgctcaggggcccccagtagaatccgcaggcgtccaggagc

SEQ ID NO: 1005 - DNA, 100 bp, Homo sapiens
  source 1..100: mol_type = other DNA
gcgctggcgcgcgtgatgcgccggtaatcggcgtgcgaacggaatgtgcggaagtgcgtgtcgccgggggccggggccgggaccgcggggcacggccgcg

SEQ ID NO: 1006 - DNA, 100 bp, Homo sapiens
  source 1..100: mol_type = other DNA
ggcgcgcgggggccgcgggcgaggaggaggaagaggaggaaggttctggccgccgtcggggctctgctgctgtggagactgcattgtcggctgccacctg

SEQ ID NO: 1007 - DNA, 100 bp, Homo sapiens
  source 1..100: mol_type = other DNA
tttaaaatcacccaaatcaaaataattttatcttcattaataaataatcatcagaagtttaactaatttttactttataatactaggtttaaaaattctt

SEQ ID NO: 1008 - DNA, 100 bp, Homo sapiens
  source 1..100: mol_type = other DNA
aatctgaatgcccaagtcgttgattgtcgtttgcctgtttccaaagattggtagatagatgcctttttaaaaatctcatttttctttaaatctggtttac

SEQ ID NO: 1009 - DNA, 100 bp, Homo sapiens
  source 1..100: mol_type = other DNA
atggaaaacgttaggagagctcatataatgaacggcaatagcaaccccctatcttgaaacgcgctctatcatcccactgaaattctaccacgtggaataa

SEQ ID NO: 1010 - DNA, 100 bp, Homo sapiens
  source 1..100: mol_type = other DNA
tgcttggagggtcagagttgtggaactgcccaataaccagtcgttactgagggttagtttgtgaaggaggggacagactgcttctaaaattctgtttaat

SEQ ID NO: 1011 - DNA, 100 bp, Homo sapiens
  source 1..100: mol_type = other DNA
gacagtcaattaagatttctgagtctggcttgagggcctttgcttccatcacagcccagtcgtccttggcaagagagtctgtatatgggccacagctcac

SEQ ID NO: 1012 - DNA, 100 bp, Homo sapiens
  source 1..100: mol_type = other DNA
aaaagcattgtttgaaaaaatttattgaaagaacattgtttgtaaaatgagtcccaatacataggacagactttcctaaggtgagatgtgttacttaccc

SEQ ID NO: 1013 - DNA, 100 bp, Homo sapiens
  source 1..100: mol_type = other DNA
agagctgtgaaaggctttacggatggaaactagagactgaattttccagaattttaagaagtctccccaaccaatggccccccactttctttttttaaac

SEQ ID NO: 1014 - DNA, 100 bp, Homo sapiens
  source 1..100: mol_type = other DNA
ggcgtgatctccgaagcccacagtacactcatccataaagtaggaaacactacaccctccagtgctgttagtagtgctttctactttatgggtgactgca

SEQ ID NO: 1015 - DNA, 100 bp, Homo sapiens
  source 1..100: mol_type = other DNA
ctgtctgtctgtccgtcggcgtgtactcttcaggctgcccaggcctcctgactcctgctccaagagccccccagccctccttgtggcttcctaagatccc

SEQ ID NO: 1016 - DNA, 100 bp, Homo sapiens
  source 1..100: mol_type = other DNA
ccctcttcccttccccctaaaggctccaccccatccccccagtttcagagacactcaggtagagactagggcctctggaggcctcaccttcagttctgtg

SEQ ID NO: 1017 - DNA, 100 bp, Homo sapiens
  source 1..100: mol_type = other DNA
aacccctggctggccgcttccagccacgctagccaccctccagcgtccaaatgaggcagccacagctcccctgccaaggtcttggtctccagtccacccc

SEQ ID NO: 1018 - DNA, 100 bp, Homo sapiens
  source 1..100: mol_type = other DNA
aaccgtgaggtcctgactgcccagagcctcagtccccacccttcagcctccccaccagcccaagatcctgaccccccagggcctaagtccccagcctccc

SEQ ID NO: 1019 - DNA, 100 bp, Homo sapiens
  source 1..100: mol_type = other DNA
caacagcccagggtcctgaccccccagggcctcaggccctggcctccccaccagcccaaggtcttgaacacaccagggcctcaattcccagcctccccac

SEQ ID NO: 1020 - DNA, 100 bp, Homo sapiens
  source 1..100: mol_type = other DNA
cagctcaaggtcctgactcccccagagcctcagtcccagcctccatagcagcccaaggtcctgaccccccagggcctcagtccccagccactccaccagc

SEQ ID NO: 1021 - DNA, 100 bp, Homo sapiens
  source 1..100: mol_type = other DNA
cccaaagtcctgactccccagagccttgattctcggcctccccaccagcccaaagtcctgactccctcactgccctgctgttcccctggcaggagcccaa

SEQ ID NO: 1022 - DNA, 100 bp, Homo sapiens
  source 1..100: mol_type = other DNA
ggctatcccaacaaaaatggtggccatgttgggcggaggaagaggctggcgccccttgagacactggtcccacttctcagcctctgcgtaccctctgcca

SEQ ID NO: 1023 - DNA, 100 bp, Homo sapiens
  source 1..100: mol_type = other DNA
tccccgccttactctccagccctcctccttggacacctctttccccgcctggggtcccggagccattttaccttccttcactagagagggtttcaaggcg

SEQ ID NO: 1024 - DNA, 100 bp, Homo sapiens
  source 1..100: mol_type = other DNA
ctaagattttcaagaagttaaacgtagaattaagattgttctaattctggttgtaaactgctattttaaaaaacaaaacaaacagaaaacatcaaaaaca

SEQ ID NO: 1025 - DNA, 100 bp, Homo sapiens
  source 1..100: mol_type = other DNA
aaacaaacagaaaacatcaaaaacacaaaaagatattaaaacagcaagtcttttgtacatcactgtagcataagctgcttgaggttgtcatgcagaatag

SEQ ID NO: 1026 - DNA, 100 bp, Homo sapiens
  source 1..100: mol_type = other DNA
tatccttcacgtcacggaaaacaaggcggatgttctccgtgttgatagcagtggtgaagtggtggtataagggcttctgttgctggtcccggcgtttgtt

SEQ ID NO: 1027 - DNA, 100 bp, Homo sapiens
  source 1..100: mol_type = other DNA
ccggaaacattccaccaggaatttttggacgtctcttaagcagtggggatccccttcaaattctaggaaatagtctttgatgctcacaatttgcaccttc

SEQ ID NO: 1028 - DNA, 100 bp, Homo sapiens
  source 1..100: mol_type = other DNA
tcctcaagcaagtctgtcttgtttaagaacagaattatggagacattgctgaaaacccggttattgacgattgtttcaaaaatgttcagagactctgtaa

SEQ ID NO: 1029 - DNA, 100 bp, Homo sapiens
  source 1..100: mol_type = other DNA
ggcgattggtcagtcgatcttccataagcacctggtcaaattcacttgaggaaacaaggaaaagtattgatgtcacactgtcgaaacattcaaaccaacg

SEQ ID NO: 1030 - DNA, 100 bp, Homo sapiens
  source 1..100: mol_type = other DNA
tttcctttctgatctctgaccacctacatcaaccattttgaaaggaacattttttatttcaaagtcgtattcatggatgcctttggtgggtcttctggca

SEQ ID NO: 1031 - DNA, 100 bp, Homo sapiens
  source 1..100: mol_type = other DNA
agcagaatatcttgttgtgatggaatataatcctggaaaagaaaaaacttgttttatacctattaatcccgaagtaatgcgaatttttaatggactacta

SEQ ID NO: 1032 - DNA, 100 bp, Homo sapiens
  source 1..100: mol_type = other DNA
tgtaaatatttggccaactaagctgagtggctaagttctcctgctgcccggagcttcttggaacatgtttccttttcgcaaggggtttccctggcttcca

SEQ ID NO: 1033 - DNA, 100 bp, Homo sapiens
  source 1..100: mol_type = other DNA
ggagggccaggaagaaattcgaattggccaccgctttctctaaaatcactccgctcaagttatcacccctctgggctcccgaagaccggctggctggagg

SEQ ID NO: 1034 - DNA, 100 bp, Homo sapiens
  source 1..100: mol_type = other DNA
ctggagatagtctcaatgctcgaaatgccgtaaccgaagctccccgcggcgccggcactgggatccagggagctgctgctacagcgcagctctggattcc

SEQ ID NO: 1035 - DNA, 100 bp, Homo sapiens
  source 1..100: mol_type = other DNA
tggatgtgttggatatgtgcagggcgttcctgggaggagcggggagggagggtgctgctggcggggctggtctgcgtgtgctttgcttctctacaatggc

SEQ ID NO: 1036 - DNA, 100 bp, Homo sapiens
  source 1..100: mol_type = other DNA
atgctgcgtgtcggccatgcagaggcatgtcagtgagcaggggctgagggatctccctaacggacctgctttcagagggtcttttcatgctgggagaacc

SEQ ID NO: 1037 - DNA, 100 bp, Homo sapiens
  source 1..100: mol_type = other DNA
ccagagactaaatcatgcagccaacggggtggtccccggcctcaaagcagggaggggcgaggagctttgtaggcaatgccatctgctcctgaaacgccgt

SEQ ID NO: 1038 - DNA, 100 bp, Homo sapiens
  source 1..100: mol_type = other DNA
cagcctccttagtagctaccgccttagtaagtaccacttagtaagtaccgccttagtaagtaccacttagtagctacctccttagtaagtaccacttagt

SEQ ID NO: 1039 - DNA, 100 bp, Homo sapiens
  source 1..100: mol_type = other DNA
aagtacctccttagtaagtaccacttagtactaccaccacgcctggctaatttcgtatttttttttttttagtagagacggggtttctccatattggtca

SEQ ID NO: 1040 - DNA, 100 bp, Homo sapiens
  source 1..100: mol_type = other DNA
aggtcaggcgcatactgcatgcgggtctcgcggtcgtgctccagccacagcacggacatctggaagagcgccagctccgactccacggggggcggcagcg

SEQ ID NO: 1041 - DNA, 100 bp, Homo sapiens
  source 1..100: mol_type = other DNA
agtccagcagggcgcgcatctcctcgaagttgagcagcagcacatcctccaccaggtacttgttggccagcttcttggtctcctccaggccgtgcagcgc

SEQ ID NO: 1042 - DNA, 100 bp, Homo sapiens
  source 1..100: mol_type = other DNA
ggcgatcttgcacacctgcttgtagttctgcaccgagatctggtcgttgaggaactgcacgcagagcttggtgacctgggggatgtgcaggatcttgctg

SEQ ID NO: 1043 - DNA, 100 bp, Homo sapiens
  source 1..100: mol_type = other DNA
accgacagcacctcctccaccgtgtccagggacagggtcacgttggccgtgtagaggtactcgagcaccaggcgcagcccgatggacgagcagccctgca

SEQ ID NO: 1044 - DNA, 100 bp, Homo sapiens
  source 1..100: mol_type = other DNA
gcaccaggttgttgatggcccgggggctggtcagcagcttgtcgtcgggggaggaagaaggagtcccgggctcctcctgcggcggcggctgctgctgctg

SEQ ID NO: 1045 - DNA, 100 bp, Homo sapiens
  source 1..100: mol_type = other DNA
tgacggctgctgctgcggcggctgctgctggtccttgggggcccccaggccgtcctggccgccgacccctcccccgagaggggggtggctggagaagagc

SEQ ID NO: 1046 - DNA, 100 bp, Homo sapiens
  source 1..100: mol_type = other DNA
gagacttcagccggagctggctattccagagatggacctcagaggattccttagtctaattaccttctgggctggggtagaagatggtgtctggagggaa

SEQ ID NO: 1047 - DNA, 100 bp, Homo sapiens
  source 1..100: mol_type = other DNA
gcacagaaccaagttccctactgccgcactagctatgcaaatactgcagggcacctgtgggctcatgtccctcctgcaagaaggtgtggtcagtccagta

SEQ ID NO: 1048 - DNA, 100 bp, Homo sapiens
  source 1..100: mol_type = other DNA
attcaaaagacgtacttctgaaataggtggagaaatgcatttatagcaaaaagtgctaaaaatatgttaatagttatgctatttggttcaccaggttagt

SEQ ID NO: 1049 - DNA, 100 bp, Homo sapiens
  source 1..100: mol_type = other DNA
gtaataaaccataacaagagagactaaaggccgtatctatatgaccttgaaatctcatcttcagcgggcttattcattcagtaaccaaactatttttgta

SEQ ID NO: 1050 - DNA, 100 bp, Homo sapiens
  source 1..100: mol_type = other DNA
aggtgctgagtatttagcttaaagctaaataagacacatgccctgccctatagtaactgcttggtaatattcccagtggcttccatgggcctgataattt

SEQ ID NO: 1051 - DNA, 100 bp, Homo sapiens
  source 1..100: mol_type = other DNA
tcttagtactgaattcaaagcactttgtgtcttgtctgcaggcccatttgcccagcagtggccttgccaggagagaacaggcccatgctcctgtcctcat

SEQ ID NO: 1052 - DNA, 100 bp, Homo sapiens
  source 1..100: mol_type = other DNA
caaacaaacaattcaagaagaggatttaaattttagaaatttaaattggggcattttagttaatcttacttttaaacaccaaacagtggcatcaatattt

SEQ ID NO: 1053 - DNA, 100 bp, Homo sapiens
  source 1..100: mol_type = other DNA
tgtcaactttggtcaaataagatcagatgttcacatcaatcatctacttttcttggccttttctctatttggcctcctagtatgagcacactttgtaaaa

SEQ ID NO: 1054 - DNA, 100 bp, Homo sapiens
  source 1..100: mol_type = other DNA
tgtaataaaaacatgtggtgtgcttcttgacatctaatccacttgcagtaatttctaggctttttgctcctgttaggtcctataaaataatgacattagt

SEQ ID NO: 1055 - DNA, 100 bp, Homo sapiens
  source 1..100: mol_type = other DNA
atagatacctagatgcaaatttttttcagccgaccacaaaattaggtccactctgagtggtgaaaaacaaaagattctaacattctagcaaactggtaaa

SEQ ID NO: 1056 - DNA, 100 bp, Homo sapiens
  source 1..100: mol_type = other DNA
ccatacacaaattatagaatacaaagaatgcagccgatgcaaattctgtcactgacaaggtagcaaagccatagcctgatactcctcaggacacctcatc

SEQ ID NO: 1057 - DNA, 100 bp, Homo sapiens
  source 1..100: mol_type = other DNA
acgcccactgggaacatggcacacactggagattccagtccaaggactttggaatgtcaacttagctctttacaaacacaactaagtttttcagggaaaa

SEQ ID NO: 1058 - DNA, 100 bp, Homo sapiens
  source 1..100: mol_type = other DNA
agacttacattggttttcctcttttggaaaattttaccgattgatgatgcccttggtcttctgtggagtctattcttctaatcgggttgttctccaattt

SEQ ID NO: 1059 - DNA, 100 bp, Homo sapiens
  source 1..100: mol_type = other DNA
tagtgtacaacgggcttgtttcaggggagcttgtttgggatgcagactgtcaagacccaacctggtatctggttcataagcagtccctgaaacctccctc

SEQ ID NO: 1060 - DNA, 100 bp, Homo sapiens
  source 1..100: mol_type = other DNA
cggttccaacaagctgctcaagccaggaaacggtggtcctggggactcctggaccttcagcttgagaaacactgaaggggtaccatttaccaccacatcc

SEQ ID NO: 1061 - DNA, 100 bp, Homo sapiens
  source 1..100: mol_type = other DNA
tactggattacaaacgctagatctttggatctccacgactagcaagcaagttaaagacttttagatggcaggcgttatcggtcaggttgggagtgaacgc

SEQ ID NO: 1062 - DNA, 100 bp, Homo sapiens
  source 1..100: mol_type = other DNA
tttgtccagaggaggaggtagggacgccgggaagcaacaactctgattttatttcgccggctccacagcctcccattgccccaggagcccacccgcactc

SEQ ID NO: 1063 - DNA, 100 bp, Homo sapiens
  source 1..100: mol_type = other DNA
caacccccgcatctcggacctgtggcctcagcccagactcacatcaccaagtgcacctacccagcctccgttatcctggatccaggtgtgcaggtgccgg

SEQ ID NO: 1064 - DNA, 100 bp, Homo sapiens
  source 1..100: mol_type = other DNA
ttcaggtactcagtcatccacagggcgatgttgtccaccaggggcgacatctcccggttgacgctctccacacacatgaccccaccgaactcaaagaagg

SEQ ID NO: 1065 - DNA, 100 bp, Homo sapiens
  source 1..100: mol_type = other DNA
ccacaatcctcccccagttcaccccgtccctgaagagctcctccaccaccgtggcaaagcgtccccgcgcggtgaagggcgtcaggtgcagctggctgga

SEQ ID NO: 1066 - DNA, 100 bp, Homo sapiens
  source 1..100: mol_type = other DNA
catctcggcgaagtcgcggcggtagcggcgggagaagtcgtcgccggcctggcggagggtcaggtggaccacaggtggcaccgggctgagcgcaggcccc

SEQ ID NO: 1067 - DNA, 100 bp, Homo sapiens
  source 1..100: mol_type = other DNA
gcggcggcgccgggggcagccggggtctgcagcggcgaggtcctggcgaccgggtcccgggatgcggctggatggggcgtgtgcccgggctgggaggaga

SEQ ID NO: 1068 - DNA, 100 bp, Homo sapiens
  source 1..100: mol_type = other DNA
agatgcccggtgcgggggcggcccccgggggcgcggcgcccacatctcccgcatcccactcgtagcccctctgcgacagcttataatggatgtacttcat

SEQ ID NO: 1069 - DNA, 100 bp, Homo sapiens
  source 1..100: mol_type = other DNA
cactatctcccggttatcgtaccctgttctcccagcgtgcgccatccttcccagaggaaaagcaacgggggccaacggcacctctcgccccagctcccac

SEQ ID NO: 1070 - DNA, 100 bp, Homo sapiens
  source 1..100: mol_type = other DNA
cccacggcccccagagaaagaagaggagttataatccagctattttattggatgtgctttgcattcttggacgagggggtgtcttcaatcacgcggaaca

SEQ ID NO: 1071 - DNA, 100 bp, Homo sapiens
  source 1..100: mol_type = other DNA
cttgattctggtgtttcccccttggcatgagatgcaggaaatttttattccaattcctttcggatctttatttcatgaggcacgttattattagtaagta

SEQ ID NO: 1072 - DNA, 100 bp, Homo sapiens
  source 1..100: mol_type = other DNA
ttgttaatatcagtctacttcctctgtgatgctgaaaggttaaagaaaaaacaaactaataagtaaaaaatcaggtgcgtttccctgtacacactgagtg

SEQ ID NO: 1073 - DNA, 100 bp, Homo sapiens
  source 1..100: mol_type = other DNA
aaagcagggcatacacactacaagtaacacggctaaaaagaatgtattaagctgcctggaaattaaatttactcgaatgcactttaagtaaaaaatctca

SEQ ID NO: 1074 - DNA, 100 bp, Homo sapiens
  source 1..100: mol_type = other DNA
aaggtttccattgaaagttacattaaaccaatttcctgtgcagagaacttacttgtattttttaagtacagcatgatcctctgtcaagtttcctttttgt

SEQ ID NO: 1075 - DNA, 100 bp, Homo sapiens
  source 1..100: mol_type = other DNA
aaaaccaaaacaaatgcataaggcaacgatcccatcaatcttcagcactctccagttatagctgatttgaaacttcccaatgaatcaggagtcgcgggga

SEQ ID NO: 1076 - DNA, 100 bp, Homo sapiens
  source 1..100: mol_type = other DNA
gagggagtaaaaattaggaggatttccagatcgattcccagacttctgcttcacagaaatgtcaatccgcaggaatcccaaccggagatctcaagagctc

SEQ ID NO: 1077 - DNA, 100 bp, Homo sapiens
  source 1..100: mol_type = other DNA
gagaaaaaaaaaaggcagcggcggcggcagatgaattacaattttcagtccggtattcgcagaagtcctgtgatgttttccccttctcggcaatttacac

SEQ ID NO: 1078 - DNA, 100 bp, Homo sapiens
  source 1..100: mol_type = other DNA
tgaaggagccggggacggaggcaggaatcctcttctgattaaactccgaacagcaaatgcattttccgaaaagctgctggataaatgaaggcaggacgcg

SEQ ID NO: 1079 - DNA, 100 bp, Homo sapiens
  source 1..100: mol_type = other DNA
cctggcccgccggtgccgagcgctagaagcccgcgctgtgtgtggtgcggcgaggggtggggagaaggaggtggtgggggagggttttattttttccctc

SEQ ID NO: 1080 - DNA, 100 bp, Homo sapiens
  source 1..100: mol_type = other DNA
ttttcctaaaaaggatgactgctacgaagttctcccccctggaccccctcttccgctgcaccccaccggcgcaccccgcctccgggctgcgcaccctttc

SEQ ID NO: 1081 - DNA, 100 bp, Homo sapiens
  source 1..100: mol_type = other DNA
gtgtgtgtctcgcctggaccttttctagccgtgtatgtgggagtgtgtgtgtcgcctggaccctttctagccgtgtatgagagtgtgtacacgcgcctac

SEQ ID NO: 1082 - DNA, 100 bp, Homo sapiens
  source 1..100: mol_type = other DNA
acacacacacgttgtgttaccggcgctcggccgccgggggaagacccaggccaatgccgccccccaccgcccccagcagtgggacctcagcgctgccctg

SEQ ID NO: 1083 - DNA, 100 bp, Homo sapiens
  source 1..100: mol_type = other DNA
ctgtgaagacaggtgactctgcacgttttaagcaatgtctagggacgccccgagcgtggtgtttactttcaagtagcttcctaggtgtccgcgcactaca

SEQ ID NO: 1084 - DNA, 100 bp, Homo sapiens
  source 1..100: mol_type = other DNA
cacgcacgcgcatccccgcccgtgtccacctgaacacctagtccgtggcccaggccatgcagaactcagcgctccagggaaggggtttatcaagggcttt

SEQ ID NO: 1085 - DNA, 100 bp, Homo sapiens
  source 1..100: mol_type = other DNA
acgacagtttaagtcaatgttttccctctgtccctaacaccttttacactggtttagtgctacacgatgaggacttccatatagtaactttcaggcccac

SEQ ID NO: 1086 - DNA, 100 bp, Homo sapiens
  source 1..100: mol_type = other DNA
cgtcctaacgctggggtgggtgggctcctaaaggtctccacctttgcctcgtagccaatcctagttggccgcactttctcaaatgaggtacatagataca

SEQ ID NO: 1087 - DNA, 100 bp, Homo sapiens
  source 1..100: mol_type = other DNA
gtgtctccatggagatggcagcaggacccgaccccgtgctggcccgcactctcggcctccttatctggtttaggaatgcgcggtatccacgctcgctcgc

SEQ ID NO: 1088 - DNA, 100 bp, Homo sapiens
  source 1..100: mol_type = other DNA
gcgggagccacgcctcctctcccccccgcccccgagaccgccacacgcgcggggcccccacgtctccaagcggcactggaaggattcctctccgtcccgc

SEQ ID NO: 1089 - DNA, 100 bp, Homo sapiens
  source 1..100: mol_type = other DNA
caggggtcccgcctcgagattctgggaagactgggggtgggggaccagatcgcagcagcagctgcaccgcgagttccgcgcctggccgtgtcgccccacg

SEQ ID NO: 1090 - DNA, 100 bp, Homo sapiens
  source 1..100: mol_type = other DNA
agggggactgtgggctcagcgcgtggggcccggagcatctgacaaggacagagacagaggagggggtggaaatccccgggtgagtcaacccgtgcctgag

SEQ ID NO: 1091 - DNA, 100 bp, Homo sapiens
  source 1..100: mol_type = other DNA
aagggggcgagttccgacgctccgcccggctcggggccacgcgaggtccgcgccacgcgcgccttcacccacgacccatccctgagccggagttgaaaga

SEQ ID NO: 1092 - DNA, 100 bp, Homo sapiens
  source 1..100: mol_type = other DNA
ggaggcgtctgagccacgcagtcactttctctttccttacaaaacaaagccacgccccccgccgggggaccggaggaggcaaacaacttggggaaaccga

SEQ ID NO: 1093 - DNA, 100 bp, Homo sapiens
  source 1..100: mol_type = other DNA
cccactttccccttctgtccctaaagttttttcttcctcttgcctcccccagcccttttgaaagctccccgcgtcgtcctcctgctgccccggctcctta

SEQ ID NO: 1094 - DNA, 100 bp, Homo sapiens
  source 1..100: mol_type = other DNA
gcagcttctgggacgcacgggagggaaaagccgcggggaccccccccaccccagcctcccagccgggtgagatttggttgctgtgtttcctcctcacttg

SEQ ID NO: 1095 - DNA, 100 bp, Homo sapiens
  source 1..100: mol_type = other DNA
ccaccccagcctcccagccgggtgagatttggttgctgtgtttcctcctcacttgggcatttaaaaaatattttaacacgaattgtccgcggaattttca

SEQ ID NO: 1096 - DNA, 100 bp, Homo sapiens
  source 1..100: mol_type = other DNA
catggcctggacccctctcctcctccagcttctcaccctctgctcaggtgactgcctgtggaatgccaaagtgattattggggacacatgggatgacttt

SEQ ID NO: 1097 - DNA, 100 bp, Homo sapiens
  source 1..100: mol_type = other DNA
tctcttatattttaacattgtggggtgggtagtgaacccagactcacctctctgtgcctgcctcctctgttccagggtcctgggcacagtctgcgctgac

SEQ ID NO: 1098 - DNA, 100 bp, Homo sapiens
  source 1..100: mol_type = other DNA
ccaggaagcctcggtgtcagggaccgtgggacagaaggtcaccctctcctgtactggaaacagcaacaacgttggaagttatgctgtgggctggtaccaa

SEQ ID NO: 1099 - DNA, 100 bp, Homo sapiens
  source 1..100: mol_type = other DNA
cagatttctcacggtgctcccaaaactgtgatgtttggaaattctctgccctcagggatccctgaccgcttctctggctcaaagtctgggaccacagcct

SEQ ID NO: 1100 - DNA, 100 bp, Homo sapiens
  source 1..100: mol_type = other DNA
ccctgactatctcgggcctctagcctgaggacgaggctgattattactgttcaacatgggactacagcctcagtgctcacacagtgctgcaggcacatgg

SEQ ID NO: 1101 - DNA, 100 bp, Homo sapiens
  source 1..100: mol_type = other DNA
ggaaccgagacaaaaacctgcccttggcctgtcccgaggctgatcactccatacttgcctatgacaaacaaagagggtgcctgtggctgatcgtacagtt

SEQ ID NO: 1102 - DNA, 100 bp, Homo sapiens
  source 1..100: mol_type = other DNA
gaaatgttgtttgctcttgtccttccttcaggccataatgagcgtctctgttttcagggtctctctcccagcctgtgctgactcaatcatcctctgcctc

SEQ ID NO: 1103 - DNA, 100 bp, Homo sapiens
  source 1..100: mol_type = other DNA
tcaagctcacctgcactctgagcagtgggcacagtagctacatcatcgcatggcatcagcagcagccagggaaggcccctcggtacttgatgaagcttga

SEQ ID NO: 1104 - DNA, 100 bp, Homo sapiens
  source 1..100: mol_type = other DNA
aggtagtggaagctacaacaaggggagcggagttcctgatcgcttctcaggctccagctctggggctgaccgctacctcaccatctccaacctccagttt

SEQ ID NO: 1105 - DNA, 100 bp, Homo sapiens
  source 1..100: mol_type = other DNA
gaggatgaggctgattattactgtgagacctgggacagtaacactcacacagtgatacaggcagatgaggaagtgggacaaaatcctcaacctgctgagg

SEQ ID NO: 1106 - DNA, 100 bp, Homo sapiens
  source 1..100: mol_type = other DNA
aaggtcaccatctcctgctctggaagcagctccaacattgggaataattatgtatcctggtaccagcagctcccaggaacagcccccaaactcctcattt

SEQ ID NO: 1107 - DNA, 100 bp, Homo sapiens
  source 1..100: mol_type = other DNA
atgacaataataagcgaccctcagggattcctgaccgattctctggctccaagtctggcacgtcagccaccctgggcatcaccggactccagactgggga

SEQ ID NO: 1108 - DNA, 100 bp, Homo sapiens
  source 1..100: mol_type = other DNA
tcagccagactcacctgcaccttgcgcagtggcatcaatcttggtagctacaggatattctggtaccagcagaagccagagagccctccccggtatctcc

SEQ ID NO: 1109 - DNA, 100 bp, Homo sapiens
  source 1..100: mol_type = other DNA
tgagctactactcagactcaagtaagcatcagggctctggagtccccagccgcttctctggatccaaagatgcttcgagcaatgcagggattttagtcat

SEQ ID NO: 1110 - DNA, 100 bp, Homo sapiens
  source 1..100: mol_type = other DNA
agagatctgggggaagctcagcttcagctgtggtagagaagacaggattcaggacaatctccagcatggccggcttccctctcctcctcaccctcctcac

SEQ ID NO: 1111 - DNA, 100 bp, Homo sapiens
  source 1..100: mol_type = other DNA
tcactgtgcaggtgacaggatggggaccaagagaggggccctgggaagcccatggggccctgctttctcctcttgtctcctttcgtctcttgtcaatcac

SEQ ID NO: 1112 - DNA, 100 bp, Homo sapiens
  source 1..100: mol_type = other DNA
catgtctgtgtctctctcacttccagggtcctgggcccagtctgtgctgactcagccaccctcagcgtctgggacccccgggcagagggtcaccatctct

SEQ ID NO: 1113 - DNA, 100 bp, Homo sapiens
  source 1..100: mol_type = other DNA
tgttctggaagcagctccaacatcggaagtaattatgtatactggtaccagcagctcccaggaacggcccccaaactcctcatctatagtaataatcagc

SEQ ID NO: 1114 - DNA, 100 bp, Homo sapiens
  source 1..100: mol_type = other DNA
ggccctcaggggtccctgaccgattctctggctccaagtctggcacctcagcctccctggccatcagtgggctccggtccgaggatgaggctgattatta

SEQ ID NO: 1115 - DNA, 100 bp, Homo sapiens
  source 1..100: mol_type = other DNA
atttgcataaagcagcacacagcacaccccctccgtgcggagagctcaataggagataaagagccatcagaatccagccccagctctggcaccaggggtc

SEQ ID NO: 1116 - DNA, 100 bp, Homo sapiens
  source 1..100: mol_type = other DNA
ccttccaatatcagcaccatggcctggactcctctctttctgttcctcctcacttgctgcccaggttaagagagatttcaaataccagcctttggaggga

SEQ ID NO: 1117 - DNA, 100 bp, Homo sapiens
  source 1..100: mol_type = other DNA
tccctttttctccctttctaattcctaatatatgtctgttttttttgtttcagggtccaattcccaggctgtggtgactcaggagccctcactgactgtg

SEQ ID NO: 1118 - DNA, 100 bp, Homo sapiens
  source 1..100: mol_type = other DNA
ggacagtcactctcacctgtggctccagcactggagctgtcaccagtggtcattatccctactggttccagcagaagcctggccaagcccccaggacact

SEQ ID NO: 1119 - DNA, 100 bp, Homo sapiens
  source 1..100: mol_type = other DNA
gatttatgatacaagcaacaaacactcctggacacctgcccggttctcaggctccctccttgggggcaaagctgccctgacccttttgggtgcgcagcct

SEQ ID NO: 1120 - DNA, 100 bp, Homo sapiens
  source 1..100: mol_type = other DNA
gaggatgaggctgagtattactgcttgctctcctatagtggtgctcggcacagtgacagacccatgagaggaaccaagacataaacctccctcggccctt

SEQ ID NO: 1121 - DNA, 100 bp, Homo sapiens
  source 1..100: mol_type = other DNA
ggtcagccacccagcctgattctgactcttctggcaaagatccctgaaaaactttaccctggtttctgccttagcacccattaatgtctgtgtttccagg

SEQ ID NO: 1122 - DNA, 100 bp, Homo sapiens
  source 1..100: mol_type = other DNA
ttccctctcgcaggctgtgctgactcagccgtcttccctctctgcatctcctggagcatcagccagtctcacctgcaccttgcgcagtggcatcaatgtt

SEQ ID NO: 1123 - DNA, 100 bp, Homo sapiens
  source 1..100: mol_type = other DNA
gcatcagccagtctcacctgcaccttgcgcagtggcatcaatgttggtacctacaggatatactggtaccagcagaagccagggagtcctccccagtatc

SEQ ID NO: 1124 - DNA, 100 bp, Homo sapiens
  source 1..100: mol_type = other DNA
tcctgaggtacaaatcagactcagataagcagcagggctctggagtccccagccgcttctctggatccaaagatgcttcggccaatgcagggattttact

SEQ ID NO: 1125 - DNA, 100 bp, Homo sapiens
  source 1..100: mol_type = other DNA
acagatggggaagtgggacaaaaacctcaccctgctctgggtcttgctctgtaccaatttttaaattttaaaataactggcctaggcacaaactatattt

SEQ ID NO: 1126 - DNA, 100 bp, Homo sapiens
  source 1..100: mol_type = other DNA
gcccagtctgtgctgactcagccaccctcagcgtctgggacccccgggcagagggtcaccatctcttgttctggaagcagctccaacatcggaagtaata

SEQ ID NO: 1127 - DNA, 100 bp, Homo sapiens
  source 1..100: mol_type = other DNA
ctgtaaactggtaccagcagctcccaggaacggcccccaaactcctcatctatagtaataatcagcggccctcaggggtccctgaccgattctctggctc

SEQ ID NO: 1128 - DNA, 100 bp, Homo sapiens
  source 1..100: mol_type = other DNA
tgctgctcaggcctggcctgtggcttctgctgctgcagcttccttcatgggtccaggggcatccagggccctgcctgagagtggaggctcctcctcccct

SEQ ID NO: 1129 - DNA, 100 bp, Homo sapiens
  source 1..100: mol_type = other DNA
tccagcactggagcagtcaccagtggttactatccaaactggttccagcagaaacctggacaagcacccagggcactgatttatagtacaagcaacaaac

SEQ ID NO: 1130 - DNA, 100 bp, Homo sapiens
  source 1..100: mol_type = other DNA
ccctccttgggggcaaagctgccctgacactgtcaggtgtgcagcctgaggacgaggctgagtattactgcctgctctactatggtggtgctcagcacag

SEQ ID NO: 1131 - DNA, 100 bp, Homo sapiens
  source 1..100: mol_type = other DNA
tgacagactcataagaggaaccaagacataaacctccctcggcccttgtgatgtggagattgtgtgatcatacacaccagctctcaagacagcctacatg

SEQ ID NO: 1132 - DNA, 100 bp, Homo sapiens
  source 1..100: mol_type = other DNA
acataaacctccctcggcccttgtgatgtggagattgtgtgatcatacacaccagctctcaagacagcctacatgtggaccagccatagaaaggggaagg

SEQ ID NO: 1133 - DNA, 100 bp, Homo sapiens
  source 1..100: mol_type = other DNA
atagaaaggggaaggaaagggtctgaattgatttctatccctccttgtgccctgaagtggaggaaatgtgagagtgatttgcagtaattgaatgagacaa

SEQ ID NO: 1134 - DNA, 100 bp, Homo sapiens
  source 1..100: mol_type = other DNA
agcaaaagttatttgttttatatgaaaaaaaaaaacagaaacagcaggatcagatctaaaggctgagtctaaatgcatttcctccagacagaagcttctt

SEQ ID NO: 1135 - DNA, 100 bp, Homo sapiens
  source 1..100: mol_type = other DNA
cagatctaaaggctgagtctaaatgcatttcctccagacagaagcttcttcaaacgatgggctttctgagctaagagcaaagaaaataaactctccacgg

SEQ ID NO: 1136 - DNA, 100 bp, Homo sapiens
  source 1..100: mol_type = other DNA
gtatattattaaagtttattttattgagttactttcaaagcaatccatgactattatataaagtcagaaagtattaaaaatcaccaagttctctgctaag

SEQ ID NO: 1137 - DNA, 100 bp, Homo sapiens
  source 1..100: mol_type = other DNA
ctaccttatcccatgcaatcaaaataagtacttttcttcatttggatgcattttttatttctgtttttaatatttccacaatggtgattaaacctggtgc

SEQ ID NO: 1138 - DNA, 100 bp, Homo sapiens
  source 1..100: mol_type = other DNA
acagggtcaggggaggggtccaggaagcccatgaggccctgctttctccttctctctctagaccaagaatcaccgtgtctgtgtctctcctgcttccacg

SEQ ID NO: 1139 - DNA, 100 bp, Homo sapiens
  source 1..100: mol_type = other DNA
gtcctgggcccagtctgtgttgacgcagccgccttcagtgtctgcggccccaggacagaaggtcaccatctcctgctctggaagcagctccgacatgggg

SEQ ID NO: 1140 - DNA, 100 bp, Homo sapiens
  source 1..100: mol_type = other DNA
aattatgcggtatcctggtaccagcagctcccaggaacagcccccaaactcctcatctatgaaaataataagcgaccctcagggattcctgaccgattct

SEQ ID NO: 1141 - DNA, 100 bp, Homo sapiens
  source 1..100: mol_type = other DNA
ctggctccaagtctggcacctcagccaccctgggcatcactggcctctggcctgaggactaggccgattattactgcttagcatgggataccagcctgag

SEQ ID NO: 1142 - DNA, 100 bp, Homo sapiens
  source 1..100: mol_type = other DNA
agcttgcacagtgctccaggccaatggggaactgagacaagaaccctcttcctcctccgccaggagggtgagtgcctgcagctgctgctcacacctgacc

SEQ ID NO: 1143 - DNA, 100 bp, Homo sapiens
  source 1..100: mol_type = other DNA
tgtagcttctgctgctgtagcttcccccatgggcctcggggcatccagggccttgcctaggagtggaggctccaccacttttgtcctcagagtcaggaac

SEQ ID NO: 1144 - DNA, 100 bp, Homo sapiens
  source 1..100: mol_type = other DNA
agggaccccaggagacagaatatcctgctcctcagcttgggacacagggtctctgcactgaaatcgtgggctgaggtggcaggtccaactgtgtcttcac

SEQ ID NO: 1145 - DNA, 100 bp, Homo sapiens
  source 1..100: mol_type = other DNA
ctctgcactgaaatcgtgggctgaggtggcaggtccaactgtgtcttcacagtccttcctgtgcctgcccatggtgtggggacggagtgaggaagtgtgg

SEQ ID NO: 1146 - DNA, 100 bp, Homo sapiens
  source 1..100: mol_type = other DNA
tcctcactctcctcgctcactgcacaggtgactggatacaggtccaggggaggggccctgggaagcctatggattcttgctttctcctgttgtctctaga

SEQ ID NO: 1147 - DNA, 100 bp, Homo sapiens
  source 1..100: mol_type = other DNA
agccgaataatgatgcctgtgtctctcccacttccagggtcctgggcccagtctgtgctgacgcagccgccctcagtgtctggggccccagggcagaggg

SEQ ID NO: 1148 - DNA, 100 bp, Homo sapiens
  source 1..100: mol_type = other DNA
tcaccatctcctgcactgggagcagctccaacatcggggcaggttatgatgtacactggtaccagcagcttccaggaacagcccccaaactcctcatcta

SEQ ID NO: 1149 - DNA, 100 bp, Homo sapiens
  source 1..100: mol_type = other DNA
ctccaggctgaggatgaggctgattattactgccagtcctatgacagcagcctgagtggttccacagtgctccaggcccggggggaactgagacaagaac

SEQ ID NO: 1150 - DNA, 100 bp, Homo sapiens
  source 1..100: mol_type = other DNA
gctcctcactctcctcactcaggacacaggtgacgcctccagggaaggggtcttggggacctctgggctgatccttggtctcctgctcctcaggctcacc

SEQ ID NO: 1151 - DNA, 100 bp, Homo sapiens
  source 1..100: mol_type = other DNA
ttccagggtcctgggcccagtctgccctgactcagcctgcctccgtgtctgggtctcctggacagtcgatcaccatctcctgcactggaaccagcagtga

SEQ ID NO: 1152 - DNA, 100 bp, Homo sapiens
  source 1..100: mol_type = other DNA
tgttgggagttataaccttgtctcctggtaccaacagcacccaggcaaagcccccaaactcatgatttatgagggcagtaagcggccctcaggggtttct

SEQ ID NO: 1153 - DNA, 100 bp, Homo sapiens
  source 1..100: mol_type = other DNA
aatcgcttctctggctccaagtctggcaacacggcctccctgacaatctctgggctccaggctgaggacgaggctgattattactgctgctcatatgcag

SEQ ID NO: 1154 - DNA, 100 bp, Homo sapiens
  source 1..100: mol_type = other DNA
gctgaggacgaggctgattattactgctgctcatatgcaggtagtagcactttccacagtggtccaagttcatggggaactgagaccaaaacctgcccag

SEQ ID NO: 1155 - DNA, 100 bp, Homo sapiens
  source 1..100: mol_type = other DNA
ggccttcagacttcctccttgctctgaagatgcttcctcacccggtgcaagaggcttgctgcagcgcggccttgagaattcttctctctcagctccttcc

SEQ ID NO: 1156 - DNA, 100 bp, Homo sapiens
  source 1..100: mol_type = other DNA
ctttccaccatgaattccaacaggaaacctgccctgtggtttcccatccaggacagggacagcttcctgatgcttgtgtgctgtggtccctgaatgtgca

SEQ ID NO: 1157 - DNA, 100 bp, Homo sapiens
  source 1..100: mol_type = other DNA
actcttcccagctcttcaaatgcagggacagtgacaaggagctgcctgattggtgcagtcactgcttttttcagggatgtcttcaccctacatgtatcat

SEQ ID NO: 1158 - DNA, 100 bp, Homo sapiens
  source 1..100: mol_type = other DNA
catcccctacactgtgggtagaattttagcaactacattctaatggttatcgccacaactttgatcttagaaataacagtgcagtgaacatccctatgca

SEQ ID NO: 1159 - DNA, 100 bp, Homo sapiens
  source 1..100: mol_type = other DNA
ggctcctttgagttcctgtgtgaatacgaccataggattcatttctaaaagtgaaattgcgggtcagaaagatgtgtgtttgtgattttcacccaatgtt

SEQ ID NO: 1160 - DNA, 100 bp, Homo sapiens
  source 1..100: mol_type = other DNA
accagcagaagccaggccaggcccctgtgctggtcgtctatgatgatagcgaccggccctcagggatccctgagcgattctctggctccaactctgggaa

SEQ ID NO: 1161 - DNA, 100 bp, Homo sapiens
  source 1..100: mol_type = other DNA
cccagcctcggtcaccctcttgctccagccccgggaagcctgttgataaagccatgagtgaatctggcccagttcacctggatctgagcctttcaggttg

SEQ ID NO: 1162 - DNA, 100 bp, Homo sapiens
  source 1..100: mol_type = other DNA
cccttccctccagccccctccaggagtctctacagaagatacatcaggcataaatatggcctggaagggccagaatcatctggtgacttggggctgttgt

SEQ ID NO: 1163 - DNA, 100 bp, Homo sapiens
  source 1..100: mol_type = other DNA
ggtcctgggcccagtctgccctgactcagcctgcctccgtgtctgggtctcctggacagtcgatcaccatctcctgcactggaaccagcagtgacgttgg

SEQ ID NO: 1164 - DNA, 100 bp, Homo sapiens
  source 1..100: mol_type = other DNA
aaagcccccaaactcatgatttatgaggtcagtaatcggccctcaggggtttctaatcgcttctctggctccaagtctggcaacacggcctccctgacca

SEQ ID NO: 1165 - DNA, 100 bp, Homo sapiens
  source 1..100: mol_type = other DNA
aggctcagtgcccatagaccccaagttggccctgccctgaaccctgtgcaaagcccagacacagtcttagggtaggacccctgggaatgggctcttgatc

SEQ ID NO: 1166 - DNA, 100 bp, Homo sapiens
  source 1..100: mol_type = other DNA
ttcaagccccctctcctgttttccttgcagtctctgaggcctcctatgagctgacacagccaccctcggtgtcagtgtccccaggacaaacggccaggat

SEQ ID NO: 1167 - DNA, 100 bp, Homo sapiens
  source 1..100: mol_type = other DNA
agaagtcaggccaggcccctgtgctggtcatctatgaggacagcaaacgaccctccgggatccctgagagattctctggctccagctcagggacaatggc

SEQ ID NO: 1168 - DNA, 100 bp, Homo sapiens
  source 1..100: mol_type = other DNA
caccttgactatcagtggggcccaggtggaggatgaagctgactactactgttactcaacagacagcagtggtaatcatagcacagtgacactggcagat

SEQ ID NO: 1169 - DNA, 100 bp, Homo sapiens
  source 1..100: mol_type = other DNA
ggggaagtgagacacaaaccccttcttcatctattttaccctctccctccagccccaggaccgctgtggaccaacccataagcaggtctggcagaattca

SEQ ID NO: 1170 - DNA, 100 bp, Homo sapiens
  source 1..100: mol_type = other DNA
aggctcacctgggcccagcactgactcactagactgtgtttctccctttccagggtcctgggcccagtctgccctgactcagcctccctccgcgtccggg

SEQ ID NO: 1171 - DNA, 100 bp, Homo sapiens
  source 1..100: mol_type = other DNA
catctcctgcactggaaccagcagtgacgttggtggttataactatgtctcctggtaccaacagcacccaggcaaagcccccaaactcatgatttatgag

SEQ ID NO: 1172 - DNA, 100 bp, Homo sapiens
  source 1..100: mol_type = other DNA
gtcagtaagcggccctcaggggtccctgatcgcttctctggctccaagtctggcaacacggcctccctgaccgtctctgggctccaggctgaggatgagg

SEQ ID NO: 1173 - DNA, 100 bp, Homo sapiens
  source 1..100: mol_type = other DNA
aggctgaggatgaggctgattattactgcagctcatatgcaggcagcaacaatttccacagtgttttaagtcaatgaggaagtaagatcaaaacctgccc

SEQ ID NO: 1174 - DNA, 100 bp, Homo sapiens
  source 1..100: mol_type = other DNA
tcaggctcagaacccataggatcctgagctgggcctgcccaaacatgagttcatcccaggcacaacctcagggtgggaccccctgggaacagattcatca

SEQ ID NO: 1175 - DNA, 100 bp, Homo sapiens
  source 1..100: mol_type = other DNA
tttacaagcctcctctcctgtcctctcttgcaagctcctatgagcttacacagccaccctcagtgtcagtgtcaccaggacaggcagccatgatcacctg

SEQ ID NO: 1176 - DNA, 100 bp, Homo sapiens
  source 1..100: mol_type = other DNA
ctcttgagataacctcaaagatgagtatgtttactggttctggcagaagccagaccaggcccatactggtgatatatgaaggcagcaagcggccctcagg

SEQ ID NO: 1177 - DNA, 100 bp, Homo sapiens
  source 1..100: mol_type = other DNA
aatttctgattttctgagtccagctcagggaacatggccaccctgaccatcagcagggctcagactgaggacgaggctgactattactgtcacaggtaca

SEQ ID NO: 1178 - DNA, 100 bp, Homo sapiens
  source 1..100: mol_type = other DNA
atagaaacagtgatgagcccacagtgacacaggcagattaggaagtgagacacaaaccccttcccaatctgtgtcaccctctttctccagccccaggatg

SEQ ID NO: 1179 - DNA, 100 bp, Homo sapiens
  source 1..100: mol_type = other DNA
gggatgagaagggaccaggggcctgggattgagctgtgaagggaaccaaaaggcaggagggacagggcaggggctgtcagctatgactcaggggaggttc

SEQ ID NO: 1180 - DNA, 100 bp, Homo sapiens
  source 1..100: mol_type = other DNA
ctgggcctcaggatcctccctctgaggccaccagggggcgggggtggcacatgcctggacctgggaggtccctgctgggcttcaccctgggtgggtccta

SEQ ID NO: 1181 - DNA, 100 bp, Homo sapiens
  source 1..100: mol_type = other DNA
atgcctggacctgggaggtccctgctgggcttcaccctgggtgggtcctaggagctccttcctcctaagtccccctaaagagacagaggcattctggggt

SEQ ID NO: 1182 - DNA, 100 bp, Homo sapiens
  source 1..100: mol_type = other DNA
cctaaatctgtcatgcccccataaatgcatttctacgagggccaataaatgaactccaggtttatccaagcagcagcttcaggcgtctgcagacacagag

SEQ ID NO: 1183 - DNA, 100 bp, Homo sapiens
  source 1..100: mol_type = other DNA
cggggaggaattagccaacctgaggcaccctagaagggctgaagggggctgaaggggactgaagggtccctgtggggcctgtggtcctggggaggggaga

SEQ ID NO: 1184 - DNA, 100 bp, Homo sapiens
  source 1..100: mol_type = other DNA
gctggggtgtctcccagccactctgggccctgtcctgacacttctcccacaaagaagggaagggaaatcctgggaccccacagccaggaccaaccgtgaa

SEQ ID NO: 1185 - DNA, 100 bp, Homo sapiens
  source 1..100: mol_type = other DNA
ccacaggacaggaaggacagggacccccaaggctggctccatttcccaggcactgtcatgggctgagtctcaggaaatccaagtcaaggagtttcaatcc

SEQ ID NO: 1186 - DNA, 100 bp, Homo sapiens
  source 1..100: mol_type = other DNA
ccaaggaaacagaagtctacgggcccaggcccaggtgagggtggggtaagaagaggagcttaggatgcagatttgcatggaggccccgccctcctctgag

SEQ ID NO: 1187 - DNA, 100 bp, Homo sapiens
  source 1..100: mol_type = other DNA
gcatcagggtaagacaaggctgggggcaggcccagtgctggggtctcaggaggcagcgctctggggacgtctccaccatggcctgggctctgctcctcct

SEQ ID NO: 1188 - DNA, 100 bp, Homo sapiens
  source 1..100: mol_type = other DNA
ctcagggcacaggtgacgcctccagggaaggggcctcggggacccttgggctgatccttggtctcctgctcctcaggctcacctgggcccagcactgact

SEQ ID NO: 1189 - DNA, 100 bp, Homo sapiens
  source 1..100: mol_type = other DNA
ttgggagttatgactatgtctcctggtaccaacagcacccaggcacagtccccaaacccatgatctacaatgtcaatactcagccctcaggggtccctga

SEQ ID NO: 1190 - DNA, 100 bp, Homo sapiens
  source 1..100: mol_type = other DNA
tcgtttctctggctccaagtctggcaatacggcctccatgaccatctctggactccaggctgaggacgaggctgattattagtgctgctcatatacaagc

SEQ ID NO: 1191 - DNA, 100 bp, Homo sapiens
  source 1..100: mol_type = other DNA
tgaggacgaggctgattattagtgctgctcatatacaagcagtgccacttaaccacagtggtccaagttcttggggaactgagacgaaaacctgccctgg

SEQ ID NO: 1192 - DNA, 100 bp, Homo sapiens
  source 1..100: mol_type = other DNA
cctgggctctcaggctccctttttgctctgaagatgtttcctcacccagtgcaacgggcttcctgaagcacagccttgagaattcttctccctcagcaac

SEQ ID NO: 1193 - DNA, 100 bp, Homo sapiens
  source 1..100: mol_type = other DNA
tctcttttcccaccatgaaatccaaaggaaacctgctctgtggtttctcatccaggacagggacagcttccttttgcttgtgtgttgtggtccctgagtg

SEQ ID NO: 1194 - DNA, 100 bp, Homo sapiens
  source 1..100: mol_type = other DNA
ggtgcaactcttcctagctttttaaattatgggagggtgacaatgagctccctgactggtgcagtccctgctgttttcaggaacatcctcatcctaaatg

SEQ ID NO: 1195 - DNA, 100 bp, Homo sapiens
  source 1..100: mol_type = other DNA
catctgaatctcccactgtgtgcagaccaatctggacagatgttattagggggagtttccagaagccacatcttactcaactctgtatccaccacactct

SEQ ID NO: 1196 - DNA, 100 bp, Homo sapiens
  source 1..100: mol_type = other DNA
tgcctcagccatggcatggatccctctcttcctcggcgtccttgcttactgcacaggtgctgcccctagggtcctagccactggtccagtcccagggctc

SEQ ID NO: 1197 - DNA, 100 bp, Homo sapiens
  source 1..100: mol_type = other DNA
tgggtccagcctggccctgactctgagctcagcagggcccccgcctgtggtgggcaggatgctcatgaccctgctgcaggtggatgggctcggcggggct

SEQ ID NO: 1198 - DNA, 100 bp, Homo sapiens
  source 1..100: mol_type = other DNA
tgggcaggatgctcatgaccctgctgcaggtggatgggctcggcggggctgaaatccccccacacagtgctcatgtgctcacactgccttagggctcttt

SEQ ID NO: 1199 - DNA, 100 bp, Homo sapiens
  source 1..100: mol_type = other DNA
catccctggatctgtgtccaggccaggcacgtgggaagatttacttggagttcagctcctcagtttcaagccttttctctcccgttttctctcctgtagg

SEQ ID NO: 1200 - DNA, 100 bp, Homo sapiens
  source 1..100: mol_type = other DNA
atccgtggcctcctatgagctgactcagccaccctcagtgtccgtgtccccaggacagacagccagcatcacctgctctggagataaattgggggataaa

SEQ ID NO: 1201 - DNA, 100 bp, Homo sapiens
  source 1..100: mol_type = other DNA
caggacagacagccagcatcacctgctctggagataaattgggggataaatatgcttgctggtatcagcagaagccaggccagtcccctgtgctggtcat

SEQ ID NO: 1202 - DNA, 100 bp, Homo sapiens
  source 1..100: mol_type = other DNA
ctatcaagatagcaagcggccctcagggatccctgagcgattctctggctccaactctgggaacacagccactctgaccatcagcgggacccaggctatg

SEQ ID NO: 1203 - DNA, 100 bp, Homo sapiens
  source 1..100: mol_type = other DNA
gatgaggctgactattactgtcaggcgtgggacagcagcactgcacacagtgacacaggcagatgcggaagtgagacagaaaccagccacctcggcctgg

SEQ ID NO: 1204 - DNA, 100 bp, Homo sapiens
  source 1..100: mol_type = other DNA
ctcacaagacccttccctctctcctgccctgtcacactgagcaggagggagccttccatgtggaatggaagtttccagtcctatccctgcccttatgttc

SEQ ID NO: 1205 - DNA, 100 bp, Homo sapiens
  source 1..100: mol_type = other DNA
ctgagagacgggagcaagttcctgcccacctctaggctcagcttatcccagaataaactgagctagtcattttgatgatcaaatgccagctcccaaaaga

SEQ ID NO: 1206 - DNA, 100 bp, Homo sapiens
  source 1..100: mol_type = other DNA
ccccagaaaccctgatatctaagtagcaccgactctattagtatcaagggagactagccctagggtggaatcattttagtgtctcagaaggcacagggca

SEQ ID NO: 1207 - DNA, 100 bp, Homo sapiens
  source 1..100: mol_type = other DNA
atggaaagtgtttatgaggtttcaggatatgcacgtgagcagttaaaggcaggtcttacaaggaaggaacctactagaattggggcccatctgtgacatc

SEQ ID NO: 1208 - DNA, 100 bp, Homo sapiens
  source 1..100: mol_type = other DNA
acatccctctgctttgggagagaagggccagggcgggacccagagagctctgcagaggcaccacagaccctcagcagggggtctgccaaacaggacagct

SEQ ID NO: 1209 - DNA, 100 bp, Homo sapiens
  source 1..100: mol_type = other DNA
ggacttggctgcttctgcccaggcctggatccagcccttgcacatctcagggcaggggataggcctgggtggccagagctgcagctgcacctgctgggga

SEQ ID NO: 1210 - DNA, 100 bp, Homo sapiens
  source 1..100: mol_type = other DNA
ggcctagtccagtcctccagggtccccagacagactcggatttccgactgcagccaccatggaaggatgtggtctgcggtgacgatgtctatccagaggc

SEQ ID NO: 1211 - DNA, 100 bp, Homo sapiens
  source 1..100: mol_type = other DNA
ccgaatatccaaggagcccaagatcagaggcaggaataggccaagctccccagtggagaagctgtgctggaccaggggtttcccagggccctcccttgtg

SEQ ID NO: 1212 - DNA, 100 bp, Homo sapiens
  source 1..100: mol_type = other DNA
ccctgaatgatgtctgttagggcacctacaccctgttactgctcagtgccttgcctattttgaaggacagggatgtgtggtgattatttgtataatccag

SEQ ID NO: 1213 - DNA, 100 bp, Homo sapiens
  source 1..100: mol_type = other DNA
cccccagcacctggtcctcaaaagttacccaagcaatgtgtataaagatccagcctggagatctttgaaaaccgattcgatgagtcgaaccattaagtca

SEQ ID NO: 1214 - DNA, 100 bp, Homo sapiens
  source 1..100: mol_type = other DNA
tgatcaccatcctcaacttcatctctttcttcctcctcctcctcattatcatcaccttcaagaactgttaagagtctgagacttcatcctatttgcagac

SEQ ID NO: 1215 - DNA, 100 bp, Homo sapiens
  source 1..100: mol_type = other DNA
tcctcctcctcctcattatcatcaccttcaagaactgttaagagtctgagacttcatcctatttgcagactaaaaagtaagcctgccacagtgccatgga

SEQ ID NO: 1216 - DNA, 100 bp, Homo sapiens
  source 1..100: mol_type = other DNA
tgctggcagaagatacaagactcctgggtcagagacaacgaataatctgtttttcacagcaatagcagttgccaaggtatcagcattgtcttgcaccagt

SEQ ID NO: 1217 - DNA, 100 bp, Homo sapiens
  source 1..100: mol_type = other DNA
tccacaaggtgatgcaaagagggccaggtgacatctgcatgccagagctcagggatcccaaatatttcatacttgacagtaagcatatatctgtgttttg

SEQ ID NO: 1218 - DNA, 100 bp, Homo sapiens
  source 1..100: mol_type = other DNA
ctccaaagagaggcattctctgtaccttccgaggttgttcactccacaaacactcttgaaaagataatccacaatcagtgcctttgcccgagagacatgc

SEQ ID NO: 1219 - DNA, 100 bp, Homo sapiens
  source 1..100: mol_type = other DNA
agaaatgcagagatccatagtagaccactgtctcccaacaaccatcaactttatcaatgaaatgaagtctcaggctatttgtctgttaccatagcccaca

SEQ ID NO: 1220 - DNA, 100 bp, Homo sapiens
  source 1..100: mol_type = other DNA
aaaatgtctggcttgattgtcaccaaatgtatcaaggaagttaaggagtatctgacacaaaatgtgaaccaagcaattctcaaaggagcctcccaggaaa

SEQ ID NO: 1221 - DNA, 100 bp, Homo sapiens
  source 1..100: mol_type = other DNA
ttcactttaggaagtcctaggaggctcctctgagagttgctaaaacaaaacattgagagtcctagagggctgcagatctgaacttgagcagatattttta

SEQ ID NO: 1222 - DNA, 100 bp, Homo sapiens
  source 1..100: mol_type = other DNA
aagattttgtggcagaaaaagaaactggaaagcaagagggcagaccctcattgcagttctgtaatgtaagggggcagagcaggggcctttctcaccagag

SEQ ID NO: 1223 - DNA, 100 bp, Homo sapiens
  source 1..100: mol_type = other DNA
gatattggaccctgcattcatcttctctggatggtaattttctcacctgtaaaacagagacactggccccaaggacaccccacaagtagttgtgaatccc

SEQ ID NO: 1224 - DNA, 100 bp, Homo sapiens
  source 1..100: mol_type = other DNA
aaagtaagagaagaacaaaaaaagaaccagaatttattcaacacccactgagtgcttagcaaacacatggtttctttaactctcataagcttcatgctgc

SEQ ID NO: 1225 - DNA, 100 bp, Homo sapiens
  source 1..100: mol_type = other DNA
agaggaactctccccattttacagataaggaaactgaggcccagaggtaacctaggtctagatagactccacatttatgacttcaccactcttccttgcc

SEQ ID NO: 1226 - DNA, 100 bp, Homo sapiens
  source 1..100: mol_type = other DNA
aaactgaggcccagaggtaacctaggtctagatagactccacatttatgacttcaccactcttccttgcctgaaggatatagaatcactccctgcagggc

SEQ ID NO: 1227 - DNA, 100 bp, Homo sapiens
  source 1..100: mol_type = other DNA
tcttgcctgactcaggaaagggccacaggatagccagccaggcttaaccaacccagccaagaaagggctggtcccaactggctggagtgcagtgtacagg

SEQ ID NO: 1228 - DNA, 100 bp, Homo sapiens
  source 1..100: mol_type = other DNA
gttggtagatgcccctctgggagagatccccaggggtgacagccatggaccctggaagggcctgggctagggacagggaccagagccagtccagggagag

SEQ ID NO: 1229 - DNA, 100 bp, Homo sapiens
  source 1..100: mol_type = other DNA
gacagagccaatggactggggtgtactgtaacagccctgctggcgagagggaccagggcaccgtcctccagggagcccatgctgcaagtcgggccagagg

SEQ ID NO: 1230 - DNA, 100 bp, Homo sapiens
  source 1..100: mol_type = other DNA
tgcccctgaacctgaaggccaatgagacccaagacaggccaagtgggttgtgagacccctgaggagctgggccctggtcccaggcagcgctggcccctgc

SEQ ID NO: 1231 - DNA, 100 bp, Homo sapiens
  source 1..100: mol_type = other DNA
tgctgctgggtctggccatggtcgcccatggcctgctgcgcccaatggttgcaccgcaaagcggggacccagaccctggagcctcagttggaagcagccg

SEQ ID NO: 1232 - DNA, 100 bp, Homo sapiens
  source 1..100: mol_type = other DNA
atccagcctgcggagcctgtggggcaggtaaggggcaagagattccaggggatgtgggggtcctgcagcagagctgggaaagggtgaccaaggggagaca

SEQ ID NO: 1233 - DNA, 100 bp, Homo sapiens
  source 1..100: mol_type = other DNA
agccagaggagtgaggaggaaggttaacccctaagaggggcctgggctgacactggctttagtaatgggttgatattttgtccatcacagatttgtttga

SEQ ID NO: 1234 - DNA, 100 bp, Homo sapiens
  source 1..100: mol_type = other DNA
attactgtttttaatatcatattacgatattatttttcttgatttctgagttttctggcgccacttaaattttcaccagggtcagtgcctcaatcaccta

SEQ ID NO: 1235 - DNA, 100 bp, Homo sapiens
  source 1..100: mol_type = other DNA
gtcctagtcctctgggtagggaaggaacagaggcagggacaggacatccacagggggtggtggccactgtccccacagggtgcccaggcctgttcctccc

SEQ ID NO: 1236 - DNA, 100 bp, Homo sapiens
  source 1..100: mol_type = other DNA
cctcctcctctctgcccatgtgcctcctgcccagtgagggcaggggccactccctggagaaggcagcaagggcttggtttggtctcccccaaggctgtct

SEQ ID NO: 1237 - DNA, 100 bp, Homo sapiens
  source 1..100: mol_type = other DNA
gttcaccaacttgcacataaatgcttactggggccaggctcaaggacacagggagggtgggatgaaccgaggggagctgtccagtcattggaacaggccc

SEQ ID NO: 1238 - DNA, 100 bp, Homo sapiens
  source 1..100: mol_type = other DNA
acggcccatgtttggagcaataaagggagaggggatctccctctgggatgatgcccaggctggtctcacagatcgaggggcactggctggtgatgggtgc

SEQ ID NO: 1239 - DNA, 100 bp, Homo sapiens
  source 1..100: mol_type = other DNA
tggtctcacagatcgaggggcactggctggtgatgggtgcccccaaaagacagagcagcgtcagaggagaggagagcacaggatgaggctgggagctcct

SEQ ID NO: 1240 - DNA, 100 bp, Homo sapiens
  source 1..100: mol_type = other DNA
gggtgactgggaaggggaggcaagaagaccatagggtccgtgcaccattcccagtccaggacgagtccttggatggatttaggtagattgattatcagag

SEQ ID NO: 1241 - DNA, 100 bp, Homo sapiens
  source 1..100: mol_type = other DNA
tcagatttgtgtttttggaaaaatcagcaccggattggaggctgatgcgacgcccgattagaggagggaggagagggggtgatggccaagtccagggtag

SEQ ID NO: 1242 - DNA, 100 bp, Homo sapiens
  source 1..100: mol_type = other DNA
gtggggatcctggaggaagccgtgccttggggatggggaggacactcagattcagagcacccaggggcccagtttcctatgaaatgggagcatgaagttg

SEQ ID NO: 1243 - DNA, 100 bp, Homo sapiens
  source 1..100: mol_type = other DNA
aagtgagggctgagcagaggggagcagacacgctcggggactgtctatgggcattaaaaatgtataaccattttagcaacaggcggcgagtcaaaaaaca

SEQ ID NO: 1244 - DNA, 100 bp, Homo sapiens
  source 1..100: mol_type = other DNA
aagtgtgtttatctaaactgggcaattccacttctaggaatttatcctaagggttggttgggggaataatcaaagctgtaaccaaatctttataacaagg

SEQ ID NO: 1245 - DNA, 100 bp, Homo sapiens
  source 1..100: mol_type = other DNA
gtggttagctcagcattattagtgatgggagaaaactggaaaaaatccaaatatctaccagaaagggtgtgaaaaaacacaattgtatttgggggactgt

SEQ ID NO: 1246 - DNA, 100 bp, Homo sapiens
  source 1..100: mol_type = other DNA
tggctaattttgattaggattattattagtttagagacagagcctcgctatattgctcaggcctgtctcaaattcctaagctcaagcaatctttctgcct

SEQ ID NO: 1247 - DNA, 100 bp, Homo sapiens
  source 1..100: mol_type = other DNA
actgcacctgacccaactgtgtttttaaagtatatatgcattttcaaaaacctgtcagaaaatatagaaaaatgtcaatggtgtgtctggctggctgatg

SEQ ID NO: 1248 - DNA, 100 bp, Homo sapiens
  source 1..100: mol_type = other DNA
ggatttcacctaattttaatgtggctttataattttctggttttgtgaagttgttcacaaaaagagacatttcttctaatataatttttaatacaacagt

SEQ ID NO: 1249 - DNA, 100 bp, Homo sapiens
  source 1..100: mol_type = other DNA
aatgtactcatgtgcattactctttttgtaatgagtatattacaaaatgtaatgacttttgtacattactcttttttcttgccaaaaaaaaaaaagatta

SEQ ID NO: 1250 - DNA, 100 bp, Homo sapiens
  source 1..100: mol_type = other DNA
agcagagaagtatataaagtaaaagcaagtgcttctgcttaccatctctcacctcttcccagagatagccactgtcaggttggtcaatatacttccagaa

SEQ ID NO: 1251 - DNA, 100 bp, Homo sapiens
  source 1..100: mol_type = other DNA
cttttcctgtgtgtgtgtgtgtccctgaaaacacacacacacacacacacacacacacacacagttggtgctgggattttattttgcaaaagtaagagcc

SEQ ID NO: 1252 - DNA, 100 bp, Homo sapiens
  source 1..100: mol_type = other DNA
cacacacagttggtgctgggattttattttgcaaaagtaagagccatattctgcatattaccaacttttaatctattattgacactttctgtatcagtcc

SEQ ID NO: 1253 - DNA, 100 bp, Homo sapiens
  source 1..100: mol_type = other DNA
atatggattaaccacattcattgcttataaactttgttttataagcaaagtttagatgagccagaatttatttccactaaaaaatctaaatgacaaatga

SEQ ID NO: 1254 - DNA, 100 bp, Homo sapiens
  source 1..100: mol_type = other DNA
tgctgcagtggaaatttgtgtgtgtgtgtgtgtgtgtgtgtgtgtgtgtgtgtgtgtgtgtgtatgtgtacaaagtgcacttatatatctccccaggata

SEQ ID NO: 1255 - DNA, 100 bp, Homo sapiens
  source 1..100: mol_type = other DNA
tgacctgggtgtttttctttttctctgtaggatgttaatagtatcttgtgtcatgctaggatgtctaggacagagggcaatacaatgaggggaaggcatt

SEQ ID NO: 1256 - DNA, 100 bp, Homo sapiens
  source 1..100: mol_type = other DNA
ctgcgatgtccccaggcctctggcttgaagagtaacttgctgaagtgaggactctgtggaggagcaagttatacagaaagaagtttagttgtgatctgtt

SEQ ID NO: 1257 - DNA, 100 bp, Homo sapiens
  source 1..100: mol_type = other DNA
gagttggaggtgtctacagggcatccaagcagacataggttgaggaggcagaatatatgtgaatctggagccaagaagagaggtaagggctggaaatagg

SEQ ID NO: 1258 - DNA, 100 bp, Homo sapiens
  source 1..100: mol_type = other DNA
gatctaagacccctggacagttgtgagtgtgcacaatgagggtcagatgcagagaaaattaggagactacagagagcagaacccagggtggggatctggg

SEQ ID NO: 1259 - DNA, 100 bp, Homo sapiens
  source 1..100: mol_type = other DNA
agtcagcagttgggcatgggcctggtagaaagggaagccaaggaggaggagagggggcagtctcagacaccaaggaggggagagtgactagaaagaaaac

SEQ ID NO: 1260 - DNA, 100 bp, Homo sapiens
  source 1..100: mol_type = other DNA
cttcttgcagagacataggggatggggaagaactgcagactgaactggggcaaaggactgttggccttaaccagagagatttgagggagagatgaggctg

SEQ ID NO: 1261 - DNA, 100 bp, Homo sapiens
  source 1..100: mol_type = other DNA
agagccaggggatcctgccatgtcccagcataaaaacagtacctgacacagatgggtgcttgggagctgttgtcggatgaatgagtggacagatgcatgg

SEQ ID NO: 1262 - DNA, 100 bp, Homo sapiens
  source 1..100: mol_type = other DNA
atggacggatggatggaaggatgatagattgatggacaaacagatgaacagatgaatagctggatggacaactggatggatgggtagacagaatgatctc

SEQ ID NO: 1263 - DNA, 100 bp, Homo sapiens
  source 1..100: mol_type = other DNA
agagatcagaaaaagcttcatgcactaagtgggactgaaccgcgtctccatgggtagaaagcagaggaatctccacttgagtcaggaatgacccagtgct

SEQ ID NO: 1264 - DNA, 100 bp, Homo sapiens
  source 1..100: mol_type = other DNA
ctcaatccagggagaaagccagcctggcttcactggggacacttgtgtgggggactcagaggccctttaaatgaggccagacgaggttggacaggtccaa

SEQ ID NO: 1265 - DNA, 100 bp, Homo sapiens
  source 1..100: mol_type = other DNA
gccaactcagcactcctctgccacactgcacaggaggggatgtgtcactcagggagttgctgggacctatgggtcccagtgttgtcatcagcaccgacag

SEQ ID NO: 1266 - DNA, 100 bp, Homo sapiens
  source 1..100: mol_type = other DNA
cctcagagaggaaagacacacactggggtaactccaaggctgtgtgtggcacttgccttggacagcagacaggcacagggacacctctagggggctggcc

SEQ ID NO: 1267 - DNA, 100 bp, Homo sapiens
  source 1..100: mol_type = other DNA
acccccctgcctcatgtctaggtcccagccccgcccactgcaaccctgtgcccgtcatgcccagcaggctcctgctccagcccagcccccagagagcaga

SEQ ID NO: 1268 - DNA, 100 bp, Homo sapiens
  source 1..100: mol_type = other DNA
cactgcaaccctgtgcccgtcatgcccagcaggctcctgctccagcccagcccccagagagcagaccccaggtgctggccccgggggttttggtctgagc

SEQ ID NO: 1269 - DNA, 100 bp, Homo sapiens
  source 1..100: mol_type = other DNA
ctcagtcactgtgttatgtcttcggaactgggaccaaggtcaccgtcctaggtaagtggctctcaacctttcccagcctgtctcaccctctgctgtccct

SEQ ID NO: 1270 - DNA, 100 bp, Homo sapiens
  source 1..100: mol_type = other DNA
ggaaaatctgttttctctctctggggcttcctcccctctgtcctcccagccttaagcactgacccttacctttctccatggggcctggaggaggtgcatt

SEQ ID NO: 1271 - DNA, 100 bp, Homo sapiens
  source 1..100: mol_type = other DNA
agtctccgggtaaccggcaggaagggcctccacagtgggagcagccggatgcagcctggtcccggggcctgagctgggattgggcagggtcagggctcct

SEQ ID NO: 1272 - DNA, 100 bp, Homo sapiens
  source 1..100: mol_type = other DNA
cctctcttccagggcagatgtctgagtgagggacagaggctggttctgatgaggggccctgcagtgtccttagggacattgcccagtgactcctggggtc

SEQ ID NO: 1273 - DNA, 100 bp, Homo sapiens
  source 1..100: mol_type = other DNA
ggacagaggctggttctgatgaggggccctgcagtgtccttagggacattgcccagtgactcctggggtcaaggacagaggctgctggggtgggcctggg

SEQ ID NO: 1274 - DNA, 100 bp, Homo sapiens
  source 1..100: mol_type = other DNA
agctgctgagtctcatagtctaggggagcagccccaagaacagctgagggtctaggctgaggactggatgccaatccagcctgggagggccacacggcct

SEQ ID NO: 1275 - DNA, 100 bp, Homo sapiens
  source 1..100: mol_type = other DNA
tctcatagtctaggggagcagccccaagaacagctgagggtctaggctgaggactggatgccaatccagcctgggagggccacacggcctggtgacacag

SEQ ID NO: 1276 - DNA, 100 bp, Homo sapiens
  source 1..100: mol_type = other DNA
aggtcaccccaaggggagaccaatggagggcacagagagggctctgggtctaggctgcagctctgtggcctgtgctgggtcatgaggacatggggacaca

SEQ ID NO: 1277 - DNA, 100 bp, Homo sapiens
  source 1..100: mol_type = other DNA
tgtgctgggtcatgaggacatggggacacagagggacgggtgagactgggtgaggtgccagaatccaaccctcccaggacagtcaccagaaaggagacag

SEQ ID NO: 1278 - DNA, 100 bp, Homo sapiens
  source 1..100: mol_type = other DNA
tctcttagggcagagatgtgtctgtccctggagccccgtcacctctggggcccagtgtctctctgttcacggatcggcctcctgccttcctcaaagggca

SEQ ID NO: 1279 - DNA, 100 bp, Homo sapiens
  source 1..100: mol_type = other DNA
tgttagactcaggaaatgaccagaggggagtgaatgaggggtgcagagaactccatggctaccaggtgaagtttggggtcatcacaggctgctggggtgg

SEQ ID NO: 1280 - DNA, 100 bp, Homo sapiens
  source 1..100: mol_type = other DNA
catagtctgtgggagcagccccaggaacagctgaggtgaagggttctgtggtcgggcttgtggagacaggaaacatctcagagcctcagaggagccctga

SEQ ID NO: 1281 - DNA, 100 bp, Homo sapiens
  source 1..100: mol_type = other DNA
ggcttgtctaggtggagcccactccttgccaggagagccaagtgggctgggctggggcagagcccggtgcctgtgagggataggaagctccagttcaaag

SEQ ID NO: 1282 - DNA, 100 bp, Homo sapiens
  source 1..100: mol_type = other DNA
caggcttgggtctccccacacactgcctgccaggacagtcctacaggatgagcaggggacccacagttcacggaggaggctctaggtcctggaagaataa

SEQ ID NO: 1283 - DNA, 100 bp, Homo sapiens
  source 1..100: mol_type = other DNA
agtgggtgatggaggggggtatagggatggaaatgagggatccaggggtcaaggccagattctaaactcagactccagagatcagagaagaaggaacaca

SEQ ID NO: 1284 - DNA, 100 bp, Homo sapiens
  source 1..100: mol_type = other DNA
gcctgccctgggtatatggagaaattgaggctgtagaggagaggggctgggccaggacacctgtgaaaggtgacttgggagggctcctaggaaggcacag

SEQ ID NO: 1285 - DNA, 100 bp, Homo sapiens
  source 1..100: mol_type = other DNA
tgaaagccccactgctatgaccaggtagccgggacgtggggtggatgccagaaaagactccacggaataagagagagcccaggacagcaggcaggctctc

SEQ ID NO: 1286 - DNA, 100 bp, Homo sapiens
  source 1..100: mol_type = other DNA
cgatccccccaggcccttgccccatacacgggctccagaacacacatttggctggaacagcctgagggaccaaaaggccccagtatcccacagagctgag

SEQ ID NO: 1287 - DNA, 100 bp, Homo sapiens
  source 1..100: mol_type = other DNA
gagccaggccagaaaagtaaccccagagttcgctgtgcaggggagacacagagctctctttatctgtcaggatggcaggaggggacagggtcagggcgct

SEQ ID NO: 1288 - DNA, 100 bp, Homo sapiens
  source 1..100: mol_type = other DNA
gagggtcagatgtcggtgttgggggccaaggccccgagagatctcaggacaggtggtcaggtgtctaaggtaaaacagctccccgtgcagatcagggcat

SEQ ID NO: 1289 - DNA, 100 bp, Homo sapiens
  source 1..100: mol_type = other DNA
atgcaggacagtccggagagggaaatcaggagaagtgaaggggtctctggggagcccagatgtgggctagaggcagaagtaagggtgaagagcacctatg

SEQ ID NO: 1290 - DNA, 100 bp, Homo sapiens
  source 1..100: mol_type = other DNA
agtcaatgtcatggtctcagcaggaacacagttgaaaatccccattccacacaagaccgtttagcaggaaaggagtccatacttgtgctgccaccaggat

SEQ ID NO: 1291 - DNA, 100 bp, Homo sapiens
  source 1..100: mol_type = other DNA
gtcctgagaagccttggagaatgaaacatacaggtgcatttcctagacttgacaatgcacgttagccaagtaaaggcaatgaaaagttctctactaggga

SEQ ID NO: 1292 - DNA, 100 bp, Homo sapiens
  source 1..100: mol_type = other DNA
tttgtttgtttctgtatcttgtctcaacttgtggtcagcctttctccctgcatcccaggcctgagcaaggacctctgccctccctgttcagacccttgct

SEQ ID NO: 1293 - DNA, 100 bp, Homo sapiens
  source 1..100: mol_type = other DNA
tgcctcagcaggtcactacaaccacttcacctctgaccgcaggggcaggggactagatagaatgacctactgagcctcgtctgtctgtctgtctgtctgt

SEQ ID NO: 1294 - DNA, 100 bp, Homo sapiens
  source 1..100: mol_type = other DNA
ctgtttgtctctctgtctgtctgacaggcgcaggctgggtctctaagccttgttctgttctggcctcctcagtctgggttcttgtcggaacagctttgcc

SEQ ID NO: 1295 - DNA, 100 bp, Homo sapiens
  source 1..100: mol_type = other DNA
cttgggttacctgggttccatctcctggggaattgggaacaaggggtctgagggaggcacctcctgggagactttagaaggacccagtgccctcggggct

SEQ ID NO: 1296 - DNA, 100 bp, Homo sapiens
  source 1..100: mol_type = other DNA
agagttcgctgtgcaggggagacacagagctctctttatctgtcaggatggcaggaggggacagggtcagggcgctgagggtcagatgtcggtgttgggg

SEQ ID NO: 1297 - DNA, 100 bp, Homo sapiens
  source 1..100: mol_type = other DNA
gccaaggccccgagagatctcaggacaggtggtcaggtgtctaaggtaaaacagctccccgtgcagatcaggacatagtggaaaacaccctgacccctct

SEQ ID NO: 1298 - DNA, 100 bp, Homo sapiens
  source 1..100: mol_type = other DNA
gcctggcatagaccttcagacacagagcccctgaacaagggcaccccaacacctcatcatatactgaggtcaggggctccccaggtggacaccaggactc

SEQ ID NO: 1299 - DNA, 100 bp, Homo sapiens
  source 1..100: mol_type = other DNA
agaatattccgtgagaaggtggccccacagcgctgggtcacacgccatcccccaagacaggcaggacaccacagacagggtggtgggtctcagaaaactc

SEQ ID NO: 1300 - DNA, 100 bp, Homo sapiens
  source 1..100: mol_type = other DNA
aggccctaaacgtggatgcttaccaattcctccactggaggaagacctcagagcagatgcccaggacagggacttctggtagggacggtgactgggacgg

SEQ ID NO: 1301 - DNA, 100 bp, Homo sapiens
  source 1..100: mol_type = other DNA
gtgcctgtttgtcagggaaaacccactggagagtcagatcccccagataacttctcacgacatggagactctttcgaacagacaaagctccacgttcagc

SEQ ID NO: 1302 - DNA, 100 bp, Homo sapiens
  source 1..100: mol_type = other DNA
tcagggagtaaaaaaaaaatgcctcaaatggaggcctttgatctactggaatccagcccccaggactgacaccctgtctcaccaggcagcccagaggggt

SEQ ID NO: 1303 - DNA, 100 bp, Homo sapiens
  source 1..100: mol_type = other DNA
cagggtccaccagaaggcatctcagaaccagccagcagtggccctgattgtcagcaggaccccagggaggggggtggccaggacagggctctgaagcccc

SEQ ID NO: 1304 - DNA, 100 bp, Homo sapiens
  source 1..100: mol_type = other DNA
caccccaggaccttccctgggcagaacgagttggtgagggagtgatgagcaaccacaggcctcctaacttcccaagctggcgattctgagaggcctcaag

SEQ ID NO: 1305 - DNA, 100 bp, Homo sapiens
  source 1..100: mol_type = other DNA
gctgagacacggttcagccttttaggccctcctgaacgtgtcccctgtctccacagcctgggaatgcactctcttttgacccagaaatcctgctcataag

SEQ ID NO: 1306 - DNA, 100 bp, Homo sapiens
  source 1..100: mol_type = other DNA
ctgtcattgtacaacacatcatttcactttgtttttcaaacatagtgaattctttcctaattaaagaagaaaagagtataaagagaaagtttccagtgca

SEQ ID NO: 1307 - DNA, 100 bp, Homo sapiens
  source 1..100: mol_type = other DNA
gtataaagagaaagtttccagtgcagcctggagatctgtactggttgtatctggaattccagactcagccttgcatttcacatagcagatagatgatgat

SEQ ID NO: 1308 - DNA, 100 bp, Homo sapiens
  source 1..100: mol_type = other DNA
gatggagaaggagaagaagaaggaggaggaggaggaaagaaggaagaagaagaagaagaggaggaggaagaagaagacgaagggaagaagaagaaggatg

SEQ ID NO: 1309 - DNA, 100 bp, Homo sapiens
  source 1..100: mol_type = other DNA
tccaggtctgccaggtgtaggggaggtgtgactggttccatcatggaccggttcctccatggaccggttcctccgtggaccggttccgccatggaccggt

SEQ ID NO: 1310 - DNA, 100 bp, Homo sapiens
  source 1..100: mol_type = other DNA
tccgccatggaccactcctgccctggaccactcctgccctggaccggttctgccgtggactggttcccgccgtggaccagttcccgctgtatactggttc

SEQ ID NO: 1311 - DNA, 100 bp, Homo sapiens
  source 1..100: mol_type = other DNA
tgccctggactggttcccgctgtggactggttccttggggctctaagtgcggaagggcccagagctggtccctgcccagcgccctgctagggctgtgtcc

SEQ ID NO: 1312 - DNA, 100 bp, Homo sapiens
  source 1..100: mol_type = other DNA
tcgtactcgtgcgcctcgcttcggtgagccccagggcccctgcctccttcctcctgccgtcctgcctccgtccccgccctttcatcatccgcgtccctgt

SEQ ID NO: 1313 - DNA, 100 bp, Homo sapiens
  source 1..100: mol_type = other DNA
gaaggcattccctaaatccgagcccgagtggttctccccgggaaggctactttggggagctggggggatgcgaaacaccctagatactggataatggggt

SEQ ID NO: 1314 - DNA, 100 bp, Homo sapiens
  source 1..100: mol_type = other DNA
ggggaaatcgatgatttaagaacaaaaccgaaaaactggcgttttgccgtgccgctcggaggggacattaaaaaatttcttagtgtttgcccgcaaaggt

SEQ ID NO: 1315 - DNA, 100 bp, Homo sapiens
  source 1..100: mol_type = other DNA
tagtgtttgcccgcaaaggtattgtgcgttgccttggaggctgagatatgggggaatagacaagtcctttgttctgaggttcatcttccgagccccgagc

SEQ ID NO: 1316 - DNA, 100 bp, Homo sapiens
  source 1..100: mol_type = other DNA
ctcctcccagcctcggacggctgcgcgggctgcatctgtgcagcctggcggcggcggggctgtgctatgacatctttacagtccttcttgcagagacatg

SEQ ID NO: 1317 - DNA, 100 bp, Homo sapiens
  source 1..100: mol_type = other DNA
tgtgccagggatgccgaattgccgggagagcaggcaagaccggcttcggggcgcgcggcggccgctttgtgtgcggggctgcattgtgacgcgggcgatg

SEQ ID NO: 1318 - DNA, 100 bp, Homo sapiens
  source 1..100: mol_type = other DNA
aagccggtagggcggtggtcggaagctccagccgcggccgccgcctttgtgagaggactagaaagccggatccggcccgcatccttgcggagaggccgcg

SEQ ID NO: 1319 - DNA, 100 bp, Homo sapiens
  source 1..100: mol_type = other DNA
gctaggaaatggaaacgcttttcctacctgggctccattttaggaattcttgccgatttttcccacttgaatttggaagtggctttcctcttctttcctt

SEQ ID NO: 1320 - DNA, 100 bp, Homo sapiens
  source 1..100: mol_type = other DNA
gtcctagccagcctttaattttaaacgctgtaattaacaattcgcagtggtcaatttcctttattctgcaagattcggctttgagaggcatccgccctct

SEQ ID NO: 1321 - DNA, 100 bp, Homo sapiens
  source 1..100: mol_type = other DNA
ttggtccacagcgttttgaaatatggggaggaggggcgcggggggtgtcgcctctttttctgtagaaagaggaagctcgtgagcgcggaacggcagcagt

SEQ ID NO: 1322 - DNA, 100 bp, Homo sapiens
  source 1..100: mol_type = other DNA
aagtgcagttcccagcccagagacagcggggcgggtggctcttcctcacgctcgctcttggcttgctccctgcagcttttcctccgcaaccatgtctgac

SEQ ID NO: 1323 - DNA, 100 bp, Homo sapiens
  source 1..100: mol_type = other DNA
aaacccgatatggctgagatcgagaaattcgataagtcgaaactgaagaagacagagacgcaagagaaaaatccactgccttccaaagaaagtgagctcc

SEQ ID NO: 1324 - DNA, 100 bp, Homo sapiens
  source 1..100: mol_type = other DNA
agacgcaagagaaaaatccactgccttccaaagaaagtgagctccgacccacccccatctttagaaaggctgggtgggagcggccggtgggagggcggga

SEQ ID NO: 1325 - DNA, 100 bp, Homo sapiens
  source 1..100: mol_type = other DNA
tttatagaaaggcatatggaacaggagtcatccaaatatatcccaggggttgcaaattgaccaaaagagtcacctttagggaagcctgcttctgaatgct

SEQ ID NO: 1326 - DNA, 100 bp, Homo sapiens
  source 1..100: mol_type = other DNA
tgtggaatttatcattcttctgaatggctgttgcatttatctgcagcttttactcaccagatgagacctcagacatttcaaattctgcggaggctggcta

SEQ ID NO: 1327 - DNA, 100 bp, Homo sapiens
  source 1..100: mol_type = other DNA
cacaccttcataggaaagctttttgctgatttccctgttggtacttttctcttacacattctatggggtatggtaaacctggaggtagagtcatagccaa

SEQ ID NO: 1328 - DNA, 100 bp, Homo sapiens
  source 1..100: mol_type = other DNA
gcacagataaagcaggcacagaatctctgaccagcctcacaaaagcagacaaacacacaatctttttgcacctgtttcttccactccggttgccgtgaat

SEQ ID NO: 1329 - DNA, 100 bp, Homo sapiens
  source 1..100: mol_type = other DNA
tagaaatggttcaaccagtccaatatcaatatagctgcttattactctattcacttacttcaaagtggcatttgttttgagtaagactttatttaattct

SEQ ID NO: 1330 - DNA, 100 bp, Homo sapiens
  source 1..100: mol_type = other DNA
taccgttagcttgaaaccatagagatcttctctctatttgccctacttccttcaaaagtcaaatgacctcctacaaataaaagacgttcttattttcatt

SEQ ID NO: 1331 - DNA, 150 bp, Homo sapiens
  source 1..150: mol_type = other DNA
cgactacgactcggtgcagccgtatttctactgcgacgaggaggagaacttctaccagcagcagcagcagagcgagctgcagcccccggcgcccagcgaggatatctggaagaaattcgagctgctgcccaccccgcccctgtcccctag

SEQ ID NO: 1332 - DNA, 150 bp, Homo sapiens
  source 1..150: mol_type = other DNA
cgactacgactcggtgcagccgtagttctactgcgacgaggaggaaaacttctaccagcagcagcagcagagcgagctgcagcccctggcgcccagcgaggatatctggaagaacttcgagctgctgcccaccccgcccctgtcccctag

SEQ ID NO: 1333 - DNA, 150 bp, Homo sapiens
  source 1..150: mol_type = other DNA
cgactacgactcggtgcagccgtagttctactgcgacgaggaggaatacttctaccagcagcagccgcagagcgagctgcagcccctggcgcccagcgagggtatctggaagaacttcgagctactgcccaccccgcccctgtcccctag

SEQ ID NO: 1334 - DNA, 150 bp, Homo sapiens
  source 1..150: mol_type = other DNA
cgactacgactcgttgcagccgtagttctactgcgacgaggaggaatacttctaccagcagcagccgcagagcgagctgcagcgcctggcgcccagcgagggtatctggaagaacttcgagctacagcccaccccgcccctgtcccctag

SEQ ID NO: 1335 - DNA, 150 bp, Homo sapiens
  source 1..150: mol_type = other DNA
cgactacgactcgttgcagccgtagatctactgcgacgaggaggaatacttctacctgcagcagccgcagagcgagctgcagcgcctggcgcccagcgagcgtatctggaagaacttcgagctacagcccaccccgcccttgtcccctag

SEQ ID NO: 1336 - DNA, 150 bp, Homo sapiens
  source 1..150: mol_type = other DNA
cgacaacgactcgttgcacccgtagatctactgcgacgaggaggaatacttctacctgcagcagccgcagagcgagctgcagcgcctggcgcccagcgagcgtatctgaaagaacttcgagctacagcccacgccgcccttgtcccctag

SEQ ID NO: 1337 - DNA, 150 bp, Homo sapiens; identical to SEQ ID NO: 1336
  source 1..150: mol_type = other DNA

SEQ ID NO: 1338 - DNA, 150 bp, Homo sapiens
  source 1..150: mol_type = other DNA
gctcacctgtacaaatctggctccgcaggtttcgcatttgtagggcttctctccagagtgaattcgagtgtgggttttcaggttggctggccggttgaactgggccccacagatgttgcaacgatagggtttctcacctattaccaagaa

SEQ ID NO: 1339 - DNA, 150 bp, Homo sapiens
  source 1..150: mol_type = other DNA
gctcacctgtacaaatctgcctccgcaggtttcgcatttgtagggctcctctccagagtgaattcgagtgtgggttttcaggttggctgggcggttgaactgggccccacagatgttgcaacgctagggtttctcacctattaccaagaa

SEQ ID NO: 1340 - DNA, 150 bp, Homo sapiens
  source 1..150: mol_type = other DNA
gctcacctgtacaaatctgcctccgcaggtttcgcctttgtagggctcctctccagagtgaattcgagtgtaggttttcaagttggctgggcggttgaactgggccccacggatgttgcaacgctagggtttctcacctattaccaagaa

SEQ ID NO: 1341 - DNA, 150 bp, Homo sapiens
  source 1..150: mol_type = other DNA
gctcacctgtacaaatctgcctccgccggtttcgcctttttagggctcctctccagagtgaattcgagtgtaggttttcaagttggctgggcggttgaactgggccccacggatgttgcaacgctagggtttctcacctatttccaagaa

SEQ ID NO: 1342 - DNA, 150 bp, Homo sapiens
  source 1..150: mol_type = other DNA
gctcacctgtacaagtctgcctccgccggttacgcctttttagggctcctctccagagtgaattcgagtgtaggttttcaagttggctgggcggttgaactgggctccacggatgttgcaacgctagggattctcacctatttccaagaa

SEQ ID NO: 1343 - DNA, 150 bp, Homo sapiens
  source 1..150: mol_type = other DNA
gctcacctggacaagtctgcctccgccggttacgactttttagggctcctctccagagtgaattcgagtgtaggctttcaagttggctgggcggttgaactgggctccacggctgttgcaacgctagggattctcacctatttccaagaa

SEQ ID NO: 1344 - DNA, 150 bp, Homo sapiens
  source 1..150: mol_type = other DNA
gctcacctggacaagtctgcctccgccggttacgactttttagggcacctctccagagtgaattcgagtgtaggctttcaagttggctgggagcttgaactgggctgcacggctgttgcaacgctagggattctcacctatttccaagaa

SEQ ID NO: 1345 - DNA, 150 bp, Homo sapiens
  source 1..150: mol_type = other DNA
ctaggggacaggggcggggtgggcagcagctcgaatttcttccagatatcctcgctgggcgccgggggctgcagctcgctctgctgctgctgctggtagaagttctcctcctcgtcgcagtagaaatacggctgcaccgagtcgtagtcg

SEQ ID NO: 1346 - DNA, 150 bp, Homo sapiens
  source 1..150: mol_type = other DNA
ctaggggacaggggcggggtgggcagcagctcgaagttcttccagatatcctcgctgggcgccaggggctgcagctcgctctgctgctgctgctggtagaagttttcctcctcgtcgcagtagaactacggctgcaccgagtcgtagtcg

SEQ ID NO: 1347 - DNA, 150 bp, Homo sapiens
  source 1..150: mol_type = other DNA
ctaggggacaggggcggggtgggcagtagctcgaagttcttccagataccctcgctgggcgccaggggctgcagctcgctctgcggctgctgctggtagaagtattcctcctcgtcgcagtagaactacggctgcaccgagtcgtagtcg

SEQ ID NO: 1348 - DNA, 150 bp, Homo sapiens
  source 1..150: mol_type = other DNA
ctaggggacaggggcggggtgggctgtagctcgaagttcttccagataccctcgctgggcgccaggcgctgcagctcgctctgcggctgctgctggtagaagtattcctcctcgtcgcagtagaactacggctgcaacgagtcgtagtcg

SEQ ID NO: 1349 - DNA, 150 bp, Homo sapiens
  source 1..150: mol_type = other DNA
ctaggggacaagggcggggtgggctgtagctcgaagttcttccagatacgctcgctgggcgccaggcgctgcagctcgctctgcggctgctgcaggtagaagtattcctcctcgtcgcagtagatctacggctgcaacgagtcgtagtcg

SEQ ID NO: 1350 - DNA, 150 bp, Homo sapiens
  source 1..150: mol_type = other DNA
ctaggggacaagggcggcgtgggctgtagctcgaagttctttcagatacgctcgctgggcgccaggcgctgcagctcgctctgcggctgctgcaggtagaagtattcctcctcgtcgcagtagatctacgggtgcaacgagtcgttgtcg

SEQ ID NO: 1351 - DNA, 150 bp, Homo sapiens
  source 1..150: mol_type = other DNA
ctaggcgacaagggcggcgtgggctgtagctcgaagttctttcagatacgctcggtgggcgccaggcgctgcagcacgctctgcggctgctgcaggtagaagtattcctcctcgtcgcagtagatctacgggtgcaacgagtcgctgtcg

SEQ ID NO: 1352 - DNA, 150 bp, Homo sapiens
  source 1..150: mol_type = other DNA
ttcttggtaataggtgagaaaccctatcgttgcaacatctgtggggcccagttcaaccggccagccaacctgaaaacccacactcgaattcactctggagagaagccctacaaatgcgaaacctgcggagccagatttgtacaggtgagc

SEQ ID NO: 1353 - DNA, 150 bp, Homo sapiens
  source 1..150: mol_type = other DNA
ttcttggtaataggtgagaaaccctagcgttgcaacatctgtggggcccagttcaaccgcccagccaacctgaaaacccacactcgaattcactctggagaggagccctacaaatgcgaaacctgcggaggcagatttgtacaggtgagc

SEQ ID NO: 1354 - DNA, 150 bp, Homo sapiens
  source 1..150: mol_type = other DNA
ttcttggtaataggtgagaaaccctagcgttgcaacatccgtggggcccagttcaaccgcccagccaacttgaaaacctacactcgaattcactctggagaggagccctacaaaggcgaaacctgcggaggcagatttgtacaggtgagc

SEQ ID NO: 1355 - DNA, 150 bp, Homo sapiens
  source 1..150: mol_type = other DNA
ttcttggaaataggtgagaaaccctagcgttgcaacatccgtggggcccagttcaaccgcccagccaacttgaaaacctacactcgaattcactctggagaggagccctaaaaaggcgaaaccggcggaggcagatttgtacaggtgagc

SEQ ID NO: 1356 - DNA, 150 bp, Homo sapiens
  source 1..150: mol_type = other DNA
ttcttggaaataggtgagaatccctagcgttgcaacatccgtggagcccagttcaaccgcccagccaacttgaaaacctacactcgaattcactctggagaggagccctaaaaaggcgtaaccggcggaggcagacttgtacaggtgagc

SEQ ID NO: 1357 - DNA, 150 bp, Homo sapiens
  source 1..150: mol_type = other DNA
ttcttggaaataggtgagaatccctagcgttgcaacagccgtggagcccagttcaaccgcccagccaacttgaaagcctacactcgaattcactctggagaggagccctaaaaagtcgtaaccggcggaggcagacttgtccaggtgagc

SEQ ID NO: 1358 - DNA, 150 bp, Homo sapiens
  source 1..150: mol_type = other DNA
ttcttggaaataggtgagaatccctagcgttgcaacagccgtgcagcccagttcaagctcccagccaacttgaaagcctacactcgaattcactctggagaggtgccctaaaaagtcgtaaccggcggaggcagacttgtccaggtgagc